European Patent Application EP 4 368 707 A1, published May 15, 2024. Title: Method for preparing a reassortant virus of the family Reoviridae. Applicant: SK bioscience Co., Ltd. The sequence listing filed with the application follows.

SEQUENCE LISTING (56 sequences)

SEQ ID NO: 1 - DNA, 3302 bp, Artificial
  VP1B gene segment cDNA
ggctattaaagctatacaatggggaagtataatctaatcttgtcagaatatttatcatttatatataactcacaatctgcagttcaaattccaatttattattcttccaatagtgaattagagaatagatgtattgaatttcattctaaatgcttagaaaactcaaagaatggactaccactaaaaaaactctttgttgaatatagcgatgttatagagaatgccacactgttgtcaatattatcgtactcttacgataaatataacgctgttgaaaggaaattagtaaaatatgcaaaaggtaagccgctagaagcagatttgacagtgaatgagttggattatgaaaataacaagataacatctgagcttttcccaacagcagaggaatatactgattcattgatggatccagcaattttaacttcattatcatcaaatttgaatgcagttatgttctggttggaaaaacatgaaaatgatgctgctgaaaaactcaaaatttacaaaaggagattggacttatttactatagtagcttcaacagtaaataaatatggtgtaccaaggcacaatgagaaatatagatatgaatatgaagtgatgaaagataagccgtactacttggtaacatgggcaaattcttcaattgaaatgctaatgtcagttttttctcatgaagattatttaattgcgagagaactgatagtactgtcatattctaatagatcgactctagcaaaactggtgtcatcaccaatgtcaattctggtagctttagtggatataaacggaacatttattacgaatgaagaattagagctagagttttcaaacaaatatgtacgagcaatagttcctgaccaaacatttgacgaattaaaacagatgcttgacaacatgagaaaagctgggttaactgacatacctaagatgatacaggactggttagccgattgctctattgaaaaatttccattgatggctaaaatatattcgtggtcatttcatgtcggattcaggaagcagaaaatgttggacgccgcgttagatcaattgaaaactgagtatacagaagatatagatgatgaaatgtatcgagaatatacaatgctaataagagatgaagttgtgaaaatgcttaaggaaccagtaaagcatgatgatcatttgttacaggattctgaattggctggtttactatcaatgtcatcagcgtcgaatggtgaatcaagacaactaaaatttggtagaaagacaattttttcgactaaaaagaatatgcatgtaatggatgacatggctaatggaaggtatacgccaggcataataccaccagtgaatgtcgataaaccgataccattaggaaggagagatgtaccaggaagacggactagaataatattcatcttaccatatgaatattttatagcacaacatgccgtagttgaaaaaatgctaatttatgcgaaacatactagagagtatgctgaattctactcacagtcaaatcagttattgtcttatggtgatgttacacgctttttatctaataactctatggtgctatatacagacgtatcccagtgggactcatctcaacacaatacgcagccatttaggaaagggataattatggggttggacatgctagctaatatgactaatgatgctagagtcatccagacactaaacttatataaacagacgcaaattaatctaatggattcatacgttcaaataccagatggtgatgttattaaaaagatacaatatggggctgtagcgtcaggagaaaagcagacgaaagcagcgaattcaatagcaaatttagcactgattaaaacagttttatcacgtatttctaacaaatattcattcgcgacgaagataataagagttgacggagatgacaattacgcagtattgcagttcaatacagaagtaactaaacaaatggttcaagatgtatcaaacgacgtgagagaaacgtatgcgcgaatgaatgctaaagtcaaagctttagtatctacagtgggaatagaaatagctaaaaggtatattgcaggtgggaaaatattctttagagctggaataaatttactgaataacgaaaagagaggacaaagtacacagtgggatcaagcagctgttctatattcgaactatattgtgaatagacttcgaggatttgaaactgacagagagttcattttgactaaaataatgcaaatgacatcagttgctattacaggatcactaagactctttccttctgaacgcgtgttaaccacgaactctacgtttaaagtgtttgactcggaggactttattatagagtatgggacaactgacgacgaagtatacatacaaagagcgttcatgtctttatctagtcagaagtcaggaatagctgatgagatagctgcatcatcaacgtttaagaattatgtatctagattatctgagcagctgttattttcaaagaataatatagtgtctaagggaatagcattgactgaaaaagcaaaattgaactcatacgcgccaatatcacttgagaaaagacgcgcgcaaatatcagctttgctgactatgctgcaaaaaccggttacttttaaatcaagtaagataacaataaatgatatacttagagatataaagccatttttcactgtaagcgaagcgcatttgccgatacaatatcaaaaatttatgccaactttaccagacaatgtacagtatataattcagtgtataggatccagaacatatcaaattgaagatgacggttcaaagtcagctatatctcgactaatatcaaagtactcagtttacaagccgtcaatcgaagagttatacaaagtaatttcactacatgagaatgaaatacaactatatttgatctcactaggcataccgaaaatagacgctgatacgtacgtcggatcgaaaatttattctcaagataaatacaggatattagagtcgtatgtatataatttattgtctattaattatggatgttatcagctattcgacttcaattcaccagatctagaaaagctgatcagaataccgtttaaaggaaagataccagctgtcacttttatattgcatttatacgctaagctggaagttataaatcatgccattaaaaatggctcatggataagtttattctgtaactacccaaaatcagaaatgataaaattatggaagaaaatgtggaacattacgtcactacgttcaccgtataccaatgcaaacttctttcaagattagagcgcttagatgtgacc

SEQ ID NO: 2 - DNA, 2687 bp, Artificial
  VP2B gene segment cDNA
ggctattaaaggctcaatggcgtacaggaaacgtggagcgcgccgtgaggcgaatataaataataatgaccgaatgcaagagaaagatgacgagaagcaggatcaaaacaatagaatgcaattatctgacaaagtactttcaaagaaagaggaagtcgtaaccgacaatcaagaggaaattaagattgctgatgaagtgaagaaatcaacgaaagaagaatctaaacaattgcttgaagttttgaaaacaaaagaagagcaccaaaaagaaatacagtatgaaattttacaaaaaacgataccaacatttgaaccaaaagagtcaatattgaagaaattggaagatatcaaaccggaacaggcgaagaagcagactaagctatttagaatatttgaaccgagacagctgccaatttatagagcaaatggtgaaaaagagttgcgtaacagatggtattggaagttgaagaaggatactttaccagatggagattatgacgttagagagtattttctaaatttgtatgatcaggttcttactgaaatgccagattatttactattaaaagatatggcagttgaaaataaaaactcaagagatgctggtaaagttgtcgattctgaaacggcaagtatctgtgatgctatatttcaagatgaggaaacagaaggcgcagtgagaagattcattgcggagatgagacaacgcgtacaagctgacaggaacgttgtcaattacccatcaatattacatccaatagattacgctttcaatgagtattttttacaacatcaattagttgaaccattaaataatgatataatattcaattacattcctgaaaggataaggaatgacgttaactatatacttaatatggacagaaatctgccatcaacagctagatatataagacctaatttactacaagacagactgaatttgcacgataattttgaatccttgtgggatacgataacaacttcaaactatattctggcaagatcggtagtaccggatttaaaggaattagtttcaaccgaagcgcaaattcaaaaaatgtcgcaagatttgcaactagaagcattaacaatacagtcagaaacgcagtttttaacaggtataaactcacaagcggcaaatgactgtttcaaaactctgattgcagcaatgttaagtcaaagaaccatgtcgcttgatttcgtgactacaaattatatgtcattaatttcaggtatgtggttactaactgtagtgccaaatgacatgttcataagggaatcattggttgcatgccaactggctatagtgaatacaataatatatccagcgttcggaatgcaacgaatgcattatagaaacggagatccacagacaccatttcagatagcagaacagcagatacaaaatttccaggtagcgaattggctgcattttgtcaataacaatcaatttagacaagtagttattgatggtgtattgaatcaggtactgaatgacaatattagaaatggacatgtcattaatcagttgatggaggctttaatgcaactatcacgacaacagtttccaacaatgcctgttgattataagaggtcaatccagcgtggaatattattgctatcaaataggcttggtcaattagttgatttaactaggttattagcttacaactacgaaacactaatggcatgtgttacgatgaatatgcaacatgttcagactttgacaacagaaaaattacagttaacttcagtcacgtcgttgtgtatgcttattggtaatgcaaccgttatacccagcccgcagacattatttcactattataatgttaatgttaattttcattcaaattataatgaaagaattaatgatgcagtggccataataactgcagctaatagactaaatttatatcagaaaaagatgaaggcaatagttgaagattttttaaaaagattacacattttcgatgtagctagagttccagatgatcaaatgtatagattaagggatagactacgactattgccagtagaagtaagacgattggatatttttaatttgatactgatgaacatggatcagatagaacgtgcctcagacaagattgcgcagggtgttattattgcataccgcgatatgcaattggaaagagatgaaatgtatggctacgtgaatatagctaggaatttagatgggttccagcaaataaacctagaagaattgatgagaacgggcgattatgcacaaataactaacatgctcttgaataatcaaccagtagcgctagttggagctcttccatttgttacagactcgtcagtcatatcgttaatagcgaagcttgacgctacagtttttgcccagatagttaaattacggaaagttgataccttgaaaccaatattgtataaaataaattcagattcgaatgacttttatctagttgccaattatgattgggtgcctacttcaaccacaaaagtatataaacaagttccacagcaatttgatttcagaaattcgatgcatatgttaacgtcaaatcttactttcaccgtttactcagatctgcttgcattcgtatcggccgatacagtagaacctataaatgcagttgcatttgataatatgcgcatcatgaacgagttgtaaacgccaaccccactgtggagatatgacc

SEQ ID NO: 3 - DNA, 2591 bp, Artificial
  VP3H gene segment cDNA
ggctattaaagcagtactagtagtgcgttttacctctgatggtgtaagcatgaaagtattagctttaagacacagtgtggctcaggtgtatgcagatactcaaacctatttacatgatgattcaaaagatgagtatgaaaatgcatttctcatttctaatctaactacacataatatattatacctgaattacaatcttaaaacattaaaaatattaaataaatcaggtatagcagcagttgaagtacaatctccagatgaattatttgcgttaataaggtgtaattttacgtacgattatgagaataacatagtttatttacatgattattcatattatactaacaatgaaataagaacagatcaacattggataactaaaactgatataattgactatctattacctggatggaagttaacgtatgtaggttataatggaaagaatacaagaggtcactataatttttcatttatatgtcaaaatgcagctacagatgatgatataataattgaatatatatactccaatgagttagactttcaaaattttctgttgagaaaaattaaagagagaatgaccacatctcttccaattgctagattatcaaatcgtgtgtttagagataaattatttccatctattgtaaacatacataaaaaagtgataaatgttgggccgaggaatgaatctatgttcacattcctaaattttccaactattaagcaattttcaaacggtgcgtatattgtgaagcataccattaaattgaagcaagagaaatggttgggtaaaagagtatcacaatttgatatcggacaatataaaaacatgttaaatgtggtcactactatttactattactataatttatactattcgaaacctataatatacatgcttggttcagctccatcttattggatttatgatattaaacagtattctgactttacatttgaaacatgggatccattagatactccgtattctacaacacatcataaagaattattttttgacaaggatgtcaataagcttaaagataattcagttttatatatagacataagaactgatagaggtaatatggattggaaagagtggagaaaaatagtagaacaacaaactgttagcaatctaaatattgcatataaatatctatcaacaggaaaagcaaaggtgtgttgtgttaaattaactgctatggacctagaattaccaataacagcaaaattacttcatcatccaactactgaagttagatcagaattttatgcaatattggatgtatgggatattattaccattaaaagatttataccaaaaggtgtattttatgcttttataaataacgtaaccacagagaatgtgtttatacaacctccttttaaattaaaaacgtcacctactgattatatagtggcattgtatgctttatccaatgacttcaattcaaggcaagatgttattaatttgattaataaacaaaaacaatcactcattactgttcgtataaataacgcttttaaagacgagccaaaagtaaattttaaaaatatttatgattggacgtttctgccaacagatttcgaacttaaagattcgataattacatcatatgatggttgtttaggcatattcggattatcaatatctttatcgtctaaacccaccggaaataatcatttatttataataaatggaactgacaaatatgataaactagaccaatatgcaaatcatatgggtatttctagaagatcgcatcaaattagattctcagagtctgcgacatcatattcgggatatatttttagagatctttcaaataataatttcaatctaataggtactaatgtggagaattcagtttcaggacatgtctataatgcattgatttactacagatataattatgcgtttgatcttaaaagatggatttatctacattcaattggaaaagtcgctgtagaaggtggaagatattatgaacatgcaccaatcgaattgatatatgcatgccgatcagctaaagaatttgctatattacaagatgacttaacggtattgagatacgctaatgaaattgaagggtatataaacaaagtatatagtataacctatgctgacgatcccaattactttataggaattaaatttaatagtataccttatgaatacgatgttaaaattccacatttgacactaggagtattatttatatctgataatatgatacatgatgtaatcatagtgctgaagaaaatgaagacagaactatttaaaatggaaattagtactagttatacttatatgctatctgataatatgtatgtagcaaatgctagtggtgtgttatcaacttattttaaattatataatatgttctatagaaatcatatcacgtttggacaatcacgaatgtttatcccacacattacgctcagttttagcaacaaacagacagttagaatagagagtacaaaactcggaatcaattcaatttacttaagaaagattaaaggtgaaaccgtatttgatatgtctgagtgagctagaaacttaacacactagtcatgatgtgacc

SEQ ID NO: 4 - DNA, 2591 bp, Artificial
  VP3B gene segment cDNA
ggctattaaagcaatattagtagtgtgttttacctctgatggtgtaaacatgaaagtattagctttaagacatagtgtggctcaggtatatgcggacactcaaatatatactcatgatgaaaccaaagatgactacgagaacgcatttttaatttctaatctcactacacataatatattgtatctaaattatagcgttaagacattgcaaatattgaataaatctggtatagctgcggtagaaatacaggagatggatgaattgtttacgctaattagatgcaacttcacatatgattatattgacgacattgtttaccttcatgattattcatactatactaataatgagataaggactgatcaacattgggtaactaaaacaaatatagaagactatttattaccaggatggaaactgacgtatgttggatataacggaaatgacacaagagggcactataacttttcttttaaatgtcaaaatgcagctacggacgatgatgcaataatagaatatatttattcaaatgaattggacttccaaaatttcatacttaaaaaaatcaaagaaaggatgacgacatcactgccaatagcgagattatcgaatcgtgtgttcagagacaaattatttaagacgctagtatcagatcacagtagagtagttaacgttggaccaagaaatgaatctatgtttacttttctagatcacccgtcaataaagcaattttcaaatggaccctatttagttaaagatacgataaagcttaaacaagagagatggctcggtaagagactatcgcaatttgacattggtcagtataagaacatgctaaatgtattaacaactttataccaatactatgacatgtatcatgagaagccaataatttacatggtaggatcagcaccttcatattggatacacgatgtcaggcaatactctaatttaaagtttgagacatgggacccattggatacaccatactctgatttgcatcataaagaattgttttatataagtgacgtaaccaaacttaaagataattcgatattatatgtagatatacgaacggatagagaaaatacagattggaaagcgtggaggaagattgtggaagagcaaactataaataatttgaatatcgcatacaaatacttatccacaggaaaagctaaagtatgttgtgttaaaatgactgccatggatttagaactaccaatatctgcaaaactactacatcatccaactacagaaattaggtcagaattttatttaataatggatatatgggattctaaaaatattaaacgatttataccgaagggcgtgttatattcatatattaacaatgtaattactgagaacgtgttcatacaacaaccgtttaaattgaaaacgttaaggaatgaatatgtggttgcattatacgcactgtctaacgactttaataatagagaggatgtgataaaattggttaacaatcagaagaatgcgttaataactgtgaggataaataatacatttaaagatgaaccaaaagtggggtttaaagatatttatgactggacttttttgccaactgatttcgaaacgaatgagtcaataatcacgtcatatgatggttgtttaggtatgtttggcttatcaatatcattagcttcaaaaccaactggaaataatcatctgttcattttgagcggtactaataaatattttaaattggatcaatttgcgaatcatatgagtatatcaagacggtcacatcaaatacgattttcggaatcagcgacttcatattcaggttacatttttagagatttatcaaataataattttaatttaataggtacgaatgttgagaattcggtatctggacatgtgtacaatgcattgatttattatagatataattattcattcgatcttaagcgatggatatacttacatgcaacaaacaaggctggcattgaaggcggcagatactatgaacatgctccgatagagttgatttacgcatgtagatcggcaaaggaattcgcaaaattgcaagatgatttaacagtactaagatattcgaatgaaatagaagattacattaataaagtgtacagtataacatacgccgacgatccgaactactttattggaattaagttcaaaaatataccatatgaatatgatgttaaagtaccgcatcttacatttggtgtattaaatatttcagattccatggtgccggatgtagtagcaattttaaagaagtttaaaagtgaattgtttagaatggatgtaaccacaagttatacgtatatgttgtcagatgaaatctatgtggcaaacgtaagtggtgtgttatcaacatattttaaactttacaatgcattctataaagagcaaattacgtttggacaatcaagaatgtttattccgcacataacattaagtttcagtaacaagaaagtagtgagaatagatagtacgcgattgaacatagactttatatatttgaggaaaataaaaggcgatacagtgttcgatatgactgagtgagctaaaaacttaacacactggtcacgatgtgacc

SEQ ID NO: 5 - DNA, 2362 bp, Artificial
  VP4B gene segment cDNA
ggctataaaatggcttcgctcatatacagacagctgctcgctaattcttacgcagtggatttgtctgatgagatacagtcagttggatcagagaagaaccagcgcgttacagtgaatccaggaccatttgcgcagacagtatatgcgccagtgaactggggacccggtgaagtgaatgactcgactgtagtacaacctgtgttggacggaccgtatcagccagcgtcgttcgatctaccagtaggaaattggatgttgttagcgccaacaggaccaggtgtggtagtggaagggacggacaattctggcagatggttatctgtaattctgattgaaccaggtgtcacatcagaaactaggacgtatacgatgtttggatcaagtaaacaggtgttagtgtcgaacgcgtctgatacgaaatggaaatttgttgaaatgatgaagacggcgattgatggtgactatgcggaatggggaacattactatcagacaccaaactctatgggatgatgaaatatggaaagagactattcatatacgaaggagaaaccccaaatgccacgaccaaaagatacattgtgacgaattatgcatcagttgaggtaaggccatatagtgacttttatataatttcaagatcacaggaatcagcatgcactgagtatataaacaacggactgccacccatccaaaataccaggaatgtagtgcctgtggcaatatcgtcaagatcaattgaaccaagaaaagtgcaggctaatgaagatattgtagtttctaagacgtcactatggaaagaaatgcaatataatagagatatcataattagatttaggtttgataactcaataataaaatctggaggtttgggctataagtgggctgaaatctcatttaaagctgcaaattatcaatacaattacatgagagacggagaagaagttacagcgcatacgacgtgctcagttaatggtgttaatgattttagctttaacggaggctcattaccaacagatttcgcaatatcgagatatgaagtaattaaagaaaattcgtatgtatacgttgattactgggacgattcacaggcattcagaaatgtggtctatgtgcgatcattggcagcgaatttgaatgacgtaatgtgttctggcggagattacagcttcgcgctacctgtcggacaatggccagtgatgaaagggggagcggtgacgttgcacacagcaggagtaacattatctacacaattcactgactacgtatcactgaactcactaaggtttagatttagactggcagtcgaagaaccatcattcacgataactagaacacgtgtatcaaaactgtatggtttaccagcggcgaacccaaacggcggaagggaatattatgaagtggcaggaaggttttcgctgatatcattggtgccatcaaatgatgactaccaaacgccaattatgaactcagtaacagtaagacaagacttggaaaggcgtttaaatgagttgagagaagagttcaataacttatcacaagagatagctgtgtcacagttaattgacttagctatgctgccactagacatgttttcgatgttctcgggaattgagggtactgtgaacgcagcaaaatcgatggctaccaacgtgatgaggaaattcaaaagttcaaaactcgcatcatcagtgtcaatgttgacggactctttgtccgatgcggcctcatctatcgcaaggagcacatcaatacgatcaataggatcgacggcatcagcttgggctaatatttcagaacaaacgcaagacgccgttaatgaagttgcgacgatatcatcacaagtgtcacaaataagtgggaaattaagattaaaagaaattacgactcaaacagaaggaatgaatttcgatgacatatcagcggcggtgctaaaagccaagatagatagatcaatacaggtcgaccaaaacgcattaccagacgtcatcacagaagcgtcagagaaattcatacgtaatagggcgtatagagtaatagacggagatgaagcatttgaggcgggcactgacggaagatttttcgcgtacaaggtggaaacgcttgaggaaatgccattcaatatagaaaaattcgcagatttagttaccaactcaccagtgatatcggcaataatagactttaagacattaaaaaacctgaatgacaattatgggataactagagagcaagcatttaatctgttacggtcaaaccccaaagttttgcgtggatttattgaccaaaacaatccaattataaaaaacagaatagaacaattaatcatgcaatgtagattgtgagcagcttctggaggatgtgacc

SEQ ID NO: 6 - DNA, 2359 bp, Artificial
  VP4P1 gene segment cDNA
ggctataaaatggcttcgctcatttatagacaacttctcacaaattcatactcagtagatttacatgatgaaatagaacaaattgggtcagaaaaaactcaaaacgtaactgtaaatccaggtccgttcgcccaaaccaggtatgctccagtcaattggggttatggagagataaatgattcaaccacagtagaaccaattttagacggtccttatcagcctactacatttacaccacctattgattattggatacttattaactcaaatacaaatggagtagtatacgagagtacgaataatagtgacttttggactgcagtcgttgctattgaaccgcacgttaatccagtagatagacaatacactgtatttggtgaaaataaacaatttaatgtaagaaatgattcagataagtggaagtttttagaaatgtttagaagtagtagtcaaaatgaattttataatagacgtacactgacttctgatactaaacttgtgggaatattaaaatatggtggaagaatatggacgtttcatggtgaaacaccgagagctactactgatagttcaaatactgcaaatttaaacgatatatcaattataatacattcagaattttatattattccaaggtctcaagagtctaagtgtaatgaatatattaataatggtttaccaccaattcaaaatactagaaatgtagtaccattatcattatcatctagatccatacagtataagagagctcaagttaatgaagaaattacaatttcgaaaacctcattatggaaagaaatgcaatataatagtgatattataattagatttaaatttggtaatagtattgtaaaactgggaggattaggttataaatggtccgaaatatcatttaaggcagcaaactatcaatataattatttacgtgatggcgaacaagtaactgcacatactacttgctcagtaaatggagtaaataattttagctataacgggggatctttacctactgattttagcatctcaagatatgaagttatcaaagaaaattcttatgtatacgtagattattgggatgattcaaaagcatttagaaatatggtatatgtcagatcattagcagctaatttaaactcagtgaaatgtgcaggtggaaggtatcactttagtttacctgtaggtgcatggccagttatgaatggaggcgctgtttcgttacattttgctggagttacattatctacgcaattcacagatttcgtatcattgaattcattacgatttagatttagtttgacagtggatgaaccatctttttcaatattgagaacacgtacggtgaatttgtacgggttaccagcagctaatccaaataatggaaatgaatactacgaaatatcaggaagactttcgctcatttctttagttccaactaatgatgattatcagactccaattatgaattcagtaacagtaagacaagatttagaacgtcaacttactgatctacgagaggaatttaattcattatcacaagaaatagctatgtcacaattaattgacttagcgctattacctttagatatgttttctatgttttcaggaattaaaagtacaattgatctgactaaatcaatggcaactagtgtaatgaaaaaatttagaaaatcaaaattagctacatcaatttcggaaatgactaattcattatcagacgcagcatcatcagcatcaagaagcgtttctatcagatcgaatatatccacaatttcgaatttgactaacgtttcaaatgatgtatcaaatgtgactaattcgttgaatgatatttcaacacaaacgtctacaatcagtaagaaacttagattaagagaaatgattactcaaactgaaggaatgagttttgatgatatttcagcggcagtattaaaaacaaaaatagatatgtctactcaaattggaaagaataccttacccgacatagtcacagaggcatctgagaaatttattccaaaacgatcatatcgaatattaaaagatgacgaagtgatggaaattaatactgaagggaaagtctttgcatataaaatagatacacttaatgaagtaccatttgacgtaaataaatttgctgaacttgtaacaaattctccagttatatcagcaataattgattttaaaacattaaaaaacttgaatgataattatggaattactcggatagaagcactaaatttaattaaatcaaatccaaatgtattacgtaatttcattaaccaaaataatccaattataaggaacagaattgaacagctaattctacaatgtaagttgtgagaatgctattgaggatgtgacc

SEQ ID NO: 7 - DNA, 1356 bp, Artificial
  VP6B gene segment cDNA
ggcttttaaacgaagtcttcaacatggatgtcctgtactccttgtcaaaaactcttaaagatgctagagacaaaattgtcgaaggcacattatactccaatgtaagtgatctaattcaacaatttaatcaaatgataattactatgaatggaaatgagttccaaactggaggaattggtaatctaccgattagaaattggaattttgattttggattacttggaacaactctattaaatctagatgctaactacgtcgaaacggcccgcaacacaattgattattttgtagattttgtagacaatgtatgtatggatgaaatggttagagaatcacaaagaaatggaattgcaccacaatcagattcacttagaaagttatcaggcattaaatttaaaagaataaattttgacaattcatcagaatacatagagaactggaatttgcaaaacagaagacaaagaacgggttttacatttcataaaccaaacattttcccttattcagcgtcattcacactgaacagatcacaaccagctcatgataacttgatgggtacgatgtggctcaatgcgggatcagaaattcaggtcgctggattcgactattcatgtgcaatcaatgcgccagccaatacacaacaatttgagcacgttgtacagctccgaagagtgttaactacagctacaataactcttttaccagatgcagaaagatttagttttccaagagtgattaattcagctgacggagcgactacatggtacttcaacccagtgattcttagaccaaataacgttgaagtagaatttctattaaacgggcagataataaatacttaccaagcaagatttggaacgatcatagctagaaattttgatacaatcagattgtcatttcagttgatgagaccaccaaatatgacaccagcggtagcggcgttatttccaaatgcacagccatttgaacatcacgcaacagtaggactcacgcttagaattgaatctgcagtttgtgaatcagtgcttgccgacgcaagtgaaacaatgctagcaaatgtgacatctgttagacaagaatacgcgataccagttggaccagtttttccaccaggtatgaattggactgatttgatcactaactattcaccatctagagaggataacttgcagcgtgtatttacagtggcttccattagaagcatgcttgtcaaatgaggaccaagctaaccacttggtatccgactttggtgagtatgtagctacgtcaagctgtttgaactctgtaagtaaggatacgtctacgtattcgctacacagagtaatcactcagatggcgtagtgagaggatgtgacc

SEQ ID NO: 8 - DNA, 1062 bp, Artificial
  VP7G1 gene segment cDNA
ggctttaaaagagagaatttccgtctggctaacggttagctccttttaatgtatggtattgaatataccacaattctaatctttttgatatcaatcattctactcaactatatattaaaatcagtgactcgaataatggactacattatatatagatttttgttgattactgtagcattatttgctttgacaagagctcagaattatggacttaacttaccaataacaggatcaatggacgctgtatatactaactctactcaagaagaagtgtttctaacttctacgttatgtctgtattatccaactgaagcaagtactcaaatcaatgatggtgactggaaagacacattgtcgcaaatgtttcttacaaagggttggccaacaggatctgtttactttaaagagtactcaagtattgttgatttttctgttgacccacagctgtattgtgactataatttagtatttatgaaatatgaccaaagtcttgaattagatatgtcagagttggctgatttaatattgaatgaatggttatgtaacccaatggatgtaacgttatactattatcaacaatcgggagaatcaaataagtggatatcgatgggatcatcatgtaccgtgaaagtgtgtccgctaaatacacaaacgttaggaataggttgtcaaacaacaaacgtagactcatttgaaatgatcgctgagaatgagaaattagctatagtggatgtcgttgatgggataaatcataaaataaatttaacaactacgacatgtactattcgaaattgtaagaaattaggtccaagagaaaatgtagctgtaatacaagttggtggttctaatgtgttagacataacagcagatccaacaactaatccacaaactgagagaatgatgagagtgaattggaaaaagtggtggcaagtattttatactatagtagattatattaatcaaattgtacaggtaatgtccaaaagatcaagatcattaaattctgcatctttttattatagagtatagatatatcttagattagaattgttcgatgtgacc

SEQ ID NO: 9 - DNA, 1062 bp, Artificial
  VP7G2 gene segment cDNA
ggctttaaaaacgagaatttccgtctggctagcggttagctctttttaatgtatggtattgaatataccacaattctgaccattttgatatctattatattattgaattatatattaaaaactataactaatacaatggactacataatctatagatttttactagtcattgttctgatatcaccatttgtaagaacacaaaattatggcatatatttaccaataacgggatcactagacgctgtatatacgaattcaactagtggagaaacatttctaacttcaacactatgcttatactatccagcagaagctaaaaatgagatttcagatgatgaatgggaaaatactctatcacaattatttttaactaaaggatggccaactggatcagtttattttaaagactacaatgacattactacattttccatgaatccacaactgtattgtgattataatgtagtattaatgagatatgataatacatctgaattagatgcatcggagttagcagatcttatattgaatgaatggctgtgcaatcctatggatatatcactttactattatcagcaaagtagcgaatcaaataaatggatctcaatgggaacggattgcacggtaaaagtttgtccacttaatacacaaacgttaggaattggatgcaaaactactgacgtgagtacatttgagatagttgcgtcgtctgaaaaattagtaattactgacgttgtaaatggtgttaatcataagataaatatttcaataagtacgtgcactatacgtaactgtaacaaattaggaccacgagaaaatgttgctataattcaagttggtggaccgaatgcattagatatcactgctgatccaacaacagttccacaaattcaaagaatcatgcgaataaattggaaaaaatggtggcaagtcttttatacagtagttgattacattaaccaaattgtacaagttatgtccaagcggtcaagatcattagacgcagctgctttttattatagagtttagatatagctttggtcagatttgtataatgtgacc

SEQ ID NO: 10 - DNA, 1062 bp, Artificial
  VP7G3 gene segment cDNA
ggctttaaaagagagaatttccgtttggctagcggctagctccttttgatgtatggtattgaatataccacagttttaacctttttgatatcagttatattgttgaattacgtactcaaatcactaactagaataatggactttatcatttacagatttcttttaattatagttatactgtcaccactccttaatgcacaaaattatggaataaatcttccgattactggatcaatggacacatcatatacgaactcaacgcgagaggaagtattcctgacttcgactttatgtttgtattatccaactgaagcagcaacagaaataaatgataactcatggaaggatacactttcgcagctatttttaactaaaggatggccaacagaatctatttattttaaagattatactgatattgcctcgttttcagttgatccacaactgtactgtgattataatttggtattaatgaagtatgacgctacactgcaattggatatgtccgaactagcagatttgttacttaatgagtggttatgtaatcctatggacatcactttgtattattatcaacaaactgatgaagcaaataaatggatttcgatgggatcatcttgtaccataaaagtatgtccattaaatacgcaaacattaggaattgggtgtctaactactgatgcaaatactttcgaagaagttgcaacagctgaaaaattagtaattactgacgttgtagatggggtcaatcataaattgaaagtgacgacggatacttgtacaattagaaattgtaaaaaattaggaccaagggaaaacgtagcagttatacaggttggtggctcagatgtacttgacataacagctgatccaacgacagcaccacaaacagaaagaatgatgcgagtgaattggaagaaatggtggcaagtattttatacaatagttgactatgtgaatcaaattgtgcaagcgatgtccaaaagatcgagatcattaaattctgctgcattttattacagagtatagatatagcttaggttaaggctgtaagatgtgacc

SEQ ID NO: 11 - DNA, 1062 bp, Artificial
  VP7G4 gene segment cDNA
ggctttaaaagagagaatttccgtttggctagcggatagctccttttaatgtatggtattgaatataccacagttctattttatttgatatcgttcgttcttgtgagttatattctgaaaactatgataaagataatggactatttaatttatagaataacatttgtaattgtagtattatcagtattatcgaatgcacaaaattatggaataaatttgccaattactggatctatggatacagcatatgctaactcaacacaagacaataattttttatcttcaactttatgtctatattatccatcagaagctccaactcaaattagtgacactgaatggaaagatacactatctcaactgtttttaaccaaaggatggccgacaggttcagtttattttaatgaatattcaaacgttttagaattttccatcgacccaaagctatactgtgattataatgttgtgttaattagattcgcttctggtgaggagttggacgtatctgaattagctgatctaatactcaatgagtggttatgtaatccaatggatataacattatattattatcaacaaactggagaggcaaataagtggatatcaatgggatcatcatgtaccgttaaagtgtgtccattaaatactcagacattaggaattggatgtcaaacgacagatactgctacttttgaaacagttgctgacagcgaaaaattggcattaattgatgttgttgacaacgtaaatcataaattagatgttacatctactacgtgtacaatacggaattgtaataaactaggacctagagaaaatgtggctataatacaggttggcggttctaatatattagatataacagctgatcccacaacttctccacaaacagaacgaatgatgcgcgtaaactggaaaaaatggtggcaagtattctatactgtagttgattacattaatcaaatagtaaaagtaatgtccaaaagatcaagatcgttagattcgtcatctttctattatagagtatagatatatcctaaaatagaactgtttgatgtgacc

SEQ ID NO: 12 - DNA, 1061 bp, Artificial
  VP7G9 gene segment cDNA
ggctttaaaagagagaatttccgcttggctaacggttagctccttttaatgtatggtattgaatataccacagttctaacctttttgatatcaatcattttgttgaattatatactaaaatcattaactagtgcaatggactttataatttatagattccttttgcttatagtcattgtatcaccatttgttaagacgcaaaattatggaattaatttaccaatcactggctccatggatacggcatatgcaaactcatcacagctagatacatttttaacttcaacgttatgtttatattaccctgctgaagcatcaactcaaattggagatacagaatggaaagacactctgtctcaattgttcttgactaaagggtggccaactgggtcagtctattttaaagaatatactgacatcgcttcattttctattgatccacaactttattgcgattataatgttgtattaatgaagtacgattcaacattagagttagacatgtctgaactagctgatttgattctaaacgaatggttatgtaatccgatggatataacactatattattatcaacaaacagatgaagcgaataaatggatagcgatgggacaatcttgtacaataaaagtgtgtccgttgaatacgcagactttaggaataggctgtacaactacaaatacagcaacatttgaggaagtggccgcaagtgaaaaattagtgataactgatgttgttgatggtgtgaatcataaactagatgtaactacaactacttgtactattagaaattgtagaaaattaggaccaagagagaatgtggcaattatacaagttggcggctcagaagtgctagatattacagcagacccaaccactgcgccacaaactgaacgtatgatgcgaataaattggaaaaaatggtggcaagttttttatacggtagtagattatatcaatcagattgtgcaagttatgtccaaaagatcgcgatcgttgaattcagcagctttctactatagagtctgatatatctcaggttagaattggtcgatgtgacc

SEQ ID NO: 13 - DNA, 1062 bp, Artificial
  VP7B gene segment cDNA
ggctttaaaagcgagaatttccgtttggctagcggttagctccttttaatgtatggtattgaatataccacaattctaatcttcttgacatcgattacattattgaattatatcttaaaatcaataacgagaataatggactatataatttatagatttttgtttatggtagtgatcttggccaccataataaatgcgcaaaactatggagtaaatttgccaattacaggttcaatggatactgcgtatgcaaactctacacaaagtgagccatttttgacatcaaccctttgtttgtattatcctgttgaggcatcaaacgaaatagctgatactgaatggaaagataccttatcacaactgttcttaacaaaaggatggccaacaggatcagtgtactttaaagaatatgctgatatagcggccttttcagtggaaccacagttatactgtgattataatttagttttaatgaaatatgactctacacaaaaactagatatgtctgaattggccgatcttatattgaatgaatggctgtgcaatccaatggacataacgctatattattatcagcagactgatgaggcaaataaatggatatcaatgggctcttcttgcacggttaaagtgtgtccattaaatacacaaacacttggtattggatgtctaataactaatccagacacgtttgaaacagttgcgacaacggagaaattagtgattacagatgttgtagatggtgtcaaccacaaattaaacgtcacaacggcaacgtgcaccatacgcaactgtaaaaagttaggaccaagggagaacgtagcagtcatacaggtaggcggcgcgaacattttagacatcacagctgatccaacaactacaccacagacagagagaatgatgcgaataaattggaaaaaatggtggcaagtgttttacacggtagtggattacgtcaatcaaataattcagacaatgtccaaaagatctagatcgcttaattcgtcggcgttctactatagagtgtaggtgcatgttagattagagttgtacgatgtgacc

SEQ ID NO: 14 - DNA, 1578 bp, Artificial
  NSP1B gene segment cDNA
ggctttttttatgaaaagtcttgtgtgagccatggcgacttttaaagacgcttgttatcattataaaaagttgaataagttaaatagtttagtgctcaaactaggagcaaatgatgaatggaggccagcaccagtgacaaaatataaaggatggtgtttagattgttgtcaatatacaaatttgacatattgcagagggtgcgctctataccatgtatgtcagtggtgcagtcagtataacaggtgtttcttagatgaagaaccccatttgctgagaatgcgaacatttaaagatgtagtaacaaaggaagatatagaagggctgctaaccatgtatgaaacgttgtttccaataaatgaaaagttggtgaataaattcataaactctgtgaaacagcgtaagtgtaggaatgaatatttgttagaatggtataatcacttactaatgccaataacattacaagcattgactataaatcttgaggataatgtatattatatatttggatactatgattgcatggagcatgaaaaccaaacaccattccaatttattaatctactagaaaaatatgataaattgctactagatgatagaaatttccatagaatgtcacacttaccagtaatattgcaacaagagtatgctttgagatatttttcaaaatcaagatttttaagtaaagggaagaagagattgagcaggagtgatttctcagatagtcttatggaagatagacatagtccaacatcattaatgcaagtggtacgtaactgcatcagtatacacataaatgattgtgaatggaataaagcgtgtacgcttatagttgatgctagaaattatattagtattatgaactcatcgtatactgagcattatagtgtgtcacaaagatgtaagttgtttactaagtataaatttgggatcgtatcaagattggtgaaaccgaattacattttttccagccatgaatcatgcgcattaaacgtacataactgtaaatggtgtcagatcaacaaccattacaaagtgtgggaagattttagacttaggaaaatatataataatgtaatggattttatcagggcacttgtgaaatcgaatggaaatgttggacattgttcatcccaggaatcagtgtataagtatataccagatttatttttaatttgtaaaacggaaaaatggaacgaagctgtcgaaatgttatttaattatctagaaccagtggacataaatggaacggagtatgtattattagactatgaagtgaactgggaagtgaggggactagtcatgcaaaacatggatgggaaagtaccaagaattttgaatatgaatgatacaaagaagatactgagtgcgatgatatttgactggtttgatacaagatatatgagagaaacaccaatgacgacgtcaacaacaaaccaacttcgaacactgaacaaaaggaatgaactcatagatgagtacgacttagaactttcagatgttgagtaaatatggtcacaactacgccagcacaagaccgtctgcactagagtagcgcctaggcagcataaaatgtgacc

SEQ ID NO: 15 - DNA, 1059 bp, Artificial
  NSP2B gene segment cDNA
ggcttttaaagcgtctcagtcgccgtttgagccttgcggtgtagccatggctgagctagcttgcttttgttatcctcatttggagaacgatagctatagattcattccatttaacagtttagctataaaatgtatgttgacagcaaaagtggacaaaaaagatcaagataaattttataattcaataatttatggtattgcaccaccgccacaattcaaaaaacgttataacacgaatgacaattcaagaggaatgaattatgaaactccaatgtttaataaagtggcggtgttaatttgtgaagcgttgaattcaattaaagttactcaatctgatgttgcgagtgtactttcaaaagtagtttctgtaagacatctagagaatttggtacggagaagagagaatcatcaggacgtgcttttccattcaaaagagttgttgttgaaatcagtactaatagctattggtcactcaaaagaaattgaaacgactgccactgctgaaggaggggaagtagtttttcaaaatgcagcttttacaatgtggaaattgacatacctggagcatagcctaatgccaattttggatcaaaattttattgaatataaaataacaatgaacgaagataaaccaatttcagaatcacatgttaaagaactgattgctgagttgcggtggcaatacaacaaatttgcagtaattacacatggtaaaggtcactacagagttgtaaaatattcatcagttgcgaatcatgcagatagagtttacgctactttcaagagtaataataagaatgggaatatgatagagtttaatctacttgatcaaagaataatatggcagaactggtatgcgtttacatcttcaatgaaacaaggtaacactcttgaagtatgtaagaaactactgttccaaaagatgaagcgagaaagtaatccgtttaagggactgtcaactgatagaaagatggatgaggtttctcaaataggaatttaattcgttatcgatttgagaatgggcatgacaaagcaagaatagaaagcgcttatgtgacc

SEQ ID NO: 16 - DNA, 1074 bp, Artificial
  NSP3B gene segment cDNA
ggcttttaatgcttttcagtggttgatgctcaagatggagtctacacagcagatggctagttcgattattaacacttcttttgaagccgcagtcgttgctgccacttcaactcttgaactcatgggcattcaatatgattataatgaagtttatactagagttaagagcaaatttgattacgtaatggatgattcaggtgttaaaaacaatctgttgggtaaagcggcaactattgatcaggcactgaatggaaaatttggttcagcagcaagaaatagaaattggatggccgatactagaactacagatagactagatgaagatgtgaacaaacttagaatgatgttatcatctaaaggaattgatcaaaaaatgagagtacttaatgcatgtttcagtgtgaagagagctccaggtaaatcatcatcaataattaaatgtactagactaatgagagataagattgaacgtggtgaagtcgaagtggatgattcgtttgttgaagaaaaaatggaagttgacacaattgattggaaatctaggtatgaacaattggaaaaacgatttgaatcactgaaacaaagggtgaatgaaaaatatacaagttgggtgcaaaaagcaaaaaaggtaaatgaaaatatgtactctctccaaaacgttatatcacaacagcagagccagattgctgatttacaaaattactgtaataaattggaagttgatctacagaataaaattagttcacttgtgtcttcagttgaatggtacctgaaatcaatggaattgcctgatgaaattaagacagatattgaacaacagctaaattccattgatgtaatcaatccaattaatgctatagatgattttgaatcactgatcagaaatattatactcgactatgacagaatatttttaatgttcaaaggattaatgaggcaatgcaactatgaatatacgtatgaatagtcacataatataattaaattaccatcttcacatgaccctctatgagcacaatagttaaaagctaacactgtcaaaaacctaaatggctataggggcgttatgtgacc

SEQ ID NO: 17 - DNA, 751 bp, Artificial
  NSP4B gene segment cDNA
ggcttttaaaagttctgttccgagagagcgcgtgcggaaagatggaaaagcttaccgacctcaactatacattgagtgtaatcactctaatgaacagcacattgcacacgatacttgaggatccaggaatggcgtattttccctatatagcatctgtcctaacagttttgttcacgttgcacaaagcatctattccaacaatgaaaattgcattgaagacgtccaagtgttcatataaagtagtgaagtattgtattgtgacgattttcaatgcgttgttgaaattggcaggttataaagaacagattaccactaaagatgagatagaaaagcaaatggacagggtagtcaaagagatgagacgtcagctagaaatgattgataagttgactacacgtgaaattgagcaggtggaattactaaaacgcattcacgataagttgatgatacgagcagtagacgaaatagatatgacgaaggaaattaaccaaaagaacgtgaaaacgctagaagaatgggaaaatggaaaaaatccttatgaaccaaaagaagtgactgcagcaatgtaagaggttgagctgccgtcgactgtcttcggaagcgacggagttcttcacagtaagccccatcggacctgatggctgactgagaagccacagtcagtcatatcgcgtgtggcttaagccttaatcccgtttaaccaatccggtcagcaccggacgttaatggaaggaacggtcttaatgtgacc

SEQ ID NO: 18 - DNA, 667 bp, Artificial
  NSP5B gene segment cDNA
ggcttttaaagcgctacagtgatgtctctcagtattgacgtgacgagtcttccttctatttcttctagtatatacaaaaatgaatcatcttcaacaacgtcaactctttctggaaaatctattggtaggagtgaacaatacatttcaccagatgcagaagcattcagtaaatacatgctgtcaaagtctccagaagatattggaccatctgattctgcttcaaacgatccactcaccagcttttcgattagatcgaatgcagttaagacaaatgcagacgctggcgtgtctatggattcatcaacacaatcacggccatcaagcaatgttgggtgcgatcaagtggatttctcctttaataaaggaattaaaatgaacgcgaacctggattcatcaatatccatatcaactatttcgaaaaaggagaaatccaaaagcgaccataaaagtaggaaacactaccctaaaatagaagcagaatctgattcagatgactacgtactcgatgattctgatagtgatgatggtaaatgtaaaaactgtaaatataagaggaagtatttcgcactaagaatgagaatgaaacaagttgcaatgcaattgatcgaagatttgtaggtctaacctgagaggtcactagggagctccccactcccgttttgtgacc

SEQ ID NO: 19 - DNA, 3527 bp, Artificial
  pTK-VP1B expression cassette
taatacgactcactataggctattaaagctatacaatggggaagtataatctaatcttgtcagaatatttatcatttatatataactcacaatctgcagttcaaattccaatttattattcttccaatagtgaattagagaatagatgtattgaatttcattctaaatgcttagaaaactcaaagaatggactaccactaaaaaaactctttgttgaatatagcgatgttatagagaatgccacactgttgtcaatattatcgtactcttacgataaatataacgctgttgaaaggaaattagtaaaatatgcaaaaggtaagccgctagaagcagatttgacagtgaatgagttggattatgaaaataacaagataacatctgagcttttcccaacagcagaggaatatactgattcattgatggatccagcaattttaacttcattatcatcaaatttgaatgcagttatgttctggttggaaaaacatgaaaatgatgctgctgaaaaactcaaaatttacaaaaggagattggacttatttactatagtagcttcaacagtaaataaatatggtgtaccaaggcacaatgagaaatatagatatgaatatgaagtgatgaaagataagccgtactacttggtaacatgggcaaattcttcaattgaaatgctaatgtcagttttttctcatgaagattatttaattgcgagagaactgatagtactgtcatattctaatagatcgactctagcaaaactggtgtcatcaccaatgtcaattctggtagctttagtggatataaacggaacatttattacgaatgaagaattagagctagagttttcaaacaaatatgtacgagcaatagttcctgaccaaacatttgacgaattaaaacagatgcttgacaacatgagaaaagctgggttaactgacatacctaagatgatacaggactggttagccgattgctctattgaaaaatttccattgatggctaaaatatattcgtggtcatttcatgtcggattcaggaagcagaaaatgttggacgccgcgttagatcaattgaaaactgagtatacagaagatatagatgatgaaatgtatcgagaatatacaatgctaataagagatgaagttgtgaaaatgcttaaggaaccagtaaagcatgatgatcatttgttacaggattctgaattggctggtttactatcaatgtcatcagcgtcgaatggtgaatcaagacaactaaaatttggtagaaagacaattttttcgactaaaaagaatatgcatgtaatggatgacatggctaatggaaggtatacgccaggcataataccaccagtgaatgtcgataaaccgataccattaggaaggagagatgtaccaggaagacggactagaataatattcatcttaccatatgaatattttatagcacaacatgccgtagttgaaaaaatgctaatttatgcgaaacatactagagagtatgctgaattctactcacagtcaaatcagttattgtcttatggtgatgttacacgctttttatctaataactctatggtgctatatacagacgtatcccagtgggactcatctcaacacaatacgcagccatttaggaaagggataattatggggttggacatgctagctaatatgactaatgatgctagagtcatccagacactaaacttatataaacagacgcaaattaatctaatggattcatacgttcaaataccagatggtgatgttattaaaaagatacaatatggggctgtagcgtcaggagaaaagcagacgaaagcagcgaattcaatagcaaatttagcactgattaaaacagttttatcacgtatttctaacaaatattcattcgcgacgaagataataagagttgacggagatgacaattacgcagtattgcagttcaatacagaagtaactaaacaaatggttcaagatgtatcaaacgacgtgagagaaacgtatgcgcgaatgaatgctaaagtcaaagctttagtatctacagtgggaatagaaatagctaaaaggtatattgcaggtgggaaaatattctttagagctggaataaatttactgaataacgaaaagagaggacaaagtacacagtgggatcaagcagctgttctatattcgaactatattgtgaatagacttcgaggatttgaaactgacagagagttcattttgactaaaataatgcaaatgacatcagttgctattacaggatcactaagactctttccttctgaacgcgtgttaaccacgaactctacgtttaaagtgtttgactcggaggactttattatagagtatgggacaactgacgacgaagtatacatacaaagagcgttcatgtctttatctagtcagaagtcaggaatagctgatgagatagctgcatcatcaacgtttaagaattatgtatctagattatctgagcagctgttattttcaaagaataatatagtgtctaagggaatagcattgactgaaaaagcaaaattgaactcatacgcgccaatatcacttgagaaaagacgcgcgcaaatatcagctttgctgactatgctgcaaaaaccggttacttttaaatcaagtaagataacaataaatgatatacttagagatataaagccatttttcactgtaagcgaagcgcatttgccgatacaatatcaaaaatttatgccaactttaccagacaatgtacagtatataattcagtgtataggatccagaacatatcaaattgaagatgacggttcaaagtcagctatatctcgactaatatcaaagtactcagtttacaagccgtcaatcgaagagttatacaaagtaatttcactacatgagaatgaaatacaactatatttgatctcactaggcataccgaaaatagacgctgatacgtacgtcggatcgaaaatttattctcaagataaatacaggatattagagtcgtatgtatataatttattgtctattaattatggatgttatcagctattcgacttcaattcaccagatctagaaaagctgatcagaataccgtttaaaggaaagataccagctgtcacttttatattgcatttatacgctaagctggaagttataaatcatgccattaaaaatggctcatggataagtttattctgtaactacccaaaatcagaaatgataaaattatggaagaaaatgtggaacattacgtcactacgttcaccgtataccaatgcaaacttctttcaagattagagcgcttagatgtgaccgggtcggcatggcatctccacctcctcgcggtccgacctgggcatccgaaggaggacgtcgtccactcggatggctaagggagagctcaaaaaaaaggatccggctgctaacaaagcccgaaaggaagctgagttggctgctgccaccgctgagcaataactagcataaccccttggggcctctaaacgggtcttgaggggttttttg

SEQ ID NO: 20 - DNA, 2912 bp, Artificial
  pTK-VP2B expression cassette
taatacgactcactataggctattaaaggctcaatggcgtacaggaaacgtggagcgcgccgtgaggcgaatataaataataatgaccgaatgcaagagaaagatgacgagaagcaggatcaaaacaatagaatgcaattatctgacaaagtactttcaaagaaagaggaagtcgtaaccgacaatcaagaggaaattaagattgctgatgaagtgaagaaatcaacgaaagaagaatctaaacaattgcttgaagttttgaaaacaaaagaagagcaccaaaaagaaatacagtatgaaattttacaaaaaacgataccaacatttgaaccaaaagagtcaatattgaagaaattggaagatatcaaaccggaacaggcgaagaagcagactaagctatttagaatatttgaaccgagacagctgccaatttatagagcaaatggtgaaaaagagttgcgtaacagatggtattggaagttgaagaaggatactttaccagatggagattatgacgttagagagtattttctaaatttgtatgatcaggttcttactgaaatgccagattatttactattaaaagatatggcagttgaaaataaaaactcaagagatgctggtaaagttgtcgattctgaaacggcaagtatctgtgatgctatatttcaagatgaggaaacagaaggcgcagtgagaagattcattgcggagatgagacaacgcgtacaagctgacaggaacgttgtcaattacccatcaatattacatccaatagattacgctttcaatgagtattttttacaacatcaattagttgaaccattaaataatgatataatattcaattacattcctgaaaggataaggaatgacgttaactatatacttaatatggacagaaatctgccatcaacagctagatatataagacctaatttactacaagacagactgaatttgcacgataattttgaatccttgtgggatacgataacaacttcaaactatattctggcaagatcggtagtaccggatttaaaggaattagtttcaaccgaagcgcaaattcaaaaaatgtcgcaagatttgcaactagaagcattaacaatacagtcagaaacgcagtttttaacaggtataaactcacaagcggcaaatgactgtttcaaaactctgattgcagcaatgttaagtcaaagaaccatgtcgcttgatttcgtgactacaaattatatgtcattaatttcaggtatgtggttactaactgtagtgccaaatgacatgttcataagggaatcattggttgcatgccaactggctatagtgaatacaataatatatccagcgttcggaatgcaacgaatgcattatagaaacggagatccacagacaccatttcagatagcagaacagcagatacaaaatttccaggtagcgaattggctgcattttgtcaataacaatcaatttagacaagtagttattgatggtgtattgaatcaggtactgaatgacaatattagaaatggacatgtcattaatcagttgatggaggctttaatgcaactatcacgacaacagtttccaacaatgcctgttgattataagaggtcaatccagcgtggaatattattgctatcaaataggcttggtcaattagttgatttaactaggttattagcttacaactacgaaacactaatggcatgtgttacgatgaatatgcaacatgttcagactttgacaacagaaaaattacagttaacttcagtcacgtcgttgtgtatgcttattggtaatgcaaccgttatacccagcccgcagacattatttcactattataatgttaatgttaattttcattcaaattataatgaaagaattaatgatgcagtggccataataactgcagctaatagactaaatttatatcagaaaaagatgaaggcaatagttgaagattttttaaaaagattacacattttcgatgtagctagagttccagatgatcaaatgtatagattaagggatagactacgactattgccagtagaagtaagacgattggatatttttaatttgatactgatgaacatggatcagatagaacgtgcctcagacaagattgcgcagggtgttattattgcataccgcgatatgcaattggaaagagatgaaatgtatggctacgtgaatatagctaggaatttagatgggttccagcaaataaacctagaagaattgatgagaacgggcgattatgcacaaataactaacatgctcttgaataatcaaccagtagcgctagttggagctcttccatttgttacagactcgtcagtcatatcgttaatagcgaagcttgacgctacagtttttgcccagatagttaaattacggaaagttgataccttgaaaccaatattgtataaaataaattcagattcgaatgacttttatctagttgccaattatgattgggtgcctacttcaaccacaaaagtatataaacaagttccacagcaatttgatttcagaaattcgatgcatatgttaacgtcaaatcttactttcaccgtttactcagatctgcttgcattcgtatcggccgatacagtagaacctataaatgcagttgcatttgataatatgcgcatcatgaacgagttgtaaacgccaaccccactgtggagatatgaccgggtcggcatggcatctccacctcctcgcggtccgacctgggcatccgaaggaggacgtcgtccactcggatggctaagggagagctcaaaaaaaaggatccggctgctaacaaagcccgaaaggaagctgagttggctgctgccaccgctgagcaataactagcataaccccttggggcctctaaacgggtcttgaggggttttttg

SEQ ID NO: 21 - DNA, 2816 bp, Artificial
  pTK-VP3H expression cassette
taatacgactcactataggctattaaagcagtactagtagtgcgttttacctctgatggtgtaagcatgaaagtattagctttaagacacagtgtggctcaggtgtatgcagatactcaaacctatttacatgatgattcaaaagatgagtatgaaaatgcatttctcatttctaatctaactacacataatatattatacctgaattacaatcttaaaacattaaaaatattaaataaatcaggtatagcagcagttgaagtacaatctccagatgaattatttgcgttaataaggtgtaattttacgtacgattatgagaataacatagtttatttacatgattattcatattatactaacaatgaaataagaacagatcaacattggataactaaaactgatataattgactatctattacctggatggaagttaacgtatgtaggttataatggaaagaatacaagaggtcactataatttttcatttatatgtcaaaatgcagctacagatgatgatataataattgaatatatatactccaatgagttagactttcaaaattttctgttgagaaaaattaaagagagaatgaccacatctcttccaattgctagattatcaaatcgtgtgtttagagataaattatttccatctattgtaaacatacataaaaaagtgataaatgttgggccgaggaatgaatctatgttcacattcctaaattttccaactattaagcaattttcaaacggtgcgtatattgtgaagcataccattaaattgaagcaagagaaatggttgggtaaaagagtatcacaatttgatatcggacaatataaaaacatgttaaatgtggtcactactatttactattactataatttatactattcgaaacctataatatacatgcttggttcagctccatcttattggatttatgatattaaacagtattctgactttacatttgaaacatgggatccattagatactccgtattctacaacacatcataaagaattattttttgacaaggatgtcaataagcttaaagataattcagttttatatatagacataagaactgatagaggtaatatggattggaaagagtggagaaaaatagtagaacaacaaactgttagcaatctaaatattgcatataaatatctatcaacaggaaaagcaaaggtgtgttgtgttaaattaactgctatggacctagaattaccaataacagcaaaattacttcatcatccaactactgaagttagatcagaattttatgcaatattggatgtatgggatattattaccattaaaagatttataccaaaaggtgtattttatgcttttataaataacgtaaccacagagaatgtgtttatacaacctccttttaaattaaaaacgtcacctactgattatatagtggcattgtatgctttatccaatgacttcaattcaaggcaagatgttattaatttgattaataaacaaaaacaatcactcattactgttcgtataaataacgcttttaaagacgagccaaaagtaaattttaaaaatatttatgattggacgtttctgccaacagatttcgaacttaaagattcgataattacatcatatgatggttgtttaggcatattcggattatcaatatctttatcgtctaaacccaccggaaataatcatttatttataataaatggaactgacaaatatgataaactagaccaatatgcaaatcatatgggtatttctagaagatcgcatcaaattagattctcagagtctgcgacatcatattcgggatatatttttagagatctttcaaataataatttcaatctaataggtactaatgtggagaattcagtttcaggacatgtctataatgcattgatttactacagatataattatgcgtttgatcttaaaagatggatttatctacattcaattggaaaagtcgctgtagaaggtggaagatattatgaacatgcaccaatcgaattgatatatgcatgccgatcagctaaagaatttgctatattacaagatgacttaacggtattgagatacgctaatgaaattgaagggtatataaacaaagtatatagtataacctatgctgacgatcccaattactttataggaattaaatttaatagtataccttatgaatacgatgttaaaattccacatttgacactaggagtattatttatatctgataatatgatacatgatgtaatcatagtgctgaagaaaatgaagacagaactatttaaaatggaaattagtactagttatacttatatgctatctgataatatgtatgtagcaaatgctagtggtgtgttatcaacttattttaaattatataatatgttctatagaaatcatatcacgtttggacaatcacgaatgtttatcccacacattacgctcagttttagcaacaaacagacagttagaatagagagtacaaaactcggaatcaattcaatttacttaagaaagattaaaggtgaaaccgtatttgatatgtctgagtgagctagaaacttaacacactagtcatgatgtgaccgggtcggcatggcatctccacctcctcgcggtccgacctgggcatccgaaggaggacgtcgtccactcggatggctaagggagagctcaaaaaaaaggatccggctgctaacaaagcccgaaaggaagctgagttggctgctgccaccgctgagcaataactagcataaccccttggggcctctaaacgggtcttgaggggttttttg

SEQ ID NO: 22 - DNA, 2816 bp, Artificial
  pTK-VP3B expression cassette
taatacgactcactataggctattaaagcaatattagtagtgtgttttacctctgatggtgtaaacatgaaagtattagctttaagacatagtgtggctcaggtatatgcggacactcaaatatatactcatgatgaaaccaaagatgactacgagaacgcatttttaatttctaatctcactacacataatatattgtatctaaattatagcgttaagacattgcaaatattgaataaatctggtatagctgcggtagaaatacaggagatggatgaattgtttacgctaattagatgcaacttcacatatgattatattgacgacattgtttaccttcatgattattcatactatactaataatgagataaggactgatcaacattgggtaactaaaacaaatatagaagactatttattaccaggatggaaactgacgtatgttggatataacggaaatgacacaagagggcactataacttttcttttaaatgtcaaaatgcagctacggacgatgatgcaataatagaatatatttattcaaatgaattggacttccaaaatttcatacttaaaaaaatcaaagaaaggatgacgacatcactgccaatagcgagattatcgaatcgtgtgttcagagacaaattatttaagacgctagtatcagatcacagtagagtagttaacgttggaccaagaaatgaatctatgtttacttttctagatcacccgtcaataaagcaattttcaaatggaccctatttagttaaagatacgataaagcttaaacaagagagatggctcggtaagagactatcgcaatttgacattggtcagtataagaacatgctaaatgtattaacaactttataccaatactatgacatgtatcatgagaagccaataatttacatggtaggatcagcaccttcatattggatacacgatgtcaggcaatactctaatttaaagtttgagacatgggacccattggatacaccatactctgatttgcatcataaagaattgttttatataagtgacgtaaccaaacttaaagataattcgatattatatgtagatatacgaacggatagagaaaatacagattggaaagcgtggaggaagattgtggaagagcaaactataaataatttgaatatcgcatacaaatacttatccacaggaaaagctaaagtatgttgtgttaaaatgactgccatggatttagaactaccaatatctgcaaaactactacatcatccaactacagaaattaggtcagaattttatttaataatggatatatgggattctaaaaatattaaacgatttataccgaagggcgtgttatattcatatattaacaatgtaattactgagaacgtgttcatacaacaaccgtttaaattgaaaacgttaaggaatgaatatgtggttgcattatacgcactgtctaacgactttaataatagagaggatgtgataaaattggttaacaatcagaagaatgcgttaataactgtgaggataaataatacatttaaagatgaaccaaaagtggggtttaaagatatttatgactggacttttttgccaactgatttcgaaacgaatgagtcaataatcacgtcatatgatggttgtttaggtatgtttggcttatcaatatcattagcttcaaaaccaactggaaataatcatctgttcattttgagcggtactaataaatattttaaattggatcaatttgcgaatcatatgagtatatcaagacggtcacatcaaatacgattttcggaatcagcgacttcatattcaggttacatttttagagatttatcaaataataattttaatttaataggtacgaatgttgagaattcggtatctggacatgtgtacaatgcattgatttattatagatataattattcattcgatcttaagcgatggatatacttacatgcaacaaacaaggctggcattgaaggcggcagatactatgaacatgctccgatagagttgatttacgcatgtagatcggcaaaggaattcgcaaaattgcaagatgatttaacagtactaagatattcgaatgaaatagaagattacattaataaagtgtacagtataacatacgccgacgatccgaactactttattggaattaagttcaaaaatataccatatgaatatgatgttaaagtaccgcatcttacatttggtgtattaaatatttcagattccatggtgccggatgtagtagcaattttaaagaagtttaaaagtgaattgtttagaatggatgtaaccacaagttatacgtatatgttgtcagatgaaatctatgtggcaaacgtaagtggtgtgttatcaacatattttaaactttacaatgcattctataaagagcaaattacgtttggacaatcaagaatgtttattccgcacataacattaagtttcagtaacaagaaagtagtgagaatagatagtacgcgattgaacatagactttatatatttgaggaaaataaaaggcgatacagtgttcgatatgactgagtgagctaaaaacttaacacactggtcacgatgtgaccgggtcggcatggcatctccacctcctcgcggtccgacctgggcatccgaaggaggacgtcgtccactcggatggctaagggagagctcaaaaaaaaggatccggctgctaacaaagcccgaaaggaagctgagttggctgctgccaccgctgagcaataactagcataaccccttggggcctctaaacgggtcttgaggggttttttg

SEQ ID NO: 23 - DNA, 2587 bp, Artificial
  pTK-VP4B expression cassette
taatacgactcactataggctataaaatggcttcgctcatatacagacagctgctcgctaattcttacgcagtggatttgtctgatgagatacagtcagttggatcagagaagaaccagcgcgttacagtgaatccaggaccatttgcgcagacagtatatgcgccagtgaactggggacccggtgaagtgaatgactcgactgtagtacaacctgtgttggacggaccgtatcagccagcgtcgttcgatctaccagtaggaaattggatgttgttagcgccaacaggaccaggtgtggtagtggaagggacggacaattctggcagatggttatctgtaattctgattgaaccaggtgtcacatcagaaactaggacgtatacgatgtttggatcaagtaaacaggtgttagtgtcgaacgcgtctgatacgaaatggaaatttgttgaaatgatgaagacggcgattgatggtgactatgcggaatggggaacattactatcagacaccaaactctatgggatgatgaaatatggaaagagactattcatatacgaaggagaaaccccaaatgccacgaccaaaagatacattgtgacgaattatgcatcagttgaggtaaggccatatagtgacttttatataatttcaagatcacaggaatcagcatgcactgagtatataaacaacggactgccacccatccaaaataccaggaatgtagtgcctgtggcaatatcgtcaagatcaattgaaccaagaaaagtgcaggctaatgaagatattgtagtttctaagacgtcactatggaaagaaatgcaatataatagagatatcataattagatttaggtttgataactcaataataaaatctggaggtttgggctataagtgggctgaaatctcatttaaagctgcaaattatcaatacaattacatgagagacggagaagaagttacagcgcatacgacgtgctcagttaatggtgttaatgattttagctttaacggaggctcattaccaacagatttcgcaatatcgagatatgaagtaattaaagaaaattcgtatgtatacgttgattactgggacgattcacaggcattcagaaatgtggtctatgtgcgatcattggcagcgaatttgaatgacgtaatgtgttctggcggagattacagcttcgcgctacctgtcggacaatggccagtgatgaaagggggagcggtgacgttgcacacagcaggagtaacattatctacacaattcactgactacgtatcactgaactcactaaggtttagatttagactggcagtcgaagaaccatcattcacgataactagaacacgtgtatcaaaactgtatggtttaccagcggcgaacccaaacggcggaagggaatattatgaagtggcaggaaggttttcgctgatatcattggtgccatcaaatgatgactaccaaacgccaattatgaactcagtaacagtaagacaagacttggaaaggcgtttaaatgagttgagagaagagttcaataacttatcacaagagatagctgtgtcacagttaattgacttagctatgctgccactagacatgttttcgatgttctcgggaattgagggtactgtgaacgcagcaaaatcgatggctaccaacgtgatgaggaaattcaaaagttcaaaactcgcatcatcagtgtcaatgttgacggactctttgtccgatgcggcctcatctatcgcaaggagcacatcaatacgatcaataggatcgacggcatcagcttgggctaatatttcagaacaaacgcaagacgccgttaatgaagttgcgacgatatcatcacaagtgtcacaaataagtgggaaattaagattaaaagaaattacgactcaaacagaaggaatgaatttcgatgacatatcagcggcggtgctaaaagccaagatagatagatcaatacaggtcgaccaaaacgcattaccagacgtcatcacagaagcgtcagagaaattcatacgtaatagggcgtatagagtaatagacggagatgaagcatttgaggcgggcactgacggaagatttttcgcgtacaaggtggaaacgcttgaggaaatgccattcaatatagaaaaattcgcagatttagttaccaactcaccagtgatatcggcaataatagactttaagacattaaaaaacctgaatgacaattatgggataactagagagcaagcatttaatctgttacggtcaaaccccaaagttttgcgtggatttattgaccaaaacaatccaattataaaaaacagaatagaacaattaatcatgcaatgtagattgtgagcagcttctggaggatgtgaccgggtcggcatggcatctccacctcctcgcggtccgacctgggcatccgaaggaggacgtcgtccactcggatggctaagggagagctcaaaaaaaaggatccggctgctaacaaagcccgaaaggaagctgagttggctgctgccaccgctgagcaataactagcataaccccttggggcctctaaacgggtcttgaggggttttttg

SEQ ID NO: 24 - DNA, 2584 bp, Artificial
  pTK-VP4P1 expression cassette
taatacgactcactataggctataaaatggcttcgctcatttatagacaacttctcacaaattcatactcagtagatttacatgatgaaatagaacaaattgggtcagaaaaaactcaaaacgtaactgtaaatccaggtccgttcgcccaaaccaggtatgctccagtcaattggggttatggagagataaatgattcaaccacagtagaaccaattttagacggtccttatcagcctactacatttacaccacctattgattattggatacttattaactcaaatacaaatggagtagtatacgagagtacgaataatagtgacttttggactgcagtcgttgctattgaaccgcacgttaatccagtagatagacaatacactgtatttggtgaaaataaacaatttaatgtaagaaatgattcagataagtggaagtttttagaaatgtttagaagtagtagtcaaaatgaattttataatagacgtacactgacttctgatactaaacttgtgggaatattaaaatatggtggaagaatatggacgtttcatggtgaaacaccgagagctactactgatagttcaaatactgcaaatttaaacgatatatcaattataatacattcagaattttatattattccaaggtctcaagagtctaagtgtaatgaatatattaataatggtttaccaccaattcaaaatactagaaatgtagtaccattatcattatcatctagatccatacagtataagagagctcaagttaatgaagaaattacaatttcgaaaacctcattatggaaagaaatgcaatataatagtgatattataattagatttaaatttggtaatagtattgtaaaactgggaggattaggttataaatggtccgaaatatcatttaaggcagcaaactatcaatataattatttacgtgatggcgaacaagtaactgcacatactacttgctcagtaaatggagtaaataattttagctataacgggggatctttacctactgattttagcatctcaagatatgaagttatcaaagaaaattcttatgtatacgtagattattgggatgattcaaaagcatttagaaatatggtatatgtcagatcattagcagctaatttaaactcagtgaaatgtgcaggtggaaggtatcactttagtttacctgtaggtgcatggccagttatgaatggaggcgctgtttcgttacattttgctggagttacattatctacgcaattcacagatttcgtatcattgaattcattacgatttagatttagtttgacagtggatgaaccatctttttcaatattgagaacacgtacggtgaatttgtacgggttaccagcagctaatccaaataatggaaatgaatactacgaaatatcaggaagactttcgctcatttctttagttccaactaatgatgattatcagactccaattatgaattcagtaacagtaagacaagatttagaacgtcaacttactgatctacgagaggaatttaattcattatcacaagaaatagctatgtcacaattaattgacttagcgctattacctttagatatgttttctatgttttcaggaattaaaagtacaattgatctgactaaatcaatggcaactagtgtaatgaaaaaatttagaaaatcaaaattagctacatcaatttcggaaatgactaattcattatcagacgcagcatcatcagcatcaagaagcgtttctatcagatcgaatatatccacaatttcgaatttgactaacgtttcaaatgatgtatcaaatgtgactaattcgttgaatgatatttcaacacaaacgtctacaatcagtaagaaacttagattaagagaaatgattactcaaactgaaggaatgagttttgatgatatttcagcggcagtattaaaaacaaaaatagatatgtctactcaaattggaaagaataccttacccgacatagtcacagaggcatctgagaaatttattccaaaacgatcatatcgaatattaaaagatgacgaagtgatggaaattaatactgaagggaaagtctttgcatataaaatagatacacttaatgaagtaccatttgacgtaaataaatttgctgaacttgtaacaaattctccagttatatcagcaataattgattttaaaacattaaaaaacttgaatgataattatggaattactcggatagaagcactaaatttaattaaatcaaatccaaatgtattacgtaatttcattaaccaaaataatccaattataaggaacagaattgaacagctaattctacaatgtaagttgtgagaatgctattgaggatgtgaccgggtcggcatggcatctccacctcctcgcggtccgacctgggcatccgaaggaggacgtcgtccactcggatggctaagggagagctcaaaaaaaaggatccggctgctaacaaagcccgaaaggaagctgagttggctgctgccaccgctgagcaataactagcataaccccttggggcctctaaacgggtcttgaggggttttttg

SEQ ID NO: 25 - DNA, 1581 bp, Artificial
  pTK-VP6B expression cassette
taatacgactcactataggcttttaaacgaagtcttcaacatggatgtcctgtactccttgtcaaaaactcttaaagatgctagagacaaaattgtcgaaggcacattatactccaatgtaagtgatctaattcaacaatttaatcaaatgataattactatgaatggaaatgagttccaaactggaggaattggtaatctaccgattagaaattggaattttgattttggattacttggaacaactctattaaatctagatgctaactacgtcgaaacggcccgcaacacaattgattattttgtagattttgtagacaatgtatgtatggatgaaatggttagagaatcacaaagaaatggaattgcaccacaatcagattcacttagaaagttatcaggcattaaatttaaaagaataaattttgacaattcatcagaatacatagagaactggaatttgcaaaacagaagacaaagaacgggttttacatttcataaaccaaacattttcccttattcagcgtcattcacactgaacagatcacaaccagctcatgataacttgatgggtacgatgtggctcaatgcgggatcagaaattcaggtcgctggattcgactattcatgtgcaatcaatgcgccagccaatacacaacaatttgagcacgttgtacagctccgaagagtgttaactacagctacaataactcttttaccagatgcagaaagatttagttttccaagagtgattaattcagctgacggagcgactacatggtacttcaacccagtgattcttagaccaaataacgttgaagtagaatttctattaaacgggcagataataaatacttaccaagcaagatttggaacgatcatagctagaaattttgatacaatcagattgtcatttcagttgatgagaccaccaaatatgacaccagcggtagcggcgttatttccaaatgcacagccatttgaacatcacgcaacagtaggactcacgcttagaattgaatctgcagtttgtgaatcagtgcttgccgacgcaagtgaaacaatgctagcaaatgtgacatctgttagacaagaatacgcgataccagttggaccagtttttccaccaggtatgaattggactgatttgatcactaactattcaccatctagagaggataacttgcagcgtgtatttacagtggcttccattagaagcatgcttgtcaaatgaggaccaagctaaccacttggtatccgactttggtgagtatgtagctacgtcaagctgtttgaactctgtaagtaaggatacgtctacgtattcgctacacagagtaatcactcagatggcgtagtgagaggatgtgaccgggtcggcatggcatctccacctcctcgcggtccgacctgggcatccgaaggaggacgtcgtccactcggatggctaagggagagctcaaaaaaaaggatccggctgctaacaaagcccgaaaggaagctgagttggctgctgccaccgctgagcaataactagcataaccccttggggcctctaaacgggtcttgaggggttttttg

SEQ ID NO: 26 - DNA, 1287 bp, Artificial
  pTK-VP7G1 expression cassette
taatacgactcactataggctttaaaagagagaatttccgtctggctaacggttagctccttttaatgtatggtattgaatataccacaattctaatctttttgatatcaatcattctactcaactatatattaaaatcagtgactcgaataatggactacattatatatagatttttgttgattactgtagcattatttgctttgacaagagctcagaattatggacttaacttaccaataacaggatcaatggacgctgtatatactaactctactcaagaagaagtgtttctaacttctacgttatgtctgtattatccaactgaagcaagtactcaaatcaatgatggtgactggaaagacacattgtcgcaaatgtttcttacaaagggttggccaacaggatctgtttactttaaagagtactcaagtattgttgatttttctgttgacccacagctgtattgtgactataatttagtatttatgaaatatgaccaaagtcttgaattagatatgtcagagttggctgatttaatattgaatgaatggttatgtaacccaatggatgtaacgttatactattatcaacaatcgggagaatcaaataagtggatatcgatgggatcatcatgtaccgtgaaagtgtgtccgctaaatacacaaacgttaggaataggttgtcaaacaacaaacgtagactcatttgaaatgatcgctgagaatgagaaattagctatagtggatgtcgttgatgggataaatcataaaataaatttaacaactacgacatgtactattcgaaattgtaagaaattaggtccaagagaaaatgtagctgtaatacaagttggtggttctaatgtgttagacataacagcagatccaacaactaatccacaaactgagagaatgatgagagtgaattggaaaaagtggtggcaagtattttatactatagtagattatattaatcaaattgtacaggtaatgtccaaaagatcaagatcattaaattctgcatctttttattatagagtatagatatatcttagattagaattgttcgatgtgaccgggtcggcatggcatctccacctcctcgcggtccgacctgggcatccgaaggaggacgtcgtccactcggatggctaagggagagctcaaaaaaaaggatccggctgctaacaaagcccgaaaggaagctgagttggctgctgccaccgctgagcaataactagcataaccccttggggcctctaaacgggtcttgaggggttttttg

SEQ ID NO: 27 - DNA, 1287 bp, Artificial
  pTK-VP7G2 expression cassette
taatacgactcactataggctttaaaaacgagaatttccgtctggctagcggttagctctttttaatgtatggtattgaatataccacaattctgaccattttgatatctattatattattgaattatatattaaaaactataactaatacaatggactacataatctatagatttttactagtcattgttctgatatcaccatttgtaagaacacaaaattatggcatatatttaccaataacgggatcactagacgctgtatatacgaattcaactagtggagaaacatttctaacttcaacactatgcttatactatccagcagaagctaaaaatgagatttcagatgatgaatgggaaaatactctatcacaattatttttaactaaaggatggccaactggatcagtttattttaaagactacaatgacattactacattttccatgaatccacaactgtattgtgattataatgtagtattaatgagatatgataatacatctgaattagatgcatcggagttagcagatcttatattgaatgaatggctgtgcaatcctatggatatatcactttactattatcagcaaagtagcgaatcaaataaatggatctcaatgggaacggattgcacggtaaaagtttgtccacttaatacacaaacgttaggaattggatgcaaaactactgacgtgagtacatttgagatagttgcgtcgtctgaaaaattagtaattactgacgttgtaaatggtgttaatcataagataaatatttcaataagtacgtgcactatacgtaactgtaacaaattaggaccacgagaaaatgttgctataattcaagttggtggaccgaatgcattagatatcactgctgatccaacaacagttccacaaattcaaagaatcatgcgaataaattggaaaaaatggtggcaagtcttttatacagtagttgattacattaaccaaattgtacaagttatgtccaagcggtcaagatcattagacgcagctgctttttattatagagtttagatatagctttggtcagatttgtataatgtgaccgggtcggcatggcatctccacctcctcgcggtccgacctgggcatccgaaggaggacgtcgtccactcggatggctaagggagagctcaaaaaaaaggatccggctgctaacaaagcccgaaaggaagctgagttggctgctgccaccgctgagcaataactagcataaccccttggggcctctaaacgggtcttgaggggttttttg

SEQ ID NO: 28 - DNA, 1287 bp, Artificial
  pTK-VP7G3 expression cassette
taatacgactcactataggctttaaaagagagaatttccgtttggctagcggctagctccttttgatgtatggtattgaatataccacagttttaacctttttgatatcagttatattgttgaattacgtactcaaatcactaactagaataatggactttatcatttacagatttcttttaattatagttatactgtcaccactccttaatgcacaaaattatggaataaatcttccgattactggatcaatggacacatcatatacgaactcaacgcgagaggaagtattcctgacttcgactttatgtttgtattatccaactgaagcagcaacagaaataaatgataactcatggaaggatacactttcgcagctatttttaactaaaggatggccaacagaatctatttattttaaagattatactgatattgcctcgttttcagttgatccacaactgtactgtgattataatttggtattaatgaagtatgacgctacactgcaattggatatgtccgaactagcagatttgttacttaatgagtggttatgtaatcctatggacatcactttgtattattatcaacaaactgatgaagcaaataaatggatttcgatgggatcatcttgtaccataaaagtatgtccattaaatacgcaaacattaggaattgggtgtctaactactgatgcaaatactttcgaagaagttgcaacagctgaaaaattagtaattactgacgttgtagatggggtcaatcataaattgaaagtgacgacggatacttgtacaattagaaattgtaaaaaattaggaccaagggaaaacgtagcagttatacaggttggtggctcagatgtacttgacataacagctgatccaacgacagcaccacaaacagaaagaatgatgcgagtgaattggaagaaatggtggcaagtattttatacaatagttgactatgtgaatcaaattgtgcaagcgatgtccaaaagatcgagatcattaaattctgctgcattttattacagagtatagatatagcttaggttaaggctgtaagatgtgaccgggtcggcatggcatctccacctcctcgcggtccgacctgggcatccgaaggaggacgtcgtccactcggatggctaagggagagctcaaaaaaaaggatccggctgctaacaaagcccgaaaggaagctgagttggctgctgccaccgctgagcaataactagcataaccccttggggcctctaaacgggtcttgaggggttttttg

SEQ ID NO: 29 - DNA, 1287 bp, Artificial
  pTK-VP7G4 expression cassette
taatacgactcactataggctttaaaagagagaatttccgtttggctagcggatagctccttttaatgtatggtattgaatataccacagttctattttatttgatatcgttcgttcttgtgagttatattctgaaaactatgataaagataatggactatttaatttatagaataacatttgtaattgtagtattatcagtattatcgaatgcacaaaattatggaataaatttgccaattactggatctatggatacagcatatgctaactcaacacaagacaataattttttatcttcaactttatgtctatattatccatcagaagctccaactcaaattagtgacactgaatggaaagatacactatctcaactgtttttaaccaaaggatggccgacaggttcagtttattttaatgaatattcaaacgttttagaattttccatcgacccaaagctatactgtgattataatgttgtgttaattagattcgcttctggtgaggagttggacgtatctgaattagctgatctaatactcaatgagtggttatgtaatccaatggatataacattatattattatcaacaaactggagaggcaaataagtggatatcaatgggatcatcatgtaccgttaaagtgtgtccattaaatactcagacattaggaattggatgtcaaacgacagatactgctacttttgaaacagttgctgacagcgaaaaattggcattaattgatgttgttgacaacgtaaatcataaattagatgttacatctactacgtgtacaatacggaattgtaataaactaggacctagagaaaatgtggctataatacaggttggcggttctaatatattagatataacagctgatcccacaacttctccacaaacagaacgaatgatgcgcgtaaactggaaaaaatggtggcaagtattctatactgtagttgattacattaatcaaatagtaaaagtaatgtccaaaagatcaagatcgttagattcgtcatctttctattatagagtatagatatatcctaaaatagaactgtttgatgtgaccgggtcggcatggcatctccacctcctcgcggtccgacctgggcatccgaaggaggacgtcgtccactcggatggctaagggagagctcaaaaaaaaggatccggctgctaacaaagcccgaaaggaagctgagttggctgctgccaccgctgagcaataactagcataaccccttggggcctctaaacgggtcttgaggggttttttg

SEQ ID NO: 30 - DNA, 1286 bp, Artificial
  pTK-VP7G9 expression cassette
taatacgactcactataggctttaaaagagagaatttccgcttggctaacggttagctccttttaatgtatggtattgaatataccacagttctaacctttttgatatcaatcattttgttgaattatatactaaaatcattaactagtgcaatggactttataatttatagattccttttgcttatagtcattgtatcaccatttgttaagacgcaaaattatggaattaatttaccaatcactggctccatggatacggcatatgcaaactcatcacagctagatacatttttaacttcaacgttatgtttatattaccctgctgaagcatcaactcaaattggagatacagaatggaaagacactctgtctcaattgttcttgactaaagggtggccaactgggtcagtctattttaaagaatatactgacatcgcttcattttctattgatccacaactttattgcgattataatgttgtattaatgaagtacgattcaacattagagttagacatgtctgaactagctgatttgattctaaacgaatggttatgtaatccgatggatataacactatattattatcaacaaacagatgaagcgaataaatggatagcgatgggacaatcttgtacaataaaagtgtgtccgttgaatacgcagactttaggaataggctgtacaactacaaatacagcaacatttgaggaagtggccgcaagtgaaaaattagtgataactgatgttgttgatggtgtgaatcataaactagatgtaactacaactacttgtactattagaaattgtagaaaattaggaccaagagagaatgtggcaattatacaagttggcggctcagaagtgctagatattacagcagacccaaccactgcgccacaaactgaacgtatgatgcgaataaattggaaaaaatggtggcaagttttttatacggtagtagattatatcaatcagattgtgcaagttatgtccaaaagatcgcgatcgttgaattcagcagctttctactatagagtctgatatatctcaggttagaattggtcgatgtgaccgggtcggcatggcatctccacctcctcgcggtccgacctgggcatccgaaggaggacgtcgtccactcggatggctaagggagagctcaaaaaaaaggatccggctgctaacaaagcccgaaaggaagctgagttggctgctgccaccgctgagcaataactagcataaccccttggggcctctaaacgggtcttgaggggttttttg

SEQ ID NO: 31 - DNA, 1287 bp, Artificial
  pTK-VP7B expression cassette
taatacgactcactataggctttaaaagcgagaatttccgtttggctagcggttagctccttttaatgtatggtattgaatataccacaattctaatcttcttgacatcgattacattattgaattatatcttaaaatcaataacgagaataatggactatataatttatagatttttgtttatggtagtgatcttggccaccataataaatgcgcaaaactatggagtaaatttgccaattacaggttcaatggatactgcgtatgcaaactctacacaaagtgagccatttttgacatcaaccctttgtttgtattatcctgttgaggcatcaaacgaaatagctgatactgaatggaaagataccttatcacaactgttcttaacaaaaggatggccaacaggatcagtgtactttaaagaatatgctgatatagcggccttttcagtggaaccacagttatactgtgattataatttagttttaatgaaatatgactctacacaaaaactagatatgtctgaattggccgatcttatattgaatgaatggctgtgcaatccaatggacataacgctatattattatcagcagactgatgaggcaaataaatggatatcaatgggctcttcttgcacggttaaagtgtgtccattaaatacacaaacacttggtattggatgtctaataactaatccagacacgtttgaaacagttgcgacaacggagaaattagtgattacagatgttgtagatggtgtcaaccacaaattaaacgtcacaacggcaacgtgcaccatacgcaactgtaaaaagttaggaccaagggagaacgtagcagtcatacaggtaggcggcgcgaacattttagacatcacagctgatccaacaactacaccacagacagagagaatgatgcgaataaattggaaaaaatggtggcaagtgttttacacggtagtggattacgtcaatcaaataattcagacaatgtccaaaagatctagatcgcttaattcgtcggcgttctactatagagtgtaggtgcatgttagattagagttgtacgatgtgaccgggtcggcatggcatctccacctcctcgcggtccgacctgggcatccgaaggaggacgtcgtccactcggatggctaagggagagctcaaaaaaaaggatccggctgctaacaaagcccgaaaggaagctgagttggctgctgccaccgctgagcaataactagcataaccccttggggcctctaaacgggtcttgaggggttttttg

SEQ ID NO: 32 - DNA, 1803 bp, Artificial
  pTK-NSP1B expression cassette
taatacgactcactataggctttttttatgaaaagtcttgtgtgagccatggcgacttttaaagacgcttgttatcattataaaaagttgaataagttaaatagtttagtgctcaaactaggagcaaatgatgaatggaggccagcaccagtgacaaaatataaaggatggtgtttagattgttgtcaatatacaaatttgacatattgcagagggtgcgctctataccatgtatgtcagtggtgcagtcagtataacaggtgtttcttagatgaagaaccccatttgctgagaatgcgaacatttaaagatgtagtaacaaaggaagatatagaagggctgctaaccatgtatgaaacgttgtttccaataaatgaaaagttggtgaataaattcataaactctgtgaaacagcgtaagtgtaggaatgaatatttgttagaatggtataatcacttactaatgccaataacattacaagcattgactataaatcttgaggataatgtatattatatatttggatactatgattgcatggagcatgaaaaccaaacaccattccaatttattaatctactagaaaaatatgataaattgctactagatgatagaaatttccatagaatgtcacacttaccagtaatattgcaacaagagtatgctttgagatatttttcaaaatcaagatttttaagtaaagggaagaagagattgagcaggagtgatttctcagatagtcttatggaagatagacatagtccaacatcattaatgcaagtggtacgtaactgcatcagtatacacataaatgattgtgaatggaataaagcgtgtacgcttatagttgatgctagaaattatattagtattatgaactcatcgtatactgagcattatagtgtgtcacaaagatgtaagttgtttactaagtataaatttgggatcgtatcaagattggtgaaaccgaattacattttttccagccatgaatcatgcgcattaaacgtacataactgtaaatggtgtcagatcaacaaccattacaaagtgtgggaagattttagacttaggaaaatatataataatgtaatggattttatcagggcacttgtgaaatcgaatggaaatgttggacattgttcatcccaggaatcagtgtataagtatataccagatttatttttaatttgtaaaacggaaaaatggaacgaagctgtcgaaatgttatttaattatctagaaccagtggacataaatggaacggagtatgtattattagactatgaagtgaactgggaagtgaggggactagtcatgcaaaacatggatgggaaagtaccaagaattttgaatatgaatgatacaaagaagatactgagtgcgatgatatttgactggtttgatacaagatatatgagagaaacaccaatgacgacgtcaacaacaaaccaacttcgaacactgaacaaaaggaatgaactcatagatgagtacgacttagaactttcagatgttgagtaaatatggtcacaactacgccagcacaagaccgtctgcactagagtagcgcctaggcagcataaaatgtgaccgggtcggcatggcatctccacctcctcgcggtccgacctgggcatccgaaggaggacgtcgtccactcggatggctaagggagagctcaaaaaaaaggatccggctgctaacaaagcccgaaaggaagctgagttggctgctgccaccgctgagcaataactagcataaccccttggggcctctaaacgggtcttgaggggttttttg

SEQ ID NO: 33 - DNA, 1284 bp, Artificial
  pTK-NSP2B expression cassette
taatacgactcactataggcttttaaagcgtctcagtcgccgtttgagccttgcggtgtagccatggctgagctagcttgcttttgttatcctcatttggagaacgatagctatagattcattccatttaacagtttagctataaaatgtatgttgacagcaaaagtggacaaaaaagatcaagataaattttataattcaataatttatggtattgcaccaccgccacaattcaaaaaacgttataacacgaatgacaattcaagaggaatgaattatgaaactccaatgtttaataaagtggcggtgttaatttgtgaagcgttgaattcaattaaagttactcaatctgatgttgcgagtgtactttcaaaagtagtttctgtaagacatctagagaatttggtacggagaagagagaatcatcaggacgtgcttttccattcaaaagagttgttgttgaaatcagtactaatagctattggtcactcaaaagaaattgaaacgactgccactgctgaaggaggggaagtagtttttcaaaatgcagcttttacaatgtggaaattgacatacctggagcatagcctaatgccaattttggatcaaaattttattgaatataaaataacaatgaacgaagataaaccaatttcagaatcacatgttaaagaactgattgctgagttgcggtggcaatacaacaaatttgcagtaattacacatggtaaaggtcactacagagttgtaaaatattcatcagttgcgaatcatgcagatagagtttacgctactttcaagagtaataataagaatgggaatatgatagagtttaatctacttgatcaaagaataatatggcagaactggtatgcgtttacatcttcaatgaaacaaggtaacactcttgaagtatgtaagaaactactgttccaaaagatgaagcgagaaagtaatccgtttaagggactgtcaactgatagaaagatggatgaggtttctcaaataggaatttaattcgttatcgatttgagaatgggcatgacaaagcaagaatagaaagcgcttatgtgaccgggtcggcatggcatctccacctcctcgcggtccgacctgggcatccgaaggaggacgtcgtccactcggatggctaagggagagctcaaaaaaaaggatccggctgctaacaaagcccgaaaggaagctgagttggctgctgccaccgctgagcaataactagcataaccccttggggcctctaaacgggtcttgaggggttttttg

SEQ ID NO: 34 - DNA, 1299 bp, Artificial
  pTK-NSP3B expression cassette
taatacgactcactataggcttttaatgcttttcagtggttgatgctcaagatggagtctacacagcagatggctagttcgattattaacacttcttttgaagccgcagtcgttgctgccacttcaactcttgaactcatgggcattcaatatgattataatgaagtttatactagagttaagagcaaatttgattacgtaatggatgattcaggtgttaaaaacaatctgttgggtaaagcggcaactattgatcaggcactgaatggaaaatttggttcagcagcaagaaatagaaattggatggccgatactagaactacagatagactagatgaagatgtgaacaaacttagaatgatgttatcatctaaaggaattgatcaaaaaatgagagtacttaatgcatgtttcagtgtgaagagagctccaggtaaatcatcatcaataattaaatgtactagactaatgagagataagattgaacgtggtgaagtcgaagtggatgattcgtttgttgaagaaaaaatggaagttgacacaattgattggaaatctaggtatgaacaattggaaaaacgatttgaatcactgaaacaaagggtgaatgaaaaatatacaagttgggtgcaaaaagcaaaaaaggtaaatgaaaatatgtactctctccaaaacgttatatcacaacagcagagccagattgctgatttacaaaattactgtaataaattggaagttgatctacagaataaaattagttcacttgtgtcttcagttgaatggtacctgaaatcaatggaattgcctgatgaaattaagacagatattgaacaacagctaaattccattgatgtaatcaatccaattaatgctatagatgattttgaatcactgatcagaaatattatactcgactatgacagaatatttttaatgttcaaaggattaatgaggcaatgcaactatgaatatacgtatgaatagtcacataatataattaaattaccatcttcacatgaccctctatgagcacaatagttaaaagctaacactgtcaaaaacctaaatggctataggggcgttatgtgaccgggtcggcatggcatctccacctcctcgcggtccgacctgggcatccgaaggaggacgtcgtccactcggatggctaagggagagctcaaaaaaaaggatccggctgctaacaaagcccgaaaggaagctgagttggctgctgccaccgctgagcaataactagcataaccccttggggcctctaaacgggtcttgaggggttttttg

SEQ ID NO: 35 - DNA, 976 bp, Artificial
  pTK-NSP4B expression cassette
taatacgactcactataggcttttaaaagttctgttccgagagagcgcgtgcggaaagatggaaaagcttaccgacctcaactatacattgagtgtaatcactctaatgaacagcacattgcacacgatacttgaggatccaggaatggcgtattttccctatatagcatctgtcctaacagttttgttcacgttgcacaaagcatctattccaacaatgaaaattgcattgaagacgtccaagtgttcatataaagtagtgaagtattgtattgtgacgattttcaatgcgttgttgaaattggcaggttataaagaacagattaccactaaagatgagatagaaaagcaaatggacagggtagtcaaagagatgagacgtcagctagaaatgattgataagttgactacacgtgaaattgagcaggtggaattactaaaacgcattcacgataagttgatgatacgagcagtagacgaaatagatatgacgaaggaaattaaccaaaagaacgtgaaaacgctagaagaatgggaaaatggaaaaaatccttatgaaccaaaagaagtgactgcagcaatgtaagaggttgagctgccgtcgactgtcttcggaagcgacggagttcttcacagtaagccccatcggacctgatggctgactgagaagccacagtcagtcatatcgcgtgtggcttaagccttaatcccgtttaaccaatccggtcagcaccggacgttaatggaaggaacggtcttaatgtgaccgggtcggcatggcatctccacctcctcgcggtccgacctgggcatccgaaggaggacgtcgtccactcggatggctaagggagagctcaaaaaaaaggatccggctgctaacaaagcccgaaaggaagctgagttggctgctgccaccgctgagcaataactagcataaccccttggggcctctaaacgggtcttgaggggttttttg

SEQ ID NO: 36 - DNA, 892 bp, Artificial
  pTK-NSP5B expression cassette
taatacgactcactataggcttttaaagcgctacagtgatgtctctcagtattgacgtgacgagtcttccttctatttcttctagtatatacaaaaatgaatcatcttcaacaacgtcaactctttctggaaaatctattggtaggagtgaacaatacatttcaccagatgcagaagcattcagtaaatacatgctgtcaaagtctccagaagatattggaccatctgattctgcttcaaacgatccactcaccagcttttcgattagatcgaatgcagttaagacaaatgcagacgctggcgtgtctatggattcatcaacacaatcacggccatcaagcaatgttgggtgcgatcaagtggatttctcctttaataaaggaattaaaatgaacgcgaacctggattcatcaatatccatatcaactatttcgaaaaaggagaaatccaaaagcgaccataaaagtaggaaacactaccctaaaatagaagcagaatctgattcagatgactacgtactcgatgattctgatagtgatgatggtaaatgtaaaaactgtaaatataagaggaagtatttcgcactaagaatgagaatgaaacaagttgcaatgcaattgatcgaagatttgtaggtctaacctgagaggtcactagggagctccccactcccgttttgtgaccgggtcggcatggcatctccacctcctcgcggtccgacctgggcatccgaaggaggacgtcgtccactcggatggctaagggagagctcaaaaaaaaggatccggctgctaacaaagcccgaaaggaagctgagttggctgctgccaccgctgagcaataactagcataaccccttggggcctctaaacgggtcttgaggggttttttg

SEQ ID NO: 37 - DNA, 6203 bp, Artificial
  pTK-VP1B
tcgcgcgtttcggtgatgacggtgaaaacctctgacacatgcagctcccggagacggtcacagcttgtctgtaagcggatgccgggagcagacaagcccgtcagggcgcgtcagcgggtgttggcgggtgtcggggctggcttaactatgcggcatcagagcagattgtactgagagtgcaccatatgcggtgtgaaataccgcacagatgcgtaaggagaaaataccgcatcaggcgccattcgccattcaggctgcgcaactgttgggaagggcgatcggtgcgggcctcttcgctattacgccagctggcgaaagggggatgtgctgcaaggcgattaagttgggtaacgccagggttttcccagtcacgacgttgtaaaacgacggccagtgaattcgagctcggtacctaatacgactcactataggctattaaagctatacaatggggaagtataatctaatcttgtcagaatatttatcatttatatataactcacaatctgcagttcaaattccaatttattattcttccaatagtgaattagagaatagatgtattgaatttcattctaaatgcttagaaaactcaaagaatggactaccactaaaaaaactctttgttgaatatagcgatgttatagagaatgccacactgttgtcaatattatcgtactcttacgataaatataacgctgttgaaaggaaattagtaaaatatgcaaaaggtaagccgctagaagcagatttgacagtgaatgagttggattatgaaaataacaagataacatctgagcttttcccaacagcagaggaatatactgattcattgatggatccagcaattttaacttcattatcatcaaatttgaatgcagttatgttctggttggaaaaacatgaaaatgatgctgctgaaaaactcaaaatttacaaaaggagattggacttatttactatagtagcttcaacagtaaataaatatggtgtaccaaggcacaatgagaaatatagatatgaatatgaagtgatgaaagataagccgtactacttggtaacatgggcaaattcttcaattgaaatgctaatgtcagttttttctcatgaagattatttaattgcgagagaactgatagtactgtcatattctaatagatcgactctagcaaaactggtgtcatcaccaatgtcaattctggtagctttagtggatataaacggaacatttattacgaatgaagaattagagctagagttttcaaacaaatatgtacgagcaatagttcctgaccaaacatttgacgaattaaaacagatgcttgacaacatgagaaaagctgggttaactgacatacctaagatgatacaggactggttagccgattgctctattgaaaaatttccattgatggctaaaatatattcgtggtcatttcatgtcggattcaggaagcagaaaatgttggacgccgcgttagatcaattgaaaactgagtatacagaagatatagatgatgaaatgtatcgagaatatacaatgctaataagagatgaagttgtgaaaatgcttaaggaaccagtaaagcatgatgatcatttgttacaggattctgaattggctggtttactatcaatgtcatcagcgtcgaatggtgaatcaagacaactaaaatttggtagaaagacaattttttcgactaaaaagaatatgcatgtaatggatgacatggctaatggaaggtatacgccaggcataataccaccagtgaatgtcgataaaccgataccattaggaaggagagatgtaccaggaagacggactagaataatattcatcttaccatatgaatattttatagcacaacatgccgtagttgaaaaaatgctaatttatgcgaaacatactagagagtatgctgaattctactcacagtcaaatcagttattgtcttatggtgatgttacacgctttttatctaataactctatggtgctatatacagacgtatcccagtgggactcatctcaacacaatacgcagccatttaggaaagggataattatggggttggacatgctagctaatatgactaatgatgctagagtcatccagacactaaacttatataaacagacgcaaattaatctaatggattcatacgttcaaataccagatggtgatgttattaaaaagatacaatatggggctgtagcgtcaggagaaaagcagacgaaagcagcgaattcaatagcaaatttagcactgattaaaacagttttatcacgtatttctaacaaatattcattcgcgacgaagataataagagttgacggagatgacaattacgcagtattgcagttcaatacagaagtaactaaacaaatggttcaagatgtatcaaacgacgtgagagaaacgtatgcgcgaatgaatgctaaagtcaaagctttagtatctacagtgggaatagaaatagctaaaaggtatattgcaggtgggaaaatattctttagagctggaataaatttactgaataacgaaaagagaggacaaagtacacagtgggatcaagcagctgttctatattcgaactatattgtgaatagacttcgaggatttgaaactgacagagagttcattttgactaaaataatgcaaatgacatcagttgctattacaggatcactaagactctttccttctgaacgcgtgttaaccacgaactctacgtttaaagtgtttgactcggaggactttattatagagtatgggacaactgacgacgaagtatacatacaaagagcgttcatgtctttatctagtcagaagtcaggaatagctgatgagatagctgcatcatcaacgtttaagaattatgtatctagattatctgagcagctgttattttcaaagaataatatagtgtctaagggaatagcattgactgaaaaagcaaaattgaactcatacgcgccaatatcacttgagaaaagacgcgcgcaaatatcagctttgctgactatgctgcaaaaaccggttacttttaaatcaagtaagataacaataaatgatatacttagagatataaagccatttttcactgtaagcgaagcgcatttgccgatacaatatcaaaaatttatgccaactttaccagacaatgtacagtatataattcagtgtataggatccagaacatatcaaattgaagatgacggttcaaagtcagctatatctcgactaatatcaaagtactcagtttacaagccgtcaatcgaagagttatacaaagtaatttcactacatgagaatgaaatacaactatatttgatctcactaggcataccgaaaatagacgctgatacgtacgtcggatcgaaaatttattctcaagataaatacaggatattagagtcgtatgtatataatttattgtctattaattatggatgttatcagctattcgacttcaattcaccagatctagaaaagctgatcagaataccgtttaaaggaaagataccagctgtcacttttatattgcatttatacgctaagctggaagttataaatcatgccattaaaaatggctcatggataagtttattctgtaactacccaaaatcagaaatgataaaattatggaagaaaatgtggaacattacgtcactacgttcaccgtataccaatgcaaacttctttcaagattagagcgcttagatgtgaccgggtcggcatggcatctccacctcctcgcggtccgacctgggcatccgaaggaggacgtcgtccactcggatggctaagggagagctcaaaaaaaaggatccggctgctaacaaagcccgaaaggaagctgagttggctgctgccaccgctgagcaataactagcataaccccttggggcctctaaacgggtcttgaggggttttttggtcgactgcagaggcctgcatgcaagcttggcgtaatcatggtcatagctgtttcctgtgtgaaattgttatccgctcacaattccacacaacatacgagccggaagcataaagtgtaaagcctggggtgcctaatgagtgagctaactcacattaattgcgttgcgctcactgcccgctttccagtcgggaaacctgtcgtgccagctgcattaatgaatcggccaacgcgcggggagaggcggtttgcgtattgggcgctcttccgcttcctcgctcactgactcgctgcgctcggtcgttcggctgcggcgagcggtatcagctcactcaaaggcggtaatacggttatccacagaatcaggggataacgcaggaaagaacatgtgagcaaaaggccagcaaaaggccaggaaccgtaaaaaggccgcgttgctggcgtttttccataggctccgcccccctgacgagcatcacaaaaatcgacgctcaagtcagaggtggcgaaacccgacaggactataaagataccaggcgtttccccctggaagctccctcgtgcgctctcctgttccgaccctgccgcttaccggatacctgtccgcctttctcccttcgggaagcgtggcgctttctcatagctcacgctgtaggtatctcagttcggtgtaggtcgttcgctccaagctgggctgtgtgcacgaaccccccgttcagcccgaccgctgcgccttatccggtaactatcgtcttgagtccaacccggtaagacacgacttatcgccactggcagcagccactggtaacaggattagcagagcgaggtatgtaggcggtgctacagagttcttgaagtggtggcctaactacggctacactagaagaacagtatttggtatctgcgctctgctgaagccagttaccttcggaaaaagagttggtagctcttgatccggcaaacaaaccaccgctggtagcggtggtttttttgtttgcaagcagcagattacgcgcagaaaaaaaggatctcaagaagatcctttgatcttttctacggggtctgacgctcagtggaacgaaaactcacgttaagggattttggtcatgagattatcaaaaaggatcttcacctagatccttttaaattaaaaatgaagttttaaatcaatctaaagtatatatgagtaaacttggtctgacagttaccaatgcttaatcagtgaggcacctatctcagcgatctgtctatttcgttcatccatagttgcctgactccccgtcgtgtagataactacgatacgggagggcttaccatctggccccagtgctgcaatgataccgcgagacccacgctcaccggctccagatttatcagcaataaaccagccagccggaagggccgagcgcagaagtggtcctgcaactttatccgcctccatccagtctattaattgttgccgggaagctagagtaagtagttcgccagttaatagtttgcgcaacgttgttgccattgctacaggcatcgtggtgtcacgctcgtcgtttggtatggcttcattcagctccggttcccaacgatcaaggcgagttacatgatcccccatgttgtgcaaaaaagcggttagctccttcggtcctccgatcgttgtcagaagtaagttggccgcagtgttatcactcatggttatggcagcactgcataattctcttactgtcatgccatccgtaagatgcttttctgtgactggtgagtactcaaccaagtcattctgagaatagtgtatgcggcgaccgagttgctcttgcccggcgtcaatacgggataataccgcgccacatagcagaactttaaaagtgctcatcattggaaaacgttcttcggggcgaaaactctcaaggatcttaccgctgttgagatccagttcgatgtaacccactcgtgcacccaactgatcttcagcatcttttactttcaccagcgtttctgggtgagcaaaaacaggaaggcaaaatgccgcaaaaaagggaataagggcgacacggaaatgttgaatactcatactcttcctttttcaatattattgaagcatttatcagggttattgtctcatgagcggatacatatttgaatgtatttagaaaaataaacaaataggggttccgcgcacatttccccgaaaagtgccacctgacgtctaagaaaccattattatcatgacattaacctataaaaataggcgtatcacgaggccctttcgtc

SEQ ID NO: 38 - DNA, 5588 bp, Artificial
  pTK-VP2B
tcgcgcgtttcggtgatgacggtgaaaacctctgacacatgcagctcccggagacggtcacagcttgtctgtaagcggatgccgggagcagacaagcccgtcagggcgcgtcagcgggtgttggcgggtgtcggggctggcttaactatgcggcatcagagcagattgtactgagagtgcaccatatgcggtgtgaaataccgcacagatgcgtaaggagaaaataccgcatcaggcgccattcgccattcaggctgcgcaactgttgggaagggcgatcggtgcgggcctcttcgctattacgccagctggcgaaagggggatgtgctgcaaggcgattaagttgggtaacgccagggttttcccagtcacgacgttgtaaaacgacggccagtgaattcgagctcggtacctaatacgactcactataggctattaaaggctcaatggcgtacaggaaacgtggagcgcgccgtgaggcgaatataaataataatgaccgaatgcaagagaaagatgacgagaagcaggatcaaaacaatagaatgcaattatctgacaaagtactttcaaagaaagaggaagtcgtaaccgacaatcaagaggaaattaagattgctgatgaagtgaagaaatcaacgaaagaagaatctaaacaattgcttgaagttttgaaaacaaaagaagagcaccaaaaagaaatacagtatgaaattttacaaaaaacgataccaacatttgaaccaaaagagtcaatattgaagaaattggaagatatcaaaccggaacaggcgaagaagcagactaagctatttagaatatttgaaccgagacagctgccaatttatagagcaaatggtgaaaaagagttgcgtaacagatggtattggaagttgaagaaggatactttaccagatggagattatgacgttagagagtattttctaaatttgtatgatcaggttcttactgaaatgccagattatttactattaaaagatatggcagttgaaaataaaaactcaagagatgctggtaaagttgtcgattctgaaacggcaagtatctgtgatgctatatttcaagatgaggaaacagaaggcgcagtgagaagattcattgcggagatgagacaacgcgtacaagctgacaggaacgttgtcaattacccatcaatattacatccaatagattacgctttcaatgagtattttttacaacatcaattagttgaaccattaaataatgatataatattcaattacattcctgaaaggataaggaatgacgttaactatatacttaatatggacagaaatctgccatcaacagctagatatataagacctaatttactacaagacagactgaatttgcacgataattttgaatccttgtgggatacgataacaacttcaaactatattctggcaagatcggtagtaccggatttaaaggaattagtttcaaccgaagcgcaaattcaaaaaatgtcgcaagatttgcaactagaagcattaacaatacagtcagaaacgcagtttttaacaggtataaactcacaagcggcaaatgactgtttcaaaactctgattgcagcaatgttaagtcaaagaaccatgtcgcttgatttcgtgactacaaattatatgtcattaatttcaggtatgtggttactaactgtagtgccaaatgacatgttcataagggaatcattggttgcatgccaactggctatagtgaatacaataatatatccagcgttcggaatgcaacgaatgcattatagaaacggagatccacagacaccatttcagatagcagaacagcagatacaaaatttccaggtagcgaattggctgcattttgtcaataacaatcaatttagacaagtagttattgatggtgtattgaatcaggtactgaatgacaatattagaaatggacatgtcattaatcagttgatggaggctttaatgcaactatcacgacaacagtttccaacaatgcctgttgattataagaggtcaatccagcgtggaatattattgctatcaaataggcttggtcaattagttgatttaactaggttattagcttacaactacgaaacactaatggcatgtgttacgatgaatatgcaacatgttcagactttgacaacagaaaaattacagttaacttcagtcacgtcgttgtgtatgcttattggtaatgcaaccgttatacccagcccgcagacattatttcactattataatgttaatgttaattttcattcaaattataatgaaagaattaatgatgcagtggccataataactgcagctaatagactaaatttatatcagaaaaagatgaaggcaatagttgaagattttttaaaaagattacacattttcgatgtagctagagttccagatgatcaaatgtatagattaagggatagactacgactattgccagtagaagtaagacgattggatatttttaatttgatactgatgaacatggatcagatagaacgtgcctcagacaagattgcgcagggtgttattattgcataccgcgatatgcaattggaaagagatgaaatgtatggctacgtgaatatagctaggaatttagatgggttccagcaaataaacctagaagaattgatgagaacgggcgattatgcacaaataactaacatgctcttgaataatcaaccagtagcgctagttggagctcttccatttgttacagactcgtcagtcatatcgttaatagcgaagcttgacgctacagtttttgcccagatagttaaattacggaaagttgataccttgaaaccaatattgtataaaataaattcagattcgaatgacttttatctagttgccaattatgattgggtgcctacttcaaccacaaaagtatataaacaagttccacagcaatttgatttcagaaattcgatgcatatgttaacgtcaaatcttactttcaccgtttactcagatctgcttgcattcgtatcggccgatacagtagaacctataaatgcagttgcatttgataatatgcgcatcatgaacgagttgtaaacgccaaccccactgtggagatatgaccgggtcggcatggcatctccacctcctcgcggtccgacctgggcatccgaaggaggacgtcgtccactcggatggctaagggagagctcaaaaaaaaggatccggctgctaacaaagcccgaaaggaagctgagttggctgctgccaccgctgagcaataactagcataaccccttggggcctctaaacgggtcttgaggggttttttggtcgactgcagaggcctgcatgcaagcttggcgtaatcatggtcatagctgtttcctgtgtgaaattgttatccgctcacaattccacacaacatacgagccggaagcataaagtgtaaagcctggggtgcctaatgagtgagctaactcacattaattgcgttgcgctcactgcccgctttccagtcgggaaacctgtcgtgccagctgcattaatgaatcggccaacgcgcggggagaggcggtttgcgtattgggcgctcttccgcttcctcgctcactgactcgctgcgctcggtcgttcggctgcggcgagcggtatcagctcactcaaaggcggtaatacggttatccacagaatcaggggataacgcaggaaagaacatgtgagcaaaaggccagcaaaaggccaggaaccgtaaaaaggccgcgttgctggcgtttttccataggctccgcccccctgacgagcatcacaaaaatcgacgctcaagtcagaggtggcgaaacccgacaggactataaagataccaggcgtttccccctggaagctccctcgtgcgctctcctgttccgaccctgccgcttaccggatacctgtccgcctttctcccttcgggaagcgtggcgctttctcatagctcacgctgtaggtatctcagttcggtgtaggtcgttcgctccaagctgggctgtgtgcacgaaccccccgttcagcccgaccgctgcgccttatccggtaactatcgtcttgagtccaacccggtaagacacgacttatcgccactggcagcagccactggtaacaggattagcagagcgaggtatgtaggcggtgctacagagttcttgaagtggtggcctaactacggctacactagaagaacagtatttggtatctgcgctctgctgaagccagttaccttcggaaaaagagttggtagctcttgatccggcaaacaaaccaccgctggtagcggtggtttttttgtttgcaagcagcagattacgcgcagaaaaaaaggatctcaagaagatcctttgatcttttctacggggtctgacgctcagtggaacgaaaactcacgttaagggattttggtcatgagattatcaaaaaggatcttcacctagatccttttaaattaaaaatgaagttttaaatcaatctaaagtatatatgagtaaacttggtctgacagttaccaatgcttaatcagtgaggcacctatctcagcgatctgtctatttcgttcatccatagttgcctgactccccgtcgtgtagataactacgatacgggagggcttaccatctggccccagtgctgcaatgataccgcgagacccacgctcaccggctccagatttatcagcaataaaccagccagccggaagggccgagcgcagaagtggtcctgcaactttatccgcctccatccagtctattaattgttgccgggaagctagagtaagtagttcgccagttaatagtttgcgcaacgttgttgccattgctacaggcatcgtggtgtcacgctcgtcgtttggtatggcttcattcagctccggttcccaacgatcaaggcgagttacatgatcccccatgttgtgcaaaaaagcggttagctccttcggtcctccgatcgttgtcagaagtaagttggccgcagtgttatcactcatggttatggcagcactgcataattctcttactgtcatgccatccgtaagatgcttttctgtgactggtgagtactcaaccaagtcattctgagaatagtgtatgcggcgaccgagttgctcttgcccggcgtcaatacgggataataccgcgccacatagcagaactttaaaagtgctcatcattggaaaacgttcttcggggcgaaaactctcaaggatcttaccgctgttgagatccagttcgatgtaacccactcgtgcacccaactgatcttcagcatcttttactttcaccagcgtttctgggtgagcaaaaacaggaaggcaaaatgccgcaaaaaagggaataagggcgacacggaaatgttgaatactcatactcttcctttttcaatattattgaagcatttatcagggttattgtctcatgagcggatacatatttgaatgtatttagaaaaataaacaaataggggttccgcgcacatttccccgaaaagtgccacctgacgtctaagaaaccattattatcatgacattaacctataaaaataggcgtatcacgaggccctttcgtc

SEQ ID NO: 39 - DNA, 5492 bp, Artificial
  pTK-VP3H
tcgcgcgtttcggtgatgacggtgaaaacctctgacacatgcagctcccggagacggtcacagcttgtctgtaagcggatgccgggagcagacaagcccgtcagggcgcgtcagcgggtgttggcgggtgtcggggctggcttaactatgcggcatcagagcagattgtactgagagtgcaccatatgcggtgtgaaataccgcacagatgcgtaaggagaaaataccgcatcaggcgccattcgccattcaggctgcgcaactgttgggaagggcgatcggtgcgggcctcttcgctattacgccagctggcgaaagggggatgtgctgcaaggcgattaagttgggtaacgccagggttttcccagtcacgacgttgtaaaacgacggccagtgaattcgagctcggtacctaatacgactcactataggctattaaagcagtactagtagtgcgttttacctctgatggtgtaagcatgaaagtattagctttaagacacagtgtggctcaggtgtatgcagatactcaaacctatttacatgatgattcaaaagatgagtatgaaaatgcatttctcatttctaatctaactacacataatatattatacctgaattacaatcttaaaacattaaaaatattaaataaatcaggtatagcagcagttgaagtacaatctccagatgaattatttgcgttaataaggtgtaattttacgtacgattatgagaataacatagtttatttacatgattattcatattatactaacaatgaaataagaacagatcaacattggataactaaaactgatataattgactatctattacctggatggaagttaacgtatgtaggttataatggaaagaatacaagaggtcactataatttttcatttatatgtcaaaatgcagctacagatgatgatataataattgaatatatatactccaatgagttagactttcaaaattttctgttgagaaaaattaaagagagaatgaccacatctcttccaattgctagattatcaaatcgtgtgtttagagataaattatttccatctattgtaaacatacataaaaaagtgataaatgttgggccgaggaatgaatctatgttcacattcctaaattttccaactattaagcaattttcaaacggtgcgtatattgtgaagcataccattaaattgaagcaagagaaatggttgggtaaaagagtatcacaatttgatatcggacaatataaaaacatgttaaatgtggtcactactatttactattactataatttatactattcgaaacctataatatacatgcttggttcagctccatcttattggatttatgatattaaacagtattctgactttacatttgaaacatgggatccattagatactccgtattctacaacacatcataaagaattattttttgacaaggatgtcaataagcttaaagataattcagttttatatatagacataagaactgatagaggtaatatggattggaaagagtggagaaaaatagtagaacaacaaactgttagcaatctaaatattgcatataaatatctatcaacaggaaaagcaaaggtgtgttgtgttaaattaactgctatggacctagaattaccaataacagcaaaattacttcatcatccaactactgaagttagatcagaattttatgcaatattggatgtatgggatattattaccattaaaagatttataccaaaaggtgtattttatgcttttataaataacgtaaccacagagaatgtgtttatacaacctccttttaaattaaaaacgtcacctactgattatatagtggcattgtatgctttatccaatgacttcaattcaaggcaagatgttattaatttgattaataaacaaaaacaatcactcattactgttcgtataaataacgcttttaaagacgagccaaaagtaaattttaaaaatatttatgattggacgtttctgccaacagatttcgaacttaaagattcgataattacatcatatgatggttgtttaggcatattcggattatcaatatctttatcgtctaaacccaccggaaataatcatttatttataataaatggaactgacaaatatgataaactagaccaatatgcaaatcatatgggtatttctagaagatcgcatcaaattagattctcagagtctgcgacatcatattcgggatatatttttagagatctttcaaataataatttcaatctaataggtactaatgtggagaattcagtttcaggacatgtctataatgcattgatttactacagatataattatgcgtttgatcttaaaagatggatttatctacattcaattggaaaagtcgctgtagaaggtggaagatattatgaacatgcaccaatcgaattgatatatgcatgccgatcagctaaagaatttgctatattacaagatgacttaacggtattgagatacgctaatgaaattgaagggtatataaacaaagtatatagtataacctatgctgacgatcccaattactttataggaattaaatttaatagtataccttatgaatacgatgttaaaattccacatttgacactaggagtattatttatatctgataatatgatacatgatgtaatcatagtgctgaagaaaatgaagacagaactatttaaaatggaaattagtactagttatacttatatgctatctgataatatgtatgtagcaaatgctagtggtgtgttatcaacttattttaaattatataatatgttctatagaaatcatatcacgtttggacaatcacgaatgtttatcccacacattacgctcagttttagcaacaaacagacagttagaatagagagtacaaaactcggaatcaattcaatttacttaagaaagattaaaggtgaaaccgtatttgatatgtctgagtgagctagaaacttaacacactagtcatgatgtgaccgggtcggcatggcatctccacctcctcgcggtccgacctgggcatccgaaggaggacgtcgtccactcggatggctaagggagagctcaaaaaaaaggatccggctgctaacaaagcccgaaaggaagctgagttggctgctgccaccgctgagcaataactagcataaccccttggggcctctaaacgggtcttgaggggttttttggtcgactgcagaggcctgcatgcaagcttggcgtaatcatggtcatagctgtttcctgtgtgaaattgttatccgctcacaattccacacaacatacgagccggaagcataaagtgtaaagcctggggtgcctaatgagtgagctaactcacattaattgcgttgcgctcactgcccgctttccagtcgggaaacctgtcgtgccagctgcattaatgaatcggccaacgcgcggggagaggcggtttgcgtattgggcgctcttccgcttcctcgctcactgactcgctgcgctcggtcgttcggctgcggcgagcggtatcagctcactcaaaggcggtaatacggttatccacagaatcaggggataacgcaggaaagaacatgtgagcaaaaggccagcaaaaggccaggaaccgtaaaaaggccgcgttgctggcgtttttccataggctccgcccccctgacgagcatcacaaaaatcgacgctcaagtcagaggtggcgaaacccgacaggactataaagataccaggcgtttccccctggaagctccctcgtgcgctctcctgttccgaccctgccgcttaccggatacctgtccgcctttctcccttcgggaagcgtggcgctttctcatagctcacgctgtaggtatctcagttcggtgtaggtcgttcgctccaagctgggctgtgtgcacgaaccccccgttcagcccgaccgctgcgccttatccggtaactatcgtcttgagtccaacccggtaagacacgacttatcgccactggcagcagccactggtaacaggattagcagagcgaggtatgtaggcggtgctacagagttcttgaagtggtggcctaactacggctacactagaagaacagtatttggtatctgcgctctgctgaagccagttaccttcggaaaaagagttggtagctcttgatccggcaaacaaaccaccgctggtagcggtggtttttttgtttgcaagcagcagattacgcgcagaaaaaaaggatctcaagaagatcctttgatcttttctacggggtctgacgctcagtggaacgaaaactcacgttaagggattttggtcatgagattatcaaaaaggatcttcacctagatccttttaaattaaaaatgaagttttaaatcaatctaaagtatatatgagtaaacttggtctgacagttaccaatgcttaatcagtgaggcacctatctcagcgatctgtctatttcgttcatccatagttgcctgactccccgtcgtgtagataactacgatacgggagggcttaccatctggccccagtgctgcaatgataccgcgagacccacgctcaccggctccagatttatcagcaataaaccagccagccggaagggccgagcgcagaagtggtcctgcaactttatccgcctccatccagtctattaattgttgccgggaagctagagtaagtagttcgccagttaatagtttgcgcaacgttgttgccattgctacaggcatcgtggtgtcacgctcgtcgtttggtatggcttcattcagctccggttcccaacgatcaaggcgagttacatgatcccccatgttgtgcaaaaaagcggttagctccttcggtcctccgatcgttgtcagaagtaagttggccgcagtgttatcactcatggttatggcagcactgcataattctcttactgtcatgccatccgtaagatgcttttctgtgactggtgagtactcaaccaagtcattctgagaatagtgtatgcggcgaccgagttgctcttgcccggcgtcaatacgggataataccgcgccacatagcagaactttaaaagtgctcatcattggaaaacgttcttcggggcgaaaactctcaaggatcttaccgctgttgagatccagttcgatgtaacccactcgtgcacccaactgatcttcagcatcttttactttcaccagcgtttctgggtgagcaaaaacaggaaggcaaaatgccgcaaaaaagggaataagggcgacacggaaatgttgaatactcatactcttcctttttcaatattattgaagcatttatcagggttattgtctcatgagcggatacatatttgaatgtatttagaaaaataaacaaataggggttccgcgcacatttccccgaaaagtgccacctgacgtctaagaaaccattattatcatgacattaacctataaaaataggcgtatcacgaggccctttcgtc

SEQ ID NO: 40 - DNA, 5492 bp, Artificial
  pTK-VP3B
tcgcgcgtttcggtgatgacggtgaaaacctctgacacatgcagctcccggagacggtcacagcttgtctgtaagcggatgccgggagcagacaagcccgtcagggcgcgtcagcgggtgttggcgggtgtcggggctggcttaactatgcggcatcagagcagattgtactgagagtgcaccatatgcggtgtgaaataccgcacagatgcgtaaggagaaaataccgcatcaggcgccattcgccattcaggctgcgcaactgttgggaagggcgatcggtgcgggcctcttcgctattacgccagctggcgaaagggggatgtgctgcaaggcgattaagttgggtaacgccagggttttcccagtcacgacgttgtaaaacgacggccagtgaattcgagctcggtacctaatacgactcactataggctattaaagcaatattagtagtgtgttttacctctgatggtgtaaacatgaaagtattagctttaagacatagtgtggctcaggtatatgcggacactcaaatatatactcatgatgaaaccaaagatgactacgagaacgcatttttaatttctaatctcactacacataatatattgtatctaaattatagcgttaagacattgcaaatattgaataaatctggtatagctgcggtagaaatacaggagatggatgaattgtttacgctaattagatgcaacttcacatatgattatattgacgacattgtttaccttcatgattattcatactatactaataatgagataaggactgatcaacattgggtaactaaaacaaatatagaagactatttattaccaggatggaaactgacgtatgttggatataacggaaatgacacaagagggcactataacttttcttttaaatgtcaaaatgcagctacggacgatgatgcaataatagaatatatttattcaaatgaattggacttccaaaatttcatacttaaaaaaatcaaagaaaggatgacgacatcactgccaatagcgagattatcgaatcgtgtgttcagagacaaattatttaagacgctagtatcagatcacagtagagtagttaacgttggaccaagaaatgaatctatgtttacttttctagatcacccgtcaataaagcaattttcaaatggaccctatttagttaaagatacgataaagcttaaacaagagagatggctcggtaagagactatcgcaatttgacattggtcagtataagaacatgctaaatgtattaacaactttataccaatactatgacatgtatcatgagaagccaataatttacatggtaggatcagcaccttcatattggatacacgatgtcaggcaatactctaatttaaagtttgagacatgggacccattggatacaccatactctgatttgcatcataaagaattgttttatataagtgacgtaaccaaacttaaagataattcgatattatatgtagatatacgaacggatagagaaaatacagattggaaagcgtggaggaagattgtggaagagcaaactataaataatttgaatatcgcatacaaatacttatccacaggaaaagctaaagtatgttgtgttaaaatgactgccatggatttagaactaccaatatctgcaaaactactacatcatccaactacagaaattaggtcagaattttatttaataatggatatatgggattctaaaaatattaaacgatttataccgaagggcgtgttatattcatatattaacaatgtaattactgagaacgtgttcatacaacaaccgtttaaattgaaaacgttaaggaatgaatatgtggttgcattatacgcactgtctaacgactttaataatagagaggatgtgataaaattggttaacaatcagaagaatgcgttaataactgtgaggataaataatacatttaaagatgaaccaaaagtggggtttaaagatatttatgactggacttttttgccaactgatttcgaaacgaatgagtcaataatcacgtcatatgatggttgtttaggtatgtttggcttatcaatatcattagcttcaaaaccaactggaaataatcatctgttcattttgagcggtactaataaatattttaaattggatcaatttgcgaatcatatgagtatatcaagacggtcacatcaaatacgattttcggaatcagcgacttcatattcaggttacatttttagagatttatcaaataataattttaatttaataggtacgaatgttgagaattcggtatctggacatgtgtacaatgcattgatttattatagatataattattcattcgatcttaagcgatggatatacttacatgcaacaaacaaggctggcattgaaggcggcagatactatgaacatgctccgatagagttgatttacgcatgtagatcggcaaaggaattcgcaaaattgcaagatgatttaacagtactaagatattcgaatgaaatagaagattacattaataaagtgtacagtataacatacgccgacgatccgaactactttattggaattaagttcaaaaatataccatatgaatatgatgttaaagtaccgcatcttacatttggtgtattaaatatttcagattccatggtgccggatgtagtagcaattttaaagaagtttaaaagtgaattgtttagaatggatgtaaccacaagttatacgtatatgttgtcagatgaaatctatgtggcaaacgtaagtggtgtgttatcaacatattttaaactttacaatgcattctataaagagcaaattacgtttggacaatcaagaatgtttattccgcacataacattaagtttcagtaacaagaaagtagtgagaatagatagtacgcgattgaacatagactttatatatttgaggaaaataaaaggcgatacagtgttcgatatgactgagtgagctaaaaacttaacacactggtcacgatgtgaccgggtcggcatggcatctccacctcctcgcggtccgacctgggcatccgaaggaggacgtcgtccactcggatggctaagggagagctcaaaaaaaaggatccggctgctaacaaagcccgaaaggaagctgagttggctgctgccaccgctgagcaataactagcataaccccttggggcctctaaacgggtcttgaggggttttttggtcgactgcagaggcctgcatgcaagcttggcgtaatcatggtcatagctgtttcctgtgtgaaattgttatccgctcacaattccacacaacatacgagccggaagcataaagtgtaaagcctggggtgcctaatgagtgagctaactcacattaattgcgttgcgctcactgcccgctttccagtcgggaaacctgtcgtgccagctgcattaatgaatcggccaacgcgcggggagaggcggtttgcgtattgggcgctcttccgcttcctcgctcactgactcgctgcgctcggtcgttcggctgcggcgagcggtatcagctcactcaaaggcggtaatacggttatccacagaatcaggggataacgcaggaaagaacatgtgagcaaaaggccagcaaaaggccaggaaccgtaaaaaggccgcgttgctggcgtttttccataggctccgcccccctgacgagcatcacaaaaatcgacgctcaagtcagaggtggcgaaacccgacaggactataaagataccaggcgtttccccctggaagctccctcgtgcgctctcctgttccgaccctgccgcttaccggatacctgtccgcctttctcccttcgggaagcgtggcgctttctcatagctcacgctgtaggtatctcagttcggtgtaggtcgttcgctccaagctgggctgtgtgcacgaaccccccgttcagcccgaccgctgcgccttatccggtaactatcgtcttgagtccaacccggtaagacacgacttatcgccactggcagcagccactggtaacaggattagcagagcgaggtatgtaggcggtgctacagagttcttgaagtggtggcctaactacggctacactagaagaacagtatttggtatctgcgctctgctgaagccagttaccttcggaaaaagagttggtagctcttgatccggcaaacaaaccaccgctggtagcggtggtttttttgtttgcaagcagcagattacgcgcagaaaaaaaggatctcaagaagatcctttgatcttttctacggggtctgacgctcagtggaacgaaaactcacgttaagggattttggtcatgagattatcaaaaaggatcttcacctagatccttttaaattaaaaatgaagttttaaatcaatctaaagtatatatgagtaaacttggtctgacagttaccaatgcttaatcagtgaggcacctatctcagcgatctgtctatttcgttcatccatagttgcctgactccccgtcgtgtagataactacgatacgggagggcttaccatctggccccagtgctgcaatgataccgcgagacccacgctcaccggctccagatttatcagcaataaaccagccagccggaagggccgagcgcagaagtggtcctgcaactttatccgcctccatccagtctattaattgttgccgggaagctagagtaagtagttcgccagttaatagtttgcgcaacgttgttgccattgctacaggcatcgtggtgtcacgctcgtcgtttggtatggcttcattcagctccggttcccaacgatcaaggcgagttacatgatcccccatgttgtgcaaaaaagcggttagctccttcggtcctccgatcgttgtcagaagtaagttggccgcagtgttatcactcatggttatggcagcactgcataattctcttactgtcatgccatccgtaagatgcttttctgtgactggtgagtactcaaccaagtcattctgagaatagtgtatgcggcgaccgagttgctcttgcccggcgtcaatacgggataataccgcgccacatagcagaactttaaaagtgctcatcattggaaaacgttcttcggggcgaaaactctcaaggatcttaccgctgttgagatccagttcgatgtaacccactcgtgcacccaactgatcttcagcatcttttactttcaccagcgtttctgggtgagcaaaaacaggaaggcaaaatgccgcaaaaaagggaataagggcgacacggaaatgttgaatactcatactcttcctttttcaatattattgaagcatttatcagggttattgtctcatgagcggatacatatttgaatgtatttagaaaaataaacaaataggggttccgcgcacatttccccgaaaagtgccacctgacgtctaagaaaccattattatcatgacattaacctataaaaataggcgtatcacgaggccctttcgtc

SEQ ID NO: 41 - DNA, 5291 bp, Artificial
  pTK-VP4B
tcgcgcgtttcggtgatgacggtgaaaacctctgacacatgcagctcccggagacggtcacagcttgtctgtaagcggatgccgggagcagacaagcccgtcagggcgcgtcagcgggtgttggcgggtgtcggggctggcttaactatgcggcatcagagcagattgtactgagagtgcaccatatgcggtgtgaaataccgcacagatgcgtaaggagaaaataccgcatcaggcgccattcgccattcaggctgcgcaactgttgggaagggcgatcggtgcgggcctcttcgctattacgccagctggcgaaagggggatgtgctgcaaggcgattaagttgggtaacgccagggttttcccagtcacgacgttgtaaaacgacggccagtgaattctaatacgactcactataggctataaaatggcttcgctcatatacagacagctgctcgctaattcttacgcagtggatttgtctgatgagatacagtcagttggatcagagaagaaccagcgcgttacagtgaatccaggaccatttgcgcagacagtatatgcgccagtgaactggggacccggtgaagtgaatgactcgactgtagtacaacctgtgttggacggaccgtatcagccagcgtcgttcgatctaccagtaggaaattggatgttgttagcgccaacaggaccaggtgtggtagtggaagggacggacaattctggcagatggttatctgtaattctgattgaaccaggtgtcacatcagaaactaggacgtatacgatgtttggatcaagtaaacaggtgttagtgtcgaacgcgtctgatacgaaatggaaatttgttgaaatgatgaagacggcgattgatggtgactatgcggaatggggaacattactatcagacaccaaactctatgggatgatgaaatatggaaagagactattcatatacgaaggagaaaccccaaatgccacgaccaaaagatacattgtgacgaattatgcatcagttgaggtaaggccatatagtgacttttatataatttcaagatcacaggaatcagcatgcactgagtatataaacaacggactgccacccatccaaaataccaggaatgtagtgcctgtggcaatatcgtcaagatcaattgaaccaagaaaagtgcaggctaatgaagatattgtagtttctaagacgtcactatggaaagaaatgcaatataatagagatatcataattagatttaggtttgataactcaataataaaatctggaggtttgggctataagtgggctgaaatctcatttaaagctgcaaattatcaatacaattacatgagagacggagaagaagttacagcgcatacgacgtgctcagttaatggtgttaatgattttagctttaacggaggctcattaccaacagatttcgcaatatcgagatatgaagtaattaaagaaaattcgtatgtatacgttgattactgggacgattcacaggcattcagaaatgtggtctatgtgcgatcattggcagcgaatttgaatgacgtaatgtgttctggcggagattacagcttcgcgctacctgtcggacaatggccagtgatgaaagggggagcggtgacgttgcacacagcaggagtaacattatctacacaattcactgactacgtatcactgaactcactaaggtttagatttagactggcagtcgaagaaccatcattcacgataactagaacacgtgtatcaaaactgtatggtttaccagcggcgaacccaaacggcggaagggaatattatgaagtggcaggaaggttttcgctgatatcattggtgccatcaaatgatgactaccaaacgccaattatgaactcagtaacagtaagacaagacttggaaaggcgtttaaatgagttgagagaagagttcaataacttatcacaagagatagctgtgtcacagttaattgacttagctatgctgccactagacatgttttcgatgttctcgggaattgagggtactgtgaacgcagcaaaatcgatggctaccaacgtgatgaggaaattcaaaagttcaaaactcgcatcatcagtgtcaatgttgacggactctttgtccgatgcggcctcatctatcgcaaggagcacatcaatacgatcaataggatcgacggcatcagcttgggctaatatttcagaacaaacgcaagacgccgttaatgaagttgcgacgatatcatcacaagtgtcacaaataagtgggaaattaagattaaaagaaattacgactcaaacagaaggaatgaatttcgatgacatatcagcggcggtgctaaaagccaagatagatagatcaatacaggtcgaccaaaacgcattaccagacgtcatcacagaagcgtcagagaaattcatacgtaatagggcgtatagagtaatagacggagatgaagcatttgaggcgggcactgacggaagatttttcgcgtacaaggtggaaacgcttgaggaaatgccattcaatatagaaaaattcgcagatttagttaccaactcaccagtgatatcggcaataatagactttaagacattaaaaaacctgaatgacaattatgggataactagagagcaagcatttaatctgttacggtcaaaccccaaagttttgcgtggatttattgaccaaaacaatccaattataaaaaacagaatagaacaattaatcatgcaatgtagattgtgagcagcttctggaggatgtgaccgggtcggcatggcatctccacctcctcgcggtccgacctgggcatccgaaggaggacgtcgtccactcggatggctaagggagagctcaaaaaaaaggatccggctgctaacaaagcccgaaaggaagctgagttggctgctgccaccgctgagcaataactagcataaccccttggggcctctaaacgggtcttgaggggttttttgggtacctcgcgaatgcatctagatatcggatcccgggcccgtcgactgcagaggcctgcatgcaagcttggcgtaatcatggtcatagctgtttcctgtgtgaaattgttatccgctcacaattccacacaacatacgagccggaagcataaagtgtaaagcctggggtgcctaatgagtgagctaactcacattaattgcgttgcgctcactgcccgctttccagtcgggaaacctgtcgtgccagctgcattaatgaatcggccaacgcgcggggagaggcggtttgcgtattgggcgctcttccgcttcctcgctcactgactcgctgcgctcggtcgttcggctgcggcgagcggtatcagctcactcaaaggcggtaatacggttatccacagaatcaggggataacgcaggaaagaacatgtgagcaaaaggccagcaaaaggccaggaaccgtaaaaaggccgcgttgctggcgtttttccataggctccgcccccctgacgagcatcacaaaaatcgacgctcaagtcagaggtggcgaaacccgacaggactataaagataccaggcgtttccccctggaagctccctcgtgcgctctcctgttccgaccctgccgcttaccggatacctgtccgcctttctcccttcgggaagcgtggcgctttctcatagctcacgctgtaggtatctcagttcggtgtaggtcgttcgctccaagctgggctgtgtgcacgaaccccccgttcagcccgaccgctgcgccttatccggtaactatcgtcttgagtccaacccggtaagacacgacttatcgccactggcagcagccactggtaacaggattagcagagcgaggtatgtaggcggtgctacagagttcttgaagtggtggcctaactacggctacactagaagaacagtatttggtatctgcgctctgctgaagccagttaccttcggaaaaagagttggtagctcttgatccggcaaacaaaccaccgctggtagcggtggtttttttgtttgcaagcagcagattacgcgcagaaaaaaaggatctcaagaagatcctttgatcttttctacggggtctgacgctcagtggaacgaaaactcacgttaagggattttggtcatgagattatcaaaaaggatcttcacctagatccttttaaattaaaaatgaagttttaaatcaatctaaagtatatatgagtaaacttggtctgacagttaccaatgcttaatcagtgaggcacctatctcagcgatctgtctatttcgttcatccatagttgcctgactccccgtcgtgtagataactacgatacgggagggcttaccatctggccccagtgctgcaatgataccgcgagacccacgctcaccggctccagatttatcagcaataaaccagccagccggaagggccgagcgcagaagtggtcctgcaactttatccgcctccatccagtctattaattgttgccgggaagctagagtaagtagttcgccagttaatagtttgcgcaacgttgttgccattgctacaggcatcgtggtgtcacgctcgtcgtttggtatggcttcattcagctccggttcccaacgatcaaggcgagttacatgatcccccatgttgtgcaaaaaagcggttagctccttcggtcctccgatcgttgtcagaagtaagttggccgcagtgttatcactcatggttatggcagcactgcataattctcttactgtcatgccatccgtaagatgcttttctgtgactggtgagtactcaaccaagtcattctgagaatagtgtatgcggcgaccgagttgctcttgcccggcgtcaatacgggataataccgcgccacatagcagaactttaaaagtgctcatcattggaaaacgttcttcggggcgaaaactctcaaggatcttaccgctgttgagatccagttcgatgtaacccactcgtgcacccaactgatcttcagcatcttttactttcaccagcgtttctgggtgagcaaaaacaggaaggcaaaatgccgcaaaaaagggaataagggcgacacggaaatgttgaatactcatactcttcctttttcaatattattgaagcatttatcagggttattgtctcatgagcggatacatatttgaatgtatttagaaaaataaacaaataggggttccgcgcacatttccccgaaaagtgccacctgacgtctaagaaaccattattatcatgacattaacctataaaaataggcgtatcacgaggccctttcgtc

SEQ ID NO: 42 - DNA, 5260 bp, Artificial
  pTK-VP4P1
tcgcgcgtttcggtgatgacggtgaaaacctctgacacatgcagctcccggagacggtcacagcttgtctgtaagcggatgccgggagcagacaagcccgtcagggcgcgtcagcgggtgttggcgggtgtcggggctggcttaactatgcggcatcagagcagattgtactgagagtgcaccatatgcggtgtgaaataccgcacagatgcgtaaggagaaaataccgcatcaggcgccattcgccattcaggctgcgcaactgttgggaagggcgatcggtgcgggcctcttcgctattacgccagctggcgaaagggggatgtgctgcaaggcgattaagttgggtaacgccagggttttcccagtcacgacgttgtaaaacgacggccagtgaattcgagctcggtacctaatacgactcactataggctataaaatggcttcgctcatttatagacaacttctcacaaattcatactcagtagatttacatgatgaaatagaacaaattgggtcagaaaaaactcaaaacgtaactgtaaatccaggtccgttcgcccaaaccaggtatgctccagtcaattggggttatggagagataaatgattcaaccacagtagaaccaattttagacggtccttatcagcctactacatttacaccacctattgattattggatacttattaactcaaatacaaatggagtagtatacgagagtacgaataatagtgacttttggactgcagtcgttgctattgaaccgcacgttaatccagtagatagacaatacactgtatttggtgaaaataaacaatttaatgtaagaaatgattcagataagtggaagtttttagaaatgtttagaagtagtagtcaaaatgaattttataatagacgtacactgacttctgatactaaacttgtgggaatattaaaatatggtggaagaatatggacgtttcatggtgaaacaccgagagctactactgatagttcaaatactgcaaatttaaacgatatatcaattataatacattcagaattttatattattccaaggtctcaagagtctaagtgtaatgaatatattaataatggtttaccaccaattcaaaatactagaaatgtagtaccattatcattatcatctagatccatacagtataagagagctcaagttaatgaagaaattacaatttcgaaaacctcattatggaaagaaatgcaatataatagtgatattataattagatttaaatttggtaatagtattgtaaaactgggaggattaggttataaatggtccgaaatatcatttaaggcagcaaactatcaatataattatttacgtgatggcgaacaagtaactgcacatactacttgctcagtaaatggagtaaataattttagctataacgggggatctttacctactgattttagcatctcaagatatgaagttatcaaagaaaattcttatgtatacgtagattattgggatgattcaaaagcatttagaaatatggtatatgtcagatcattagcagctaatttaaactcagtgaaatgtgcaggtggaaggtatcactttagtttacctgtaggtgcatggccagttatgaatggaggcgctgtttcgttacattttgctggagttacattatctacgcaattcacagatttcgtatcattgaattcattacgatttagatttagtttgacagtggatgaaccatctttttcaatattgagaacacgtacggtgaatttgtacgggttaccagcagctaatccaaataatggaaatgaatactacgaaatatcaggaagactttcgctcatttctttagttccaactaatgatgattatcagactccaattatgaattcagtaacagtaagacaagatttagaacgtcaacttactgatctacgagaggaatttaattcattatcacaagaaatagctatgtcacaattaattgacttagcgctattacctttagatatgttttctatgttttcaggaattaaaagtacaattgatctgactaaatcaatggcaactagtgtaatgaaaaaatttagaaaatcaaaattagctacatcaatttcggaaatgactaattcattatcagacgcagcatcatcagcatcaagaagcgtttctatcagatcgaatatatccacaatttcgaatttgactaacgtttcaaatgatgtatcaaatgtgactaattcgttgaatgatatttcaacacaaacgtctacaatcagtaagaaacttagattaagagaaatgattactcaaactgaaggaatgagttttgatgatatttcagcggcagtattaaaaacaaaaatagatatgtctactcaaattggaaagaataccttacccgacatagtcacagaggcatctgagaaatttattccaaaacgatcatatcgaatattaaaagatgacgaagtgatggaaattaatactgaagggaaagtctttgcatataaaatagatacacttaatgaagtaccatttgacgtaaataaatttgctgaacttgtaacaaattctccagttatatcagcaataattgattttaaaacattaaaaaacttgaatgataattatggaattactcggatagaagcactaaatttaattaaatcaaatccaaatgtattacgtaatttcattaaccaaaataatccaattataaggaacagaattgaacagctaattctacaatgtaagttgtgagaatgctattgaggatgtgaccgggtcggcatggcatctccacctcctcgcggtccgacctgggcatccgaaggaggacgtcgtccactcggatggctaagggagagctcaaaaaaaaggatccggctgctaacaaagcccgaaaggaagctgagttggctgctgccaccgctgagcaataactagcataaccccttggggcctctaaacgggtcttgaggggttttttggtcgactgcagaggcctgcatgcaagcttggcgtaatcatggtcatagctgtttcctgtgtgaaattgttatccgctcacaattccacacaacatacgagccggaagcataaagtgtaaagcctggggtgcctaatgagtgagctaactcacattaattgcgttgcgctcactgcccgctttccagtcgggaaacctgtcgtgccagctgcattaatgaatcggccaacgcgcggggagaggcggtttgcgtattgggcgctcttccgcttcctcgctcactgactcgctgcgctcggtcgttcggctgcggcgagcggtatcagctcactcaaaggcggtaatacggttatccacagaatcaggggataacgcaggaaagaacatgtgagcaaaaggccagcaaaaggccaggaaccgtaaaaaggccgcgttgctggcgtttttccataggctccgcccccctgacgagcatcacaaaaatcgacgctcaagtcagaggtggcgaaacccgacaggactataaagataccaggcgtttccccctggaagctccctcgtgcgctctcctgttccgaccctgccgcttaccggatacctgtccgcctttctcccttcgggaagcgtggcgctttctcatagctcacgctgtaggtatctcagttcggtgtaggtcgttcgctccaagctgggctgtgtgcacgaaccccccgttcagcccgaccgctgcgccttatccggtaactatcgtcttgagtccaacccggtaagacacgacttatcgccactggcagcagccactggtaacaggattagcagagcgaggtatgtaggcggtgctacagagttcttgaagtggtggcctaactacggctacactagaagaacagtatttggtatctgcgctctgctgaagccagttaccttcggaaaaagagttggtagctcttgatccggcaaacaaaccaccgctggtagcggtggtttttttgtttgcaagcagcagattacgcgcagaaaaaaaggatctcaagaagatcctttgatcttttctacggggtctgacgctcagtggaacgaaaactcacgttaagggattttggtcatgagattatcaaaaaggatcttcacctagatccttttaaattaaaaatgaagttttaaatcaatctaaagtatatatgagtaaacttggtctgacagttaccaatgcttaatcagtgaggcacctatctcagcgatctgtctatttcgttcatccatagttgcctgactccccgtcgtgtagataactacgatacgggagggcttaccatctggccccagtgctgcaatgataccgcgagacccacgctcaccggctccagatttatcagcaataaaccagccagccggaagggccgagcgcagaagtggtcctgcaactttatccgcctccatccagtctattaattgttgccgggaagctagagtaagtagttcgccagttaatagtttgcgcaacgttgttgccattgctacaggcatcgtggtgtcacgctcgtcgtttggtatggcttcattcagctccggttcccaacgatcaaggcgagttacatgatcccccatgttgtgcaaaaaagcggttagctccttcggtcctccgatcgttgtcagaagtaagttggccgcagtgttatcactcatggttatggcagcactgcataattctcttactgtcatgccatccgtaagatgcttttctgtgactggtgagtactcaaccaagtcattctgagaatagtgtatgcggcgaccgagttgctcttgcccggcgtcaatacgggataataccgcgccacatagcagaactttaaaagtgctcatcattggaaaacgttcttcggggcgaaaactctcaaggatcttaccgctgttgagatccagttcgatgtaacccactcgtgcacccaactgatcttcagcatcttttactttcaccagcgtttctgggtgagcaaaaacaggaaggcaaaatgccgcaaaaaagggaataagggcgacacggaaatgttgaatactcatactcttcctttttcaatattattgaagcatttatcagggttattgtctcatgagcggatacatatttgaatgtatttagaaaaataaacaaataggggttccgcgcacatttccccgaaaagtgccacctgacgtctaagaaaccattattatcatgacattaacctataaaaataggcgtatcacgaggccctttcgtc

SEQ ID NO: 43 - DNA, 4257 bp, Artificial
  pTK-VP6B
tcgcgcgtttcggtgatgacggtgaaaacctctgacacatgcagctcccggagacggtcacagcttgtctgtaagcggatgccgggagcagacaagcccgtcagggcgcgtcagcgggtgttggcgggtgtcggggctggcttaactatgcggcatcagagcagattgtactgagagtgcaccatatgcggtgtgaaataccgcacagatgcgtaaggagaaaataccgcatcaggcgccattcgccattcaggctgcgcaactgttgggaagggcgatcggtgcgggcctcttcgctattacgccagctggcgaaagggggatgtgctgcaaggcgattaagttgggtaacgccagggttttcccagtcacgacgttgtaaaacgacggccagtgaattcgagctcggtacctaatacgactcactataggcttttaaacgaagtcttcaacatggatgtcctgtactccttgtcaaaaactcttaaagatgctagagacaaaattgtcgaaggcacattatactccaatgtaagtgatctaattcaacaatttaatcaaatgataattactatgaatggaaatgagttccaaactggaggaattggtaatctaccgattagaaattggaattttgattttggattacttggaacaactctattaaatctagatgctaactacgtcgaaacggcccgcaacacaattgattattttgtagattttgtagacaatgtatgtatggatgaaatggttagagaatcacaaagaaatggaattgcaccacaatcagattcacttagaaagttatcaggcattaaatttaaaagaataaattttgacaattcatcagaatacatagagaactggaatttgcaaaacagaagacaaagaacgggttttacatttcataaaccaaacattttcccttattcagcgtcattcacactgaacagatcacaaccagctcatgataacttgatgggtacgatgtggctcaatgcgggatcagaaattcaggtcgctggattcgactattcatgtgcaatcaatgcgccagccaatacacaacaatttgagcacgttgtacagctccgaagagtgttaactacagctacaataactcttttaccagatgcagaaagatttagttttccaagagtgattaattcagctgacggagcgactacatggtacttcaacccagtgattcttagaccaaataacgttgaagtagaatttctattaaacgggcagataataaatacttaccaagcaagatttggaacgatcatagctagaaattttgatacaatcagattgtcatttcagttgatgagaccaccaaatatgacaccagcggtagcggcgttatttccaaatgcacagccatttgaacatcacgcaacagtaggactcacgcttagaattgaatctgcagtttgtgaatcagtgcttgccgacgcaagtgaaacaatgctagcaaatgtgacatctgttagacaagaatacgcgataccagttggaccagtttttccaccaggtatgaattggactgatttgatcactaactattcaccatctagagaggataacttgcagcgtgtatttacagtggcttccattagaagcatgcttgtcaaatgaggaccaagctaaccacttggtatccgactttggtgagtatgtagctacgtcaagctgtttgaactctgtaagtaaggatacgtctacgtattcgctacacagagtaatcactcagatggcgtagtgagaggatgtgaccgggtcggcatggcatctccacctcctcgcggtccgacctgggcatccgaaggaggacgtcgtccactcggatggctaagggagagctcaaaaaaaaggatccggctgctaacaaagcccgaaaggaagctgagttggctgctgccaccgctgagcaataactagcataaccccttggggcctctaaacgggtcttgaggggttttttggtcgactgcagaggcctgcatgcaagcttggcgtaatcatggtcatagctgtttcctgtgtgaaattgttatccgctcacaattccacacaacatacgagccggaagcataaagtgtaaagcctggggtgcctaatgagtgagctaactcacattaattgcgttgcgctcactgcccgctttccagtcgggaaacctgtcgtgccagctgcattaatgaatcggccaacgcgcggggagaggcggtttgcgtattgggcgctcttccgcttcctcgctcactgactcgctgcgctcggtcgttcggctgcggcgagcggtatcagctcactcaaaggcggtaatacggttatccacagaatcaggggataacgcaggaaagaacatgtgagcaaaaggccagcaaaaggccaggaaccgtaaaaaggccgcgttgctggcgtttttccataggctccgcccccctgacgagcatcacaaaaatcgacgctcaagtcagaggtggcgaaacccgacaggactataaagataccaggcgtttccccctggaagctccctcgtgcgctctcctgttccgaccctgccgcttaccggatacctgtccgcctttctcccttcgggaagcgtggcgctttctcatagctcacgctgtaggtatctcagttcggtgtaggtcgttcgctccaagctgggctgtgtgcacgaaccccccgttcagcccgaccgctgcgccttatccggtaactatcgtcttgagtccaacccggtaagacacgacttatcgccactggcagcagccactggtaacaggattagcagagcgaggtatgtaggcggtgctacagagttcttgaagtggtggcctaactacggctacactagaagaacagtatttggtatctgcgctctgctgaagccagttaccttcggaaaaagagttggtagctcttgatccggcaaacaaaccaccgctggtagcggtggtttttttgtttgcaagcagcagattacgcgcagaaaaaaaggatctcaagaagatcctttgatcttttctacggggtctgacgctcagtggaacgaaaactcacgttaagggattttggtcatgagattatcaaaaaggatcttcacctagatccttttaaattaaaaatgaagttttaaatcaatctaaagtatatatgagtaaacttggtctgacagttaccaatgcttaatcagtgaggcacctatctcagcgatctgtctatttcgttcatccatagttgcctgactccccgtcgtgtagataactacgatacgggagggcttaccatctggccccagtgctgcaatgataccgcgagacccacgctcaccggctccagatttatcagcaataaaccagccagccggaagggccgagcgcagaagtggtcctgcaactttatccgcctccatccagtctattaattgttgccgggaagctagagtaagtagttcgccagttaatagtttgcgcaacgttgttgccattgctacaggcatcgtggtgtcacgctcgtcgtttggtatggcttcattcagctccggttcccaacgatcaaggcgagttacatgatcccccatgttgtgcaaaaaagcggttagctccttcggtcctccgatcgttgtcagaagtaagttggccgcagtgttatcactcatggttatggcagcactgcataattctcttactgtcatgccatccgtaagatgcttttctgtgactggtgagtactcaaccaagtcattctgagaatagtgtatgcggcgaccgagttgctcttgcccggcgtcaatacgggataataccgcgccacatagcagaactttaaaagtgctcatcattggaaaacgttcttcggggcgaaaactctcaaggatcttaccgctgttgagatccagttcgatgtaacccactcgtgcacccaactgatcttcagcatcttttactttcaccagcgtttctgggtgagcaaaaacaggaaggcaaaatgccgcaaaaaagggaataagggcgacacggaaatgttgaatactcatactcttcctttttcaatattattgaagcatttatcagggttattgtctcatgagcggatacatatttgaatgtatttagaaaaataaacaaataggggttccgcgcacatttccccgaaaagtgccacctgacgtctaagaaaccattattatcatgacattaacctataaaaataggcgtatcacgaggccctttcgtc

SEQ ID NO: 44 - DNA, 9352 bp, Artificial
  pTK-VP7G1
gcggccgcaaggggttcgcgtcagcgggtgttggcgggtgtcggggctggcttaactatgcggcatcagagcagattgtactgagagtgcaccatatgcggtgtgaaataccgcacagatgcgtaaggagaaaataccgcatcaggcgccattcgccattcagctgcgcaactgttgggaagggcgatcggtgcgggcctcttcgctattacgccagctggcgaaagggggatgtgctgcaaggcgattaagttgggtaacgccagggttttcccagtcacgacgttgtaaaacgacggccagtgaattggggcggtacctaatacgactcactataggctttaaaagagagaatttccgtctggctaacggttagctccttttaatgtatggtattgaatataccacaattctaatctttttgatatcaatcattctactcaactatatattaaaatcagtgactcgaataatggactacattatatatagatttttgttgattactgtagcattatttgctttgacaagagctcagaattatggacttaacttaccaataacaggatcaatggacgctgtatatactaactctactcaagaagaagtgtttctaacttctacgttatgtctgtattatccaactgaagcaagtactcaaatcaatgatggtgactggaaagacacattgtcgcaaatgtttcttacaaagggttggccaacaggatctgtttactttaaagagtactcaagtattgttgatttttctgttgacccacagctgtattgtgactataatttagtatttatgaaatatgaccaaagtcttgaattagatatgtcagagttggctgatttaatattgaatgaatggttatgtaacccaatggatgtaacgttatactattatcaacaatcgggagaatcaaataagtggatatcgatgggatcatcatgtaccgtgaaagtgtgtccgctaaatacacaaacgttaggaataggttgtcaaacaacaaacgtagactcatttgaaatgatcgctgagaatgagaaattagctatagtggatgtcgttgatgggataaatcataaaataaatttaacaactacgacatgtactattcgaaattgtaagaaattaggtccaagagaaaatgtagctgtaatacaagttggtggttctaatgtgttagacataacagcagatccaacaactaatccacaaactgagagaatgatgagagtgaattggaaaaagtggtggcaagtattttatactatagtagattatattaatcaaattgtacaggtaatgtccaaaagatcaagatcattaaattctgcatctttttattatagagtatagatatatcttagattagaattgttcgatgtgaccgggtcggcatggcatctccacctcctcgcggtccgacctgggcatccgaaggaggacgtcgtccactcggatggctaagggagagctcaaaaaaaaggatccggctgctaacaaagcccgaaaggaagctgagttggctgctgccaccgctgagcaataactagcataaccccttggggcctctaaacgggtcttgaggggttttttggtcgacgagtattctatagtctcacctaaatagcttggcgtaatcatggtcatagctgtttcctgtgtgaaattgttatccgctcacaattccacacaacatacgagccggaagcataaagtgtaaagcctggggtgcctaatgagtgagctaactcacattaattgcgttgcgctcactgcccgctttccagtcgggaaacctgtcgtgccagctgcattaatgaatcggccaacgcgaaccccttgcggccgcccgggccgtcgaccaattctcatgtttgacagcttatcatcgaatttctgccattcatccgcttattatcacttattcaggcgtagcaaccaggcgtttaagggcaccaataactgccttaaaaaaattacgccccgccctgccactcatcgcagtactgttgtaattcattaagcattctgccgacatggaagccatcacaaacggcatgatgaacctgaatcgccagcggcatcagcaccttgtcgccttgcgtataatatttgcccatggtgaaaacgggggcgaagaagttgtccatattggccacgtttaaatcaaaactggtgaaactcacccagggattggctgagacgaaaaacatattctcaataaaccctttagggaaataggccaggttttcaccgtaacacgccacatcttgcgaatatatgtgtagaaactgccggaaatcgtcgtggtattcactccagagcgatgaaaacgtttcagtttgctcatggaaaacggtgtaacaagggtgaacactatcccatatcaccagctcaccgtctttcattgccatacgaaattccggatgagcattcatcaggcgggcaagaatgtgaataaaggccggataaaacttgtgcttatttttctttacggtctttaaaaaggccgtaatatccagctgaacggtctggttataggtacattgagcaactgactgaaatgcctcaaaatgttctttacgatgccattgggatatatcaacggtggtatatccagtgatttttttctccattttagcttccttagctcctgaaaatctcgataactcaaaaaatacgcccggtagtgatcttatttcattatggtgaaagttggaacctcttacgtgccgatcaacgtctcattttcgccaaaagttggcccagggcttcccggtatcaacagggacaccaggatttatttattctgcgaagtgatcttccgtcacaggtatttattcgcgataagctcatggagcggcgtaaccgtcgcacaggaaggacagagaaagcgcggatctgggaagtgacggacagaacggtcaggacctggattggggaggcggttgccgccgctgctgctgacggtgtgacgttctctgttccggtcacaccacatacgttccgccattcctatgcgatgcacatgctgtatgccggtataccgctgaaagttctgcaaagcctgatgggacataagtccatcagttcaacggaagtctacacgaaggtttttgcgctggatgtggctgcccggcaccgggtgcagtttgcgatgccggagtctgatgcggttgcgatgctgaaacaattatcctgagaataaatgccttggcctttatatggaaatgtggaactgagtggatatgctgtttttgtctgttaaacagagaagctggctgttatccactgagaagcgaacgaaacagtcgggaaaatctcccattatcgtagagatccgcattattaatctcaggagcctgtgtagcgtttataggaagtagtgttctgtcatgatgcctgcaagcggtaacgaaaacgatttgaatatgccttcaggaacaatagaaatcttcgtgcggtgttacgttgaagtggagcggattatgtcagcaatggacagaacaacctaatgaacacagaaccatgatgtggtctgtccttttacagccagtagtgctcgccgcagtcgagcgacagggcgaagccctcggctggttgccctcgccgctgggctggcggccgtctatggccctgcaaacgcgccagaaacgccgtcgaagccgtgtgcgagacaccgcggccggccgccggcgttgtggatacctcgcggaaaacttggccctcactgacagatgaggggcggacgttgacacttgaggggccgactcacccggcgcggcgttgacagatgaggggcaggctcgatttcggccggcgacgtggagctggccagcctcgcaaatcggcgaaaacgcctgattttacgcgagtttcccacagatgatgtggacaagcctggggataagtgccctgcggtattgacacttgaggggcgcgactactgacagatgaggggcgcgatccttgacacttgaggggcagagtgctgacagatgaggggcgcacctattgacatttgaggggctgtccacaggcagaaaatccagcatttgcaagggtttccgcccgtttttcggccaccgctaacctgtcttttaacctgcttttaaaccaatatttataaaccttgtttttaaccagggctgcgccctgtgcgcgtgaccgcgcacgccgaaggggggtgcccccccttctcgaaccctcccggtcgagtgagcgaggaagcaccagggaacagcacttatatattctgcttacacacgatgcctgaaaaaacttcccttggggttatccacttatccacggggatatttttataattattttttttatagtttttagatcttcttttttagagcgccttgtaggcctttatccatgctggttctagagaaggtgttgtgacaaattgccctttcagtgtgacaaatcaccctcaaatgacagtcctgtctgtgacaaattgcccttaaccctgtgacaaattgccctcagaagaagctgttttttcacaaagttatccctgcttattgactcttttttatttagtgtgacaatctaaaaacttgtcacacttcacatggatctgtcatggcggaaacagcggttatcaatcacaagaaacgtaaaaatagcccgcgaatcgtccagtcaaacgacctcactgaggcggcatatagtctctcccgggatcaaaaacgtatgctgtatctgttcgttgaccagatcagaaaatctgatggcaccctacaggaacatgacggtatctgcgagatccatgttgctaaatatgctgaaatattcggattgacctctgcggaagccagtaaggatatacggcaggcattgaagagtttcgcggggaaggaagtggttttttatcgccctgaagaggatgccggcgatgaaaaaggctatgaatcttttccttggtttatcaaacgtgcgcacagtccatccagagggctttacagtgtacatatcaacccatatctcattcccttctttatcgggttacagaaccggtttacgcagtttcggcttagtgaaacaaaagaaatcaccaatccgtatgccatgcgtttatacgaatccctgtgtcagtatcgtaagccggatggctcaggcatcgtctctctgaaaatcgactggatcatagagcgttaccagctgcctcaaagttaccagcgtatgcctgacttccgccgccgcttcctgcaggtctgtgttaatgagatcaacagcagaactccaatgcgcctctcatacattgagaaaaagaaaggccgccagacgactcatatcgtattttccttccgcgatatcacttccatgacgacaggatagtctgagggttatctgtcacagatttgagggtggttcgtcacatttgttctgacctactgagggtaatttgtcacagttttgctgtttccttcagcctgcatggattttctcatactttttgaactgtaatttttaaggaagccaaatttgagggcagtttgtcacagttgatttccttctctttcccttcgtcatgtgacctgatatcgggggttagttcgtcatcattgatgagggttgattatcacagtttattactctgaattggctatccgcgtgtgtacctctacctggagtttttcccacggtggatatttcttcttgcgctgagcgtaagagctatctgacagaacagttcttctttgcttcctcgccagttcgctcgctatgctcggttacacggctgcggcgagcgctagtgataataagtgactgaggtatgtgctcttcttatctccttttgtagtgttgctcttattttaaacaactttgcggttttttgatgactttgcgattttgttgttgctttgcagtaaattgcaagatttaataaaaaaacgcaaagcaatgattaaaggatgttcagaatgaaactcatggaaacacttaaccagtgcataaacgctggtcatgaaatgacgaaggctatcgccattgcacagtttaatgatgacagcccggaagcgaggaaaataacccggcgctggagaataggtgaagcagcggatttagttggggtttcttctcaggctatcagagatgccgagaaagcagggcgactaccgcacccggatatggaaattcgaggacgggttgagcaacgtgttggttatacaattgaacaaattaatcatatgcgtgatgtgtttggtacgcgattgcgacgtgctgaagacgtatttccaccggtgatcggggttgctgcccataaaggtggcgtttacaaaacctcagtttctgttcatcttgctcaggatctggctctgaaggggctacgtgttttgctcgtggaaggtaacgacccccagggaacagcctcaatgtatcacggatgggtaccagatcttcatattcatgcagaagacactctcctgcctttctatcttggggaaaaggacgatgtcacttatgcaataaagcccacttgctggccggggcttgacattattccttcctgtctggctctgcaccgtattgaaactgagttaatgggcaaatttgatgaaggtaaactgcccaccgatccacacctgatgctccgactggccattgaaactgttgctcatgactatgatgtcatagttattgacagcgcgcctaacctgggtatcggcacgattaatgtcgtatgtgctgctgatgtgctgattgttcccacgcctgctgagttgtttgactacacctccgcactgcagtttttcgatatgcttcgtgatctgctcaagaacgttgatcttaaagggttcgagcctgatgtacgtattttgcttaccaaatacagcaatagtaatggctctcagtccccgtggatggaggagcaaattcgggatgcctggggaagcatggttctaaaaaatgttgtacgtgaaacggatgaagttggtaaaggtcagatccggatgagaactgtttttgaacaggccattgatcaacgctcttcaactggtgcctggagaaatgctctttctatttgggaacctgtctgcaatgaaattttcgatcgtctgattaaaccacgctgggagattagataatgaagcgtgcgcctgttattccaaaacatacgctcaatactcaaccggttgaagatacttcgttatcgacaccagctgccccgatggtggattcgttaattgcgcgcgtaggagtaatggctcgcggtaatgccattactttgcctgtatgtggtcgggatgtgaagtttactcttgaagtgctccggggtgatagtgttgagaagacctctcgggtatggtcaggtaatgaacgtgaccaggagctgcttactgaggacgcactggatgatctcatcccttcttttctactgactggtcaacagacaccggcgttcggtcgaagagtatctggtgtcatagaaattgccgatgggagtcgccgtcgtaaagctgctgcacttaccgaaagtgattatcgtgttctggttggcgagctggatgatgagcagatggctgcattatccagattgggtaacgattatcgcccaacaagtgcttatgaacgtggtcagcgttatgcaagccgattgcagaatgaatttgctggaaatatttctgcgctggctgatgcggaaaatatttcacgtaagattattacccgctgtatcaacaccgccaaattgcctaaatcagttgttgctcttttttctcaccccggtgaactatctgcccggtcaggtgatgcacttcaaaaagcctttacagataaagaggaattacttaagcagcaggcatctaaccttcatgagcagaaaaaagctggggtgatatttgaagctgaagaagttatcactcttttaacttctgtgcttaaaacgtcatctgcatcaagaactagtttaagctcacgacatcagtttgctcctggagcgacagtattgtataagggcgataaaatggtgcttaacctggacaggtctcgtgttccaactgagtgtatagagaaaattgaggccattcttaaggaacttgaaaagccagcaccctgatgcgaccacgttttagtctacgtttatctgtctttacttaatgtcctttgttacaggccagaaagcataactggcctgaatattctctctgggcccactgttccacttgtatcgtcggtctgataatcagactgggaccacggtcccactcgtatcgtcggtctgattattagtctgggaccacggtcccactcgtatcgtcggtctgattattagtctgggaccacggtcccactcgtatcgtcggtctgataatcagactgggaccacggtcccactcgtatcgtcggtctgattattagtctgggaccatggtcccactcgtatcgtcggtctgattattagtctgggaccacggtcccactcgtatcgtcggtctgattattagtctggaaccacggtcccactcgtatcgtcggtctgattattagtctgggaccacggtcccactcgtatcgtcggtctgattattagtctgggaccacgatcccactcgtgttgtcggtctgattatcggtctgggaccacggtcccacttgtattgtcgatcagactatcagcgtgagactacgattccatcaatgcctgtcaagggcaagtattgacatgtcgtcgtaacctgtagaacggagtaacctcggtgtgcggttgtatgcctgctgtggattgctgctgtgtcctgcttatccacaacattttgcgcacggttatgtggacaaaatacctggttacccaggccgtgccggcacgttaaccgggctgcatccgatgcaagtgtgtcgctgtcgacgagctcgcgagctcggacatgaggttgccccgtattcagtgtcgctgatttgtattgtctgaagttgtttttacgttaagttgatgcagatcaattaatacgatacctgcgtcataattgattatttgacgtggtttgatggcctccacgcacgttgtgatatgtagatgataatcattatcactttacgggtcctttccggtgatccgacaggttacggggcggcgacctcgcgggttttcgctatttatgaaaattttccggtttaaggcgtttccgttcttcttcgtcataacttaatgtttttatttaaaataccctctgaaaagaaaggaaacgacaggtgctgaaagcgagctttttggcctctgtcgtttcctttctctgtttttgtccgtggaatgaacaatggaagtccgagctcatcgctaataacttcgtatagcatacattatacgaagttatattcgat

SEQ ID NO: 45 - DNA, 3963 bp, Artificial
  pTK-VP7G2
tcgcgcgtttcggtgatgacggtgaaaacctctgacacatgcagctcccggagacggtcacagcttgtctgtaagcggatgccgggagcagacaagcccgtcagggcgcgtcagcgggtgttggcgggtgtcggggctggcttaactatgcggcatcagagcagattgtactgagagtgcaccatatgcggtgtgaaataccgcacagatgcgtaaggagaaaataccgcatcaggcgccattcgccattcaggctgcgcaactgttgggaagggcgatcggtgcgggcctcttcgctattacgccagctggcgaaagggggatgtgctgcaaggcgattaagttgggtaacgccagggttttcccagtcacgacgttgtaaaacgacggccagtgaattcgagctcggtacctaatacgactcactataggctttaaaaacgagaatttccgtctggctagcggttagctctttttaatgtatggtattgaatataccacaattctgaccattttgatatctattatattattgaattatatattaaaaactataactaatacaatggactacataatctatagatttttactagtcattgttctgatatcaccatttgtaagaacacaaaattatggcatatatttaccaataacgggatcactagacgctgtatatacgaattcaactagtggagaaacatttctaacttcaacactatgcttatactatccagcagaagctaaaaatgagatttcagatgatgaatgggaaaatactctatcacaattatttttaactaaaggatggccaactggatcagtttattttaaagactacaatgacattactacattttccatgaatccacaactgtattgtgattataatgtagtattaatgagatatgataatacatctgaattagatgcatcggagttagcagatcttatattgaatgaatggctgtgcaatcctatggatatatcactttactattatcagcaaagtagcgaatcaaataaatggatctcaatgggaacggattgcacggtaaaagtttgtccacttaatacacaaacgttaggaattggatgcaaaactactgacgtgagtacatttgagatagttgcgtcgtctgaaaaattagtaattactgacgttgtaaatggtgttaatcataagataaatatttcaataagtacgtgcactatacgtaactgtaacaaattaggaccacgagaaaatgttgctataattcaagttggtggaccgaatgcattagatatcactgctgatccaacaacagttccacaaattcaaagaatcatgcgaataaattggaaaaaatggtggcaagtcttttatacagtagttgattacattaaccaaattgtacaagttatgtccaagcggtcaagatcattagacgcagctgctttttattatagagtttagatatagctttggtcagatttgtataatgtgaccgggtcggcatggcatctccacctcctcgcggtccgacctgggcatccgaaggaggacgtcgtccactcggatggctaagggagagctcaaaaaaaaggatccggctgctaacaaagcccgaaaggaagctgagttggctgctgccaccgctgagcaataactagcataaccccttggggcctctaaacgggtcttgaggggttttttggtcgactgcagaggcctgcatgcaagcttggcgtaatcatggtcatagctgtttcctgtgtgaaattgttatccgctcacaattccacacaacatacgagccggaagcataaagtgtaaagcctggggtgcctaatgagtgagctaactcacattaattgcgttgcgctcactgcccgctttccagtcgggaaacctgtcgtgccagctgcattaatgaatcggccaacgcgcggggagaggcggtttgcgtattgggcgctcttccgcttcctcgctcactgactcgctgcgctcggtcgttcggctgcggcgagcggtatcagctcactcaaaggcggtaatacggttatccacagaatcaggggataacgcaggaaagaacatgtgagcaaaaggccagcaaaaggccaggaaccgtaaaaaggccgcgttgctggcgtttttccataggctccgcccccctgacgagcatcacaaaaatcgacgctcaagtcagaggtggcgaaacccgacaggactataaagataccaggcgtttccccctggaagctccctcgtgcgctctcctgttccgaccctgccgcttaccggatacctgtccgcctttctcccttcgggaagcgtggcgctttctcatagctcacgctgtaggtatctcagttcggtgtaggtcgttcgctccaagctgggctgtgtgcacgaaccccccgttcagcccgaccgctgcgccttatccggtaactatcgtcttgagtccaacccggtaagacacgacttatcgccactggcagcagccactggtaacaggattagcagagcgaggtatgtaggcggtgctacagagttcttgaagtggtggcctaactacggctacactagaagaacagtatttggtatctgcgctctgctgaagccagttaccttcggaaaaagagttggtagctcttgatccggcaaacaaaccaccgctggtagcggtggtttttttgtttgcaagcagcagattacgcgcagaaaaaaaggatctcaagaagatcctttgatcttttctacggggtctgacgctcagtggaacgaaaactcacgttaagggattttggtcatgagattatcaaaaaggatcttcacctagatccttttaaattaaaaatgaagttttaaatcaatctaaagtatatatgagtaaacttggtctgacagttaccaatgcttaatcagtgaggcacctatctcagcgatctgtctatttcgttcatccatagttgcctgactccccgtcgtgtagataactacgatacgggagggcttaccatctggccccagtgctgcaatgataccgcgagacccacgctcaccggctccagatttatcagcaataaaccagccagccggaagggccgagcgcagaagtggtcctgcaactttatccgcctccatccagtctattaattgttgccgggaagctagagtaagtagttcgccagttaatagtttgcgcaacgttgttgccattgctacaggcatcgtggtgtcacgctcgtcgtttggtatggcttcattcagctccggttcccaacgatcaaggcgagttacatgatcccccatgttgtgcaaaaaagcggttagctccttcggtcctccgatcgttgtcagaagtaagttggccgcagtgttatcactcatggttatggcagcactgcataattctcttactgtcatgccatccgtaagatgcttttctgtgactggtgagtactcaaccaagtcattctgagaatagtgtatgcggcgaccgagttgctcttgcccggcgtcaatacgggataataccgcgccacatagcagaactttaaaagtgctcatcattggaaaacgttcttcggggcgaaaactctcaaggatcttaccgctgttgagatccagttcgatgtaacccactcgtgcacccaactgatcttcagcatcttttactttcaccagcgtttctgggtgagcaaaaacaggaaggcaaaatgccgcaaaaaagggaataagggcgacacggaaatgttgaatactcatactcttcctttttcaatattattgaagcatttatcagggttattgtctcatgagcggatacatatttgaatgtatttagaaaaataaacaaataggggttccgcgcacatttccccgaaaagtgccacctgacgtctaagaaaccattattatcatgacattaacctataaaaataggcgtatcacgaggccctttcgtc

SEQ ID NO: 46 - DNA, 3963 bp, Artificial
  pTK-VP7G3
tcgcgcgtttcggtgatgacggtgaaaacctctgacacatgcagctcccggagacggtcacagcttgtctgtaagcggatgccgggagcagacaagcccgtcagggcgcgtcagcgggtgttggcgggtgtcggggctggcttaactatgcggcatcagagcagattgtactgagagtgcaccatatgcggtgtgaaataccgcacagatgcgtaaggagaaaataccgcatcaggcgccattcgccattcaggctgcgcaactgttgggaagggcgatcggtgcgggcctcttcgctattacgccagctggcgaaagggggatgtgctgcaaggcgattaagttgggtaacgccagggttttcccagtcacgacgttgtaaaacgacggccagtgaattcgagctcggtacctaatacgactcactataggctttaaaagagagaatttccgtttggctagcggctagctccttttgatgtatggtattgaatataccacagttttaacctttttgatatcagttatattgttgaattacgtactcaaatcactaactagaataatggactttatcatttacagatttcttttaattatagttatactgtcaccactccttaatgcacaaaattatggaataaatcttccgattactggatcaatggacacatcatatacgaactcaacgcgagaggaagtattcctgacttcgactttatgtttgtattatccaactgaagcagcaacagaaataaatgataactcatggaaggatacactttcgcagctatttttaactaaaggatggccaacagaatctatttattttaaagattatactgatattgcctcgttttcagttgatccacaactgtactgtgattataatttggtattaatgaagtatgacgctacactgcaattggatatgtccgaactagcagatttgttacttaatgagtggttatgtaatcctatggacatcactttgtattattatcaacaaactgatgaagcaaataaatggatttcgatgggatcatcttgtaccataaaagtatgtccattaaatacgcaaacattaggaattgggtgtctaactactgatgcaaatactttcgaagaagttgcaacagctgaaaaattagtaattactgacgttgtagatggggtcaatcataaattgaaagtgacgacggatacttgtacaattagaaattgtaaaaaattaggaccaagggaaaacgtagcagttatacaggttggtggctcagatgtacttgacataacagctgatccaacgacagcaccacaaacagaaagaatgatgcgagtgaattggaagaaatggtggcaagtattttatacaatagttgactatgtgaatcaaattgtgcaagcgatgtccaaaagatcgagatcattaaattctgctgcattttattacagagtatagatatagcttaggttaaggctgtaagatgtgaccgggtcggcatggcatctccacctcctcgcggtccgacctgggcatccgaaggaggacgtcgtccactcggatggctaagggagagctcaaaaaaaaggatccggctgctaacaaagcccgaaaggaagctgagttggctgctgccaccgctgagcaataactagcataaccccttggggcctctaaacgggtcttgaggggttttttggtcgactgcagaggcctgcatgcaagcttggcgtaatcatggtcatagctgtttcctgtgtgaaattgttatccgctcacaattccacacaacatacgagccggaagcataaagtgtaaagcctggggtgcctaatgagtgagctaactcacattaattgcgttgcgctcactgcccgctttccagtcgggaaacctgtcgtgccagctgcattaatgaatcggccaacgcgcggggagaggcggtttgcgtattgggcgctcttccgcttcctcgctcactgactcgctgcgctcggtcgttcggctgcggcgagcggtatcagctcactcaaaggcggtaatacggttatccacagaatcaggggataacgcaggaaagaacatgtgagcaaaaggccagcaaaaggccaggaaccgtaaaaaggccgcgttgctggcgtttttccataggctccgcccccctgacgagcatcacaaaaatcgacgctcaagtcagaggtggcgaaacccgacaggactataaagataccaggcgtttccccctggaagctccctcgtgcgctctcctgttccgaccctgccgcttaccggatacctgtccgcctttctcccttcgggaagcgtggcgctttctcatagctcacgctgtaggtatctcagttcggtgtaggtcgttcgctccaagctgggctgtgtgcacgaaccccccgttcagcccgaccgctgcgccttatccggtaactatcgtcttgagtccaacccggtaagacacgacttatcgccactggcagcagccactggtaacaggattagcagagcgaggtatgtaggcggtgctacagagttcttgaagtggtggcctaactacggctacactagaagaacagtatttggtatctgcgctctgctgaagccagttaccttcggaaaaagagttggtagctcttgatccggcaaacaaaccaccgctggtagcggtggtttttttgtttgcaagcagcagattacgcgcagaaaaaaaggatctcaagaagatcctttgatcttttctacggggtctgacgctcagtggaacgaaaactcacgttaagggattttggtcatgagattatcaaaaaggatcttcacctagatccttttaaattaaaaatgaagttttaaatcaatctaaagtatatatgagtaaacttggtctgacagttaccaatgcttaatcagtgaggcacctatctcagcgatctgtctatttcgttcatccatagttgcctgactccccgtcgtgtagataactacgatacgggagggcttaccatctggccccagtgctgcaatgataccgcgagacccacgctcaccggctccagatttatcagcaataaaccagccagccggaagggccgagcgcagaagtggtcctgcaactttatccgcctccatccagtctattaattgttgccgggaagctagagtaagtagttcgccagttaatagtttgcgcaacgttgttgccattgctacaggcatcgtggtgtcacgctcgtcgtttggtatggcttcattcagctccggttcccaacgatcaaggcgagttacatgatcccccatgttgtgcaaaaaagcggttagctccttcggtcctccgatcgttgtcagaagtaagttggccgcagtgttatcactcatggttatggcagcactgcataattctcttactgtcatgccatccgtaagatgcttttctgtgactggtgagtactcaaccaagtcattctgagaatagtgtatgcggcgaccgagttgctcttgcccggcgtcaatacgggataataccgcgccacatagcagaactttaaaagtgctcatcattggaaaacgttcttcggggcgaaaactctcaaggatcttaccgctgttgagatccagttcgatgtaacccactcgtgcacccaactgatcttcagcatcttttactttcaccagcgtttctgggtgagcaaaaacaggaaggcaaaatgccgcaaaaaagggaataagggcgacacggaaatgttgaatactcatactcttcctttttcaatattattgaagcatttatcagggttattgtctcatgagcggatacatatttgaatgtatttagaaaaataaacaaataggggttccgcgcacatttccccgaaaagtgccacctgacgtctaagaaaccattattatcatgacattaacctataaaaataggcgtatcacgaggccctttcgtc

SEQ ID NO: 47 - DNA, 3963 bp, Artificial
  pTK-VP7G4
tcgcgcgtttcggtgatgacggtgaaaacctctgacacatgcagctcccggagacggtcacagcttgtctgtaagcggatgccgggagcagacaagcccgtcagggcgcgtcagcgggtgttggcgggtgtcggggctggcttaactatgcggcatcagagcagattgtactgagagtgcaccatatgcggtgtgaaataccgcacagatgcgtaaggagaaaataccgcatcaggcgccattcgccattcaggctgcgcaactgttgggaagggcgatcggtgcgggcctcttcgctattacgccagctggcgaaagggggatgtgctgcaaggcgattaagttgggtaacgccagggttttcccagtcacgacgttgtaaaacgacggccagtgaattcgagctcggtacctaatacgactcactataggctttaaaagagagaatttccgtttggctagcggatagctccttttaatgtatggtattgaatataccacagttctattttatttgatatcgttcgttcttgtgagttatattctgaaaactatgataaagataatggactatttaatttatagaataacatttgtaattgtagtattatcagtattatcgaatgcacaaaattatggaataaatttgccaattactggatctatggatacagcatatgctaactcaacacaagacaataattttttatcttcaactttatgtctatattatccatcagaagctccaactcaaattagtgacactgaatggaaagatacactatctcaactgtttttaaccaaaggatggccgacaggttcagtttattttaatgaatattcaaacgttttagaattttccatcgacccaaagctatactgtgattataatgttgtgttaattagattcgcttctggtgaggagttggacgtatctgaattagctgatctaatactcaatgagtggttatgtaatccaatggatataacattatattattatcaacaaactggagaggcaaataagtggatatcaatgggatcatcatgtaccgttaaagtgtgtccattaaatactcagacattaggaattggatgtcaaacgacagatactgctacttttgaaacagttgctgacagcgaaaaattggcattaattgatgttgttgacaacgtaaatcataaattagatgttacatctactacgtgtacaatacggaattgtaataaactaggacctagagaaaatgtggctataatacaggttggcggttctaatatattagatataacagctgatcccacaacttctccacaaacagaacgaatgatgcgcgtaaactggaaaaaatggtggcaagtattctatactgtagttgattacattaatcaaatagtaaaagtaatgtccaaaagatcaagatcgttagattcgtcatctttctattatagagtatagatatatcctaaaatagaactgtttgatgtgaccgggtcggcatggcatctccacctcctcgcggtccgacctgggcatccgaaggaggacgtcgtccactcggatggctaagggagagctcaaaaaaaaggatccggctgctaacaaagcccgaaaggaagctgagttggctgctgccaccgctgagcaataactagcataaccccttggggcctctaaacgggtcttgaggggttttttggtcgactgcagaggcctgcatgcaagcttggcgtaatcatggtcatagctgtttcctgtgtgaaattgttatccgctcacaattccacacaacatacgagccggaagcataaagtgtaaagcctggggtgcctaatgagtgagctaactcacattaattgcgttgcgctcactgcccgctttccagtcgggaaacctgtcgtgccagctgcattaatgaatcggccaacgcgcggggagaggcggtttgcgtattgggcgctcttccgcttcctcgctcactgactcgctgcgctcggtcgttcggctgcggcgagcggtatcagctcactcaaaggcggtaatacggttatccacagaatcaggggataacgcaggaaagaacatgtgagcaaaaggccagcaaaaggccaggaaccgtaaaaaggccgcgttgctggcgtttttccataggctccgcccccctgacgagcatcacaaaaatcgacgctcaagtcagaggtggcgaaacccgacaggactataaagataccaggcgtttccccctggaagctccctcgtgcgctctcctgttccgaccctgccgcttaccggatacctgtccgcctttctcccttcgggaagcgtggcgctttctcatagctcacgctgtaggtatctcagttcggtgtaggtcgttcgctccaagctgggctgtgtgcacgaaccccccgttcagcccgaccgctgcgccttatccggtaactatcgtcttgagtccaacccggtaagacacgacttatcgccactggcagcagccactggtaacaggattagcagagcgaggtatgtaggcggtgctacagagttcttgaagtggtggcctaactacggctacactagaagaacagtatttggtatctgcgctctgctgaagccagttaccttcggaaaaagagttggtagctcttgatccggcaaacaaaccaccgctggtagcggtggtttttttgtttgcaagcagcagattacgcgcagaaaaaaaggatctcaagaagatcctttgatcttttctacggggtctgacgctcagtggaacgaaaactcacgttaagggattttggtcatgagattatcaaaaaggatcttcacctagatccttttaaattaaaaatgaagttttaaatcaatctaaagtatatatgagtaaacttggtctgacagttaccaatgcttaatcagtgaggcacctatctcagcgatctgtctatttcgttcatccatagttgcctgactccccgtcgtgtagataactacgatacgggagggcttaccatctggccccagtgctgcaatgataccgcgagacccacgctcaccggctccagatttatcagcaataaaccagccagccggaagggccgagcgcagaagtggtcctgcaactttatccgcctccatccagtctattaattgttgccgggaagctagagtaagtagttcgccagttaatagtttgcgcaacgttgttgccattgctacaggcatcgtggtgtcacgctcgtcgtttggtatggcttcattcagctccggttcccaacgatcaaggcgagttacatgatcccccatgttgtgcaaaaaagcggttagctccttcggtcctccgatcgttgtcagaagtaagttggccgcagtgttatcactcatggttatggcagcactgcataattctcttactgtcatgccatccgtaagatgcttttctgtgactggtgagtactcaaccaagtcattctgagaatagtgtatgcggcgaccgagttgctcttgcccggcgtcaatacgggataataccgcgccacatagcagaactttaaaagtgctcatcattggaaaacgttcttcggggcgaaaactctcaaggatcttaccgctgttgagatccagttcgatgtaacccactcgtgcacccaactgatcttcagcatcttttactttcaccagcgtttctgggtgagcaaaaacaggaaggcaaaatgccgcaaaaaagggaataagggcgacacggaaatgttgaatactcatactcttcctttttcaatattattgaagcatttatcagggttattgtctcatgagcggatacatatttgaatgtatttagaaaaataaacaaataggggttccgcgcacatttccccgaaaagtgccacctgacgtctaagaaaccattattatcatgacattaacctataaaaataggcgtatcacgaggccctttcgtc

SEQ ID NO: 48 - DNA, 3962 bp, Artificial
  pTK-VP7G9
tcgcgcgtttcggtgatgacggtgaaaacctctgacacatgcagctcccggagacggtcacagcttgtctgtaagcggatgccgggagcagacaagcccgtcagggcgcgtcagcgggtgttggcgggtgtcggggctggcttaactatgcggcatcagagcagattgtactgagagtgcaccatatgcggtgtgaaataccgcacagatgcgtaaggagaaaataccgcatcaggcgccattcgccattcaggctgcgcaactgttgggaagggcgatcggtgcgggcctcttcgctattacgccagctggcgaaagggggatgtgctgcaaggcgattaagttgggtaacgccagggttttcccagtcacgacgttgtaaaacgacggccagtgaattcgagctcggtacctaatacgactcactataggctttaaaagagagaatttccgcttggctaacggttagctccttttaatgtatggtattgaatataccacagttctaacctttttgatatcaatcattttgttgaattatatactaaaatcattaactagtgcaatggactttataatttatagattccttttgcttatagtcattgtatcaccatttgttaagacgcaaaattatggaattaatttaccaatcactggctccatggatacggcatatgcaaactcatcacagctagatacatttttaacttcaacgttatgtttatattaccctgctgaagcatcaactcaaattggagatacagaatggaaagacactctgtctcaattgttcttgactaaagggtggccaactgggtcagtctattttaaagaatatactgacatcgcttcattttctattgatccacaactttattgcgattataatgttgtattaatgaagtacgattcaacattagagttagacatgtctgaactagctgatttgattctaaacgaatggttatgtaatccgatggatataacactatattattatcaacaaacagatgaagcgaataaatggatagcgatgggacaatcttgtacaataaaagtgtgtccgttgaatacgcagactttaggaataggctgtacaactacaaatacagcaacatttgaggaagtggccgcaagtgaaaaattagtgataactgatgttgttgatggtgtgaatcataaactagatgtaactacaactacttgtactattagaaattgtagaaaattaggaccaagagagaatgtggcaattatacaagttggcggctcagaagtgctagatattacagcagacccaaccactgcgccacaaactgaacgtatgatgcgaataaattggaaaaaatggtggcaagttttttatacggtagtagattatatcaatcagattgtgcaagttatgtccaaaagatcgcgatcgttgaattcagcagctttctactatagagtctgatatatctcaggttagaattggtcgatgtgaccgggtcggcatggcatctccacctcctcgcggtccgacctgggcatccgaaggaggacgtcgtccactcggatggctaagggagagctcaaaaaaaaggatccggctgctaacaaagcccgaaaggaagctgagttggctgctgccaccgctgagcaataactagcataaccccttggggcctctaaacgggtcttgaggggttttttggtcgactgcagaggcctgcatgcaagcttggcgtaatcatggtcatagctgtttcctgtgtgaaattgttatccgctcacaattccacacaacatacgagccggaagcataaagtgtaaagcctggggtgcctaatgagtgagctaactcacattaattgcgttgcgctcactgcccgctttccagtcgggaaacctgtcgtgccagctgcattaatgaatcggccaacgcgcggggagaggcggtttgcgtattgggcgctcttccgcttcctcgctcactgactcgctgcgctcggtcgttcggctgcggcgagcggtatcagctcactcaaaggcggtaatacggttatccacagaatcaggggataacgcaggaaagaacatgtgagcaaaaggccagcaaaaggccaggaaccgtaaaaaggccgcgttgctggcgtttttccataggctccgcccccctgacgagcatcacaaaaatcgacgctcaagtcagaggtggcgaaacccgacaggactataaagataccaggcgtttccccctggaagctccctcgtgcgctctcctgttccgaccctgccgcttaccggatacctgtccgcctttctcccttcgggaagcgtggcgctttctcatagctcacgctgtaggtatctcagttcggtgtaggtcgttcgctccaagctgggctgtgtgcacgaaccccccgttcagcccgaccgctgcgccttatccggtaactatcgtcttgagtccaacccggtaagacacgacttatcgccactggcagcagccactggtaacaggattagcagagcgaggtatgtaggcggtgctacagagttcttgaagtggtggcctaactacggctacactagaagaacagtatttggtatctgcgctctgctgaagccagttaccttcggaaaaagagttggtagctcttgatccggcaaacaaaccaccgctggtagcggtggtttttttgtttgcaagcagcagattacgcgcagaaaaaaaggatctcaagaagatcctttgatcttttctacggggtctgacgctcagtggaacgaaaactcacgttaagggattttggtcatgagattatcaaaaaggatcttcacctagatccttttaaattaaaaatgaagttttaaatcaatctaaagtatatatgagtaaacttggtctgacagttaccaatgcttaatcagtgaggcacctatctcagcgatctgtctatttcgttcatccatagttgcctgactccccgtcgtgtagataactacgatacgggagggcttaccatctggccccagtgctgcaatgataccgcgagacccacgctcaccggctccagatttatcagcaataaaccagccagccggaagggccgagcgcagaagtggtcctgcaactttatccgcctccatccagtctattaattgttgccgggaagctagagtaagtagttcgccagttaatagtttgcgcaacgttgttgccattgctacaggcatcgtggtgtcacgctcgtcgtttggtatggcttcattcagctccggttcccaacgatcaaggcgagttacatgatcccccatgttgtgcaaaaaagcggttagctccttcggtcctccgatcgttgtcagaagtaagttggccgcagtgttatcactcatggttatggcagcactgcataattctcttactgtcatgccatccgtaagatgcttttctgtgactggtgagtactcaaccaagtcattctgagaatagtgtatgcggcgaccgagttgctcttgcccggcgtcaatacgggataataccgcgccacatagcagaactttaaaagtgctcatcattggaaaacgttcttcggggcgaaaactctcaaggatcttaccgctgttgagatccagttcgatgtaacccactcgtgcacccaactgatcttcagcatcttttactttcaccagcgtttctgggtgagcaaaaacaggaaggcaaaatgccgcaaaaaagggaataagggcgacacggaaatgttgaatactcatactcttcctttttcaatattattgaagcatttatcagggttattgtctcatgagcggatacatatttgaatgtatttagaaaaataaacaaataggggttccgcgcacatttccccgaaaagtgccacctgacgtctaagaaaccattattatcatgacattaacctataaaaataggcgtatcacgaggccctttcgtc

SEQ ID NO: 49 - DNA, 3963 bp, Artificial
  pTK-VP7B
tcgcgcgtttcggtgatgacggtgaaaacctctgacacatgcagctcccggagacggtcacagcttgtctgtaagcggatgccgggagcagacaagcccgtcagggcgcgtcagcgggtgttggcgggtgtcggggctggcttaactatgcggcatcagagcagattgtactgagagtgcaccatatgcggtgtgaaataccgcacagatgcgtaaggagaaaataccgcatcaggcgccattcgccattcaggctgcgcaactgttgggaagggcgatcggtgcgggcctcttcgctattacgccagctggcgaaagggggatgtgctgcaaggcgattaagttgggtaacgccagggttttcccagtcacgacgttgtaaaacgacggccagtgaattcgagctcggtacctaatacgactcactataggctttaaaagcgagaatttccgtttggctagcggttagctccttttaatgtatggtattgaatataccacaattctaatcttcttgacatcgattacattattgaattatatcttaaaatcaataacgagaataatggactatataatttatagatttttgtttatggtagtgatcttggccaccataataaatgcgcaaaactatggagtaaatttgccaattacaggttcaatggatactgcgtatgcaaactctacacaaagtgagccatttttgacatcaaccctttgtttgtattatcctgttgaggcatcaaacgaaatagctgatactgaatggaaagataccttatcacaactgttcttaacaaaaggatggccaacaggatcagtgtactttaaagaatatgctgatatagcggccttttcagtggaaccacagttatactgtgattataatttagttttaatgaaatatgactctacacaaaaactagatatgtctgaattggccgatcttatattgaatgaatggctgtgcaatccaatggacataacgctatattattatcagcagactgatgaggcaaataaatggatatcaatgggctcttcttgcacggttaaagtgtgtccattaaatacacaaacacttggtattggatgtctaataactaatccagacacgtttgaaacagttgcgacaacggagaaattagtgattacagatgttgtagatggtgtcaaccacaaattaaacgtcacaacggcaacgtgcaccatacgcaactgtaaaaagttaggaccaagggagaacgtagcagtcatacaggtaggcggcgcgaacattttagacatcacagctgatccaacaactacaccacagacagagagaatgatgcgaataaattggaaaaaatggtggcaagtgttttacacggtagtggattacgtcaatcaaataattcagacaatgtccaaaagatctagatcgcttaattcgtcggcgttctactatagagtgtaggtgcatgttagattagagttgtacgatgtgaccgggtcggcatggcatctccacctcctcgcggtccgacctgggcatccgaaggaggacgtcgtccactcggatggctaagggagagctcaaaaaaaaggatccggctgctaacaaagcccgaaaggaagctgagttggctgctgccaccgctgagcaataactagcataaccccttggggcctctaaacgggtcttgaggggttttttggtcgactgcagaggcctgcatgcaagcttggcgtaatcatggtcatagctgtttcctgtgtgaaattgttatccgctcacaattccacacaacatacgagccggaagcataaagtgtaaagcctggggtgcctaatgagtgagctaactcacattaattgcgttgcgctcactgcccgctttccagtcgggaaacctgtcgtgccagctgcattaatgaatcggccaacgcgcggggagaggcggtttgcgtattgggcgctcttccgcttcctcgctcactgactcgctgcgctcggtcgttcggctgcggcgagcggtatcagctcactcaaaggcggtaatacggttatccacagaatcaggggataacgcaggaaagaacatgtgagcaaaaggccagcaaaaggccaggaaccgtaaaaaggccgcgttgctggcgtttttccataggctccgcccccctgacgagcatcacaaaaatcgacgctcaagtcagaggtggcgaaacccgacaggactataaagataccaggcgtttccccctggaagctccctcgtgcgctctcctgttccgaccctgccgcttaccggatacctgtccgcctttctcccttcgggaagcgtggcgctttctcatagctcacgctgtaggtatctcagttcggtgtaggtcgttcgctccaagctgggctgtgtgcacgaaccccccgttcagcccgaccgctgcgccttatccggtaactatcgtcttgagtccaacccggtaagacacgacttatcgccactggcagcagccactggtaacaggattagcagagcgaggtatgtaggcggtgctacagagttcttgaagtggtggcctaactacggctacactagaagaacagtatttggtatctgcgctctgctgaagccagttaccttcggaaaaagagttggtagctcttgatccggcaaacaaaccaccgctggtagcggtggtttttttgtttgcaagcagcagattacgcgcagaaaaaaaggatctcaagaagatcctttgatcttttctacggggtctgacgctcagtggaacgaaaactcacgttaagggattttggtcatgagattatcaaaaaggatcttcacctagatccttttaaattaaaaatgaagttttaaatcaatctaaagtatatatgagtaaacttggtctgacagttaccaatgcttaatcagtgaggcacctatctcagcgatctgtctatttcgttcatccatagttgcctgactccccgtcgtgtagataactacgatacgggagggcttaccatctggccccagtgctgcaatgataccgcgagacccacgctcaccggctccagatttatcagcaataaaccagccagccggaagggccgagcgcagaagtggtcctgcaactttatccgcctccatccagtctattaattgttgccgggaagctagagtaagtagttcgccagttaatagtttgcgcaacgttgttgccattgctacaggcatcgtggtgtcacgctcgtcgtttggtatggcttcattcagctccggttcccaacgatcaaggcgagttacatgatcccccatgttgtgcaaaaaagcggttagctccttcggtcctccgatcgttgtcagaagtaagttggccgcagtgttatcactcatggttatggcagcactgcataattctcttactgtcatgccatccgtaagatgcttttctgtgactggtgagtactcaaccaagtcattctgagaatagtgtatgcggcgaccgagttgctcttgcccggcgtcaatacgggataataccgcgccacatagcagaactttaaaagtgctcatcattggaaaacgttcttcggggcgaaaactctcaaggatcttaccgctgttgagatccagttcgatgtaacccactcgtgcacccaactgatcttcagcatcttttactttcaccagcgtttctgggtgagcaaaaacaggaaggcaaaatgccgcaaaaaagggaataagggcgacacggaaatgttgaatactcatactcttcctttttcaatattattgaagcatttatcagggttattgtctcatgagcggatacatatttgaatgtatttagaaaaataaacaaataggggttccgcgcacatttccccgaaaagtgccacctgacgtctaagaaaccattattatcatgacattaacctataaaaataggcgtatcacgaggccctttcgtc

SEQ ID NO: 50 - DNA, 4479 bp, Artificial
  pTK-NSP1B
tcgcgcgtttcggtgatgacggtgaaaacctctgacacatgcagctcccggagacggtcacagcttgtctgtaagcggatgccgggagcagacaagcccgtcagggcgcgtcagcgggtgttggcgggtgtcggggctggcttaactatgcggcatcagagcagattgtactgagagtgcaccatatgcggtgtgaaataccgcacagatgcgtaaggagaaaataccgcatcaggcgccattcgccattcaggctgcgcaactgttgggaagggcgatcggtgcgggcctcttcgctattacgccagctggcgaaagggggatgtgctgcaaggcgattaagttgggtaacgccagggttttcccagtcacgacgttgtaaaacgacggccagtgaattcgagctcggtacctaatacgactcactataggctttttttatgaaaagtcttgtgtgagccatggcgacttttaaagacgcttgttatcattataaaaagttgaataagttaaatagtttagtgctcaaactaggagcaaatgatgaatggaggccagcaccagtgacaaaatataaaggatggtgtttagattgttgtcaatatacaaatttgacatattgcagagggtgcgctctataccatgtatgtcagtggtgcagtcagtataacaggtgtttcttagatgaagaaccccatttgctgagaatgcgaacatttaaagatgtagtaacaaaggaagatatagaagggctgctaaccatgtatgaaacgttgtttccaataaatgaaaagttggtgaataaattcataaactctgtgaaacagcgtaagtgtaggaatgaatatttgttagaatggtataatcacttactaatgccaataacattacaagcattgactataaatcttgaggataatgtatattatatatttggatactatgattgcatggagcatgaaaaccaaacaccattccaatttattaatctactagaaaaatatgataaattgctactagatgatagaaatttccatagaatgtcacacttaccagtaatattgcaacaagagtatgctttgagatatttttcaaaatcaagatttttaagtaaagggaagaagagattgagcaggagtgatttctcagatagtcttatggaagatagacatagtccaacatcattaatgcaagtggtacgtaactgcatcagtatacacataaatgattgtgaatggaataaagcgtgtacgcttatagttgatgctagaaattatattagtattatgaactcatcgtatactgagcattatagtgtgtcacaaagatgtaagttgtttactaagtataaatttgggatcgtatcaagattggtgaaaccgaattacattttttccagccatgaatcatgcgcattaaacgtacataactgtaaatggtgtcagatcaacaaccattacaaagtgtgggaagattttagacttaggaaaatatataataatgtaatggattttatcagggcacttgtgaaatcgaatggaaatgttggacattgttcatcccaggaatcagtgtataagtatataccagatttatttttaatttgtaaaacggaaaaatggaacgaagctgtcgaaatgttatttaattatctagaaccagtggacataaatggaacggagtatgtattattagactatgaagtgaactgggaagtgaggggactagtcatgcaaaacatggatgggaaagtaccaagaattttgaatatgaatgatacaaagaagatactgagtgcgatgatatttgactggtttgatacaagatatatgagagaaacaccaatgacgacgtcaacaacaaaccaacttcgaacactgaacaaaaggaatgaactcatagatgagtacgacttagaactttcagatgttgagtaaatatggtcacaactacgccagcacaagaccgtctgcactagagtagcgcctaggcagcataaaatgtgaccgggtcggcatggcatctccacctcctcgcggtccgacctgggcatccgaaggaggacgtcgtccactcggatggctaagggagagctcaaaaaaaaggatccggctgctaacaaagcccgaaaggaagctgagttggctgctgccaccgctgagcaataactagcataaccccttggggcctctaaacgggtcttgaggggttttttggtcgactgcagaggcctgcatgcaagcttggcgtaatcatggtcatagctgtttcctgtgtgaaattgttatccgctcacaattccacacaacatacgagccggaagcataaagtgtaaagcctggggtgcctaatgagtgagctaactcacattaattgcgttgcgctcactgcccgctttccagtcgggaaacctgtcgtgccagctgcattaatgaatcggccaacgcgcggggagaggcggtttgcgtattgggcgctcttccgcttcctcgctcactgactcgctgcgctcggtcgttcggctgcggcgagcggtatcagctcactcaaaggcggtaatacggttatccacagaatcaggggataacgcaggaaagaacatgtgagcaaaaggccagcaaaaggccaggaaccgtaaaaaggccgcgttgctggcgtttttccataggctccgcccccctgacgagcatcacaaaaatcgacgctcaagtcagaggtggcgaaacccgacaggactataaagataccaggcgtttccccctggaagctccctcgtgcgctctcctgttccgaccctgccgcttaccggatacctgtccgcctttctcccttcgggaagcgtggcgctttctcatagctcacgctgtaggtatctcagttcggtgtaggtcgttcgctccaagctgggctgtgtgcacgaaccccccgttcagcccgaccgctgcgccttatccggtaactatcgtcttgagtccaacccggtaagacacgacttatcgccactggcagcagccactggtaacaggattagcagagcgaggtatgtaggcggtgctacagagttcttgaagtggtggcctaactacggctacactagaagaacagtatttggtatctgcgctctgctgaagccagttaccttcggaaaaagagttggtagctcttgatccggcaaacaaaccaccgctggtagcggtggtttttttgtttgcaagcagcagattacgcgcagaaaaaaaggatctcaagaagatcctttgatcttttctacggggtctgacgctcagtggaacgaaaactcacgttaagggattttggtcatgagattatcaaaaaggatcttcacctagatccttttaaattaaaaatgaagttttaaatcaatctaaagtatatatgagtaaacttggtctgacagttaccaatgcttaatcagtgaggcacctatctcagcgatctgtctatttcgttcatccatagttgcctgactccccgtcgtgtagataactacgatacgggagggcttaccatctggccccagtgctgcaatgataccgcgagacccacgctcaccggctccagatttatcagcaataaaccagccagccggaagggccgagcgcagaagtggtcctgcaactttatccgcctccatccagtctattaattgttgccgggaagctagagtaagtagttcgccagttaatagtttgcgcaacgttgttgccattgctacaggcatcgtggtgtcacgctcgtcgtttggtatggcttcattcagctccggttcccaacgatcaaggcgagttacatgatcccccatgttgtgcaaaaaagcggttagctccttcggtcctccgatcgttgtcagaagtaagttggccgcagtgttatcactcatggttatggcagcactgcataattctcttactgtcatgccatccgtaagatgcttttctgtgactggtgagtactcaaccaagtcattctgagaatagtgtatgcggcgaccgagttgctcttgcccggcgtcaatacgggataataccgcgccacatagcagaactttaaaagtgctcatcattggaaaacgttcttcggggcgaaaactctcaaggatcttaccgctgttgagatccagttcgatgtaacccactcgtgcacccaactgatcttcagcatcttttactttcaccagcgtttctgggtgagcaaaaacaggaaggcaaaatgccgcaaaaaagggaataagggcgacacggaaatgttgaatactcatactcttcctttttcaatattattgaagcatttatcagggttattgtctcatgagcggatacatatttgaatgtatttagaaaaataaacaaataggggttccgcgcacatttccccgaaaagtgccacctgacgtctaagaaaccattattatcatgacattaacctataaaaataggcgtatcacgaggccctttcgtc

SEQ ID NO: 51 - DNA, 3960 bp, Artificial
  pTK-NSP2B
tcgcgcgtttcggtgatgacggtgaaaacctctgacacatgcagctcccggagacggtcacagcttgtctgtaagcggatgccgggagcagacaagcccgtcagggcgcgtcagcgggtgttggcgggtgtcggggctggcttaactatgcggcatcagagcagattgtactgagagtgcaccatatgcggtgtgaaataccgcacagatgcgtaaggagaaaataccgcatcaggcgccattcgccattcaggctgcgcaactgttgggaagggcgatcggtgcgggcctcttcgctattacgccagctggcgaaagggggatgtgctgcaaggcgattaagttgggtaacgccagggttttcccagtcacgacgttgtaaaacgacggccagtgaattcgagctcggtacctaatacgactcactataggcttttaaagcgtctcagtcgccgtttgagccttgcggtgtagccatggctgagctagcttgcttttgttatcctcatttggagaacgatagctatagattcattccatttaacagtttagctataaaatgtatgttgacagcaaaagtggacaaaaaagatcaagataaattttataattcaataatttatggtattgcaccaccgccacaattcaaaaaacgttataacacgaatgacaattcaagaggaatgaattatgaaactccaatgtttaataaagtggcggtgttaatttgtgaagcgttgaattcaattaaagttactcaatctgatgttgcgagtgtactttcaaaagtagtttctgtaagacatctagagaatttggtacggagaagagagaatcatcaggacgtgcttttccattcaaaagagttgttgttgaaatcagtactaatagctattggtcactcaaaagaaattgaaacgactgccactgctgaaggaggggaagtagtttttcaaaatgcagcttttacaatgtggaaattgacatacctggagcatagcctaatgccaattttggatcaaaattttattgaatataaaataacaatgaacgaagataaaccaatttcagaatcacatgttaaagaactgattgctgagttgcggtggcaatacaacaaatttgcagtaattacacatggtaaaggtcactacagagttgtaaaatattcatcagttgcgaatcatgcagatagagtttacgctactttcaagagtaataataagaatgggaatatgatagagtttaatctacttgatcaaagaataatatggcagaactggtatgcgtttacatcttcaatgaaacaaggtaacactcttgaagtatgtaagaaactactgttccaaaagatgaagcgagaaagtaatccgtttaagggactgtcaactgatagaaagatggatgaggtttctcaaataggaatttaattcgttatcgatttgagaatgggcatgacaaagcaagaatagaaagcgcttatgtgaccgggtcggcatggcatctccacctcctcgcggtccgacctgggcatccgaaggaggacgtcgtccactcggatggctaagggagagctcaaaaaaaaggatccggctgctaacaaagcccgaaaggaagctgagttggctgctgccaccgctgagcaataactagcataaccccttggggcctctaaacgggtcttgaggggttttttggtcgactgcagaggcctgcatgcaagcttggcgtaatcatggtcatagctgtttcctgtgtgaaattgttatccgctcacaattccacacaacatacgagccggaagcataaagtgtaaagcctggggtgcctaatgagtgagctaactcacattaattgcgttgcgctcactgcccgctttccagtcgggaaacctgtcgtgccagctgcattaatgaatcggccaacgcgcggggagaggcggtttgcgtattgggcgctcttccgcttcctcgctcactgactcgctgcgctcggtcgttcggctgcggcgagcggtatcagctcactcaaaggcggtaatacggttatccacagaatcaggggataacgcaggaaagaacatgtgagcaaaaggccagcaaaaggccaggaaccgtaaaaaggccgcgttgctggcgtttttccataggctccgcccccctgacgagcatcacaaaaatcgacgctcaagtcagaggtggcgaaacccgacaggactataaagataccaggcgtttccccctggaagctccctcgtgcgctctcctgttccgaccctgccgcttaccggatacctgtccgcctttctcccttcgggaagcgtggcgctttctcatagctcacgctgtaggtatctcagttcggtgtaggtcgttcgctccaagctgggctgtgtgcacgaaccccccgttcagcccgaccgctgcgccttatccggtaactatcgtcttgagtccaacccggtaagacacgacttatcgccactggcagcagccactggtaacaggattagcagagcgaggtatgtaggcggtgctacagagttcttgaagtggtggcctaactacggctacactagaagaacagtatttggtatctgcgctctgctgaagccagttaccttcggaaaaagagttggtagctcttgatccggcaaacaaaccaccgctggtagcggtggtttttttgtttgcaagcagcagattacgcgcagaaaaaaaggatctcaagaagatcctttgatcttttctacggggtctgacgctcagtggaacgaaaactcacgttaagggattttggtcatgagattatcaaaaaggatcttcacctagatccttttaaattaaaaatgaagttttaaatcaatctaaagtatatatgagtaaacttggtctgacagttaccaatgcttaatcagtgaggcacctatctcagcgatctgtctatttcgttcatccatagttgcctgactccccgtcgtgtagataactacgatacgggagggcttaccatctggccccagtgctgcaatgataccgcgagacccacgctcaccggctccagatttatcagcaataaaccagccagccggaagggccgagcgcagaagtggtcctgcaactttatccgcctccatccagtctattaattgttgccgggaagctagagtaagtagttcgccagttaatagtttgcgcaacgttgttgccattgctacaggcatcgtggtgtcacgctcgtcgtttggtatggcttcattcagctccggttcccaacgatcaaggcgagttacatgatcccccatgttgtgcaaaaaagcggttagctccttcggtcctccgatcgttgtcagaagtaagttggccgcagtgttatcactcatggttatggcagcactgcataattctcttactgtcatgccatccgtaagatgcttttctgtgactggtgagtactcaaccaagtcattctgagaatagtgtatgcggcgaccgagttgctcttgcccggcgtcaatacgggataataccgcgccacatagcagaactttaaaagtgctcatcattggaaaacgttcttcggggcgaaaactctcaaggatcttaccgctgttgagatccagttcgatgtaacccactcgtgcacccaactgatcttcagcatcttttactttcaccagcgtttctgggtgagcaaaaacaggaaggcaaaatgccgcaaaaaagggaataagggcgacacggaaatgttgaatactcatactcttcctttttcaatattattgaagcatttatcagggttattgtctcatgagcggatacatatttgaatgtatttagaaaaataaacaaataggggttccgcgcacatttccccgaaaagtgccacctgacgtctaagaaaccattattatcatgacattaacctataaaaataggcgtatcacgaggccctttcgtc

SEQ ID NO: 52 - DNA, 3963 bp, Artificial
  pTK-NSP3B
tcgcgcgtttcggtgatgacggtgaaaacctctgacacatgcagctcccggagacggtcacagcttgtctgtaagcggatgccgggagcagacaagcccgtcagggcgcgtcagcgggtgttggcgggtgtcggggctggcttaactatgcggcatcagagcagattgtactgagagtgcaccatatgcggtgtgaaataccgcacagatgcgtaaggagaaaataccgcatcaggcgccattcgccattcaggctgcgcaactgttgggaagggcgatcggtgcgggcctcttcgctattacgccagctggcgaaagggggatgtgctgcaaggcgattaagttgggtaacgccagggttttcccagtcacgacgttgtaaaacgacggccagtgaattctaatacgactcactataggcttttaatgcttttcagtggttgatgctcaagatggagtctacacagcagatggctagttcgattattaacacttcttttgaagccgcagtcgttgctgccacttcaactcttgaactcatgggcattcaatatgattataatgaagtttatactagagttaagagcaaatttgattacgtaatggatgattcaggtgttaaaaacaatctgttgggtaaagcggcaactattgatcaggcactgaatggaaaatttggttcagcagcaagaaatagaaattggatggccgatactagaactacagatagactagatgaagatgtgaacaaacttagaatgatgttatcatctaaaggaattgatcaaaaaatgagagtacttaatgcatgtttcagtgtgaagagagctccaggtaaatcatcatcaataattaaatgtactagactaatgagagataagattgaacgtggtgaagtcgaagtggatgattcgtttgttgaagaaaaaatggaagttgacacaattgattggaaatctaggtatgaacaattggaaaaacgatttgaatcactgaaacaaagggtgaatgaaaaatatacaagttgggtgcaaaaagcaaaaaaggtaaatgaaaatatgtactctctccaaaacgttatatcacaacagcagagccagattgctgatttacaaaattactgtaataaattggaagttgatctacagaataaaattagttcacttgtgtcttcagttgaatggtacctgaaatcaatggaattgcctgatgaaattaagacagatattgaacaacagctaaattccattgatgtaatcaatccaattaatgctatagatgattttgaatcactgatcagaaatattatactcgactatgacagaatatttttaatgttcaaaggattaatgaggcaatgcaactatgaatatacgtatgaatagtcacataatataattaaattaccatcttcacatgaccctctatgagcacaatagttaaaagctaacactgtcaaaaacctaaatggctataggggcgttatgtgaccgggtcggcatggcatctccacctcctcgcggtccgacctgggcatccgaaggaggacgtcgtccactcggatggctaagggagagctcaaaaaaaaggatccggctgctaacaaagcccgaaaggaagctgagttggctgctgccaccgctgagcaataactagcataaccccttggggcctctaaacgggtcttgaggggttttttggtcgactgcagaggcctgcatgcaagcttggcgtaatcatggtcatagctgtttcctgtgtgaaattgttatccgctcacaattccacacaacatacgagccggaagcataaagtgtaaagcctggggtgcctaatgagtgagctaactcacattaattgcgttgcgctcactgcccgctttccagtcgggaaacctgtcgtgccagctgcattaatgaatcggccaacgcgcggggagaggcggtttgcgtattgggcgctcttccgcttcctcgctcactgactcgctgcgctcggtcgttcggctgcggcgagcggtatcagctcactcaaaggcggtaatacggttatccacagaatcaggggataacgcaggaaagaacatgtgagcaaaaggccagcaaaaggccaggaaccgtaaaaaggccgcgttgctggcgtttttccataggctccgcccccctgacgagcatcacaaaaatcgacgctcaagtcagaggtggcgaaacccgacaggactataaagataccaggcgtttccccctggaagctccctcgtgcgctctcctgttccgaccctgccgcttaccggatacctgtccgcctttctcccttcgggaagcgtggcgctttctcatagctcacgctgtaggtatctcagttcggtgtaggtcgttcgctccaagctgggctgtgtgcacgaaccccccgttcagcccgaccgctgcgccttatccggtaactatcgtcttgagtccaacccggtaagacacgacttatcgccactggcagcagccactggtaacaggattagcagagcgaggtatgtaggcggtgctacagagttcttgaagtggtggcctaactacggctacactagaagaacagtatttggtatctgcgctctgctgaagccagttaccttcggaaaaagagttggtagctcttgatccggcaaacaaaccaccgctggtagcggtggtttttttgtttgcaagcagcagattacgcgcagaaaaaaaggatctcaagaagatcctttgatcttttctacggggtctgacgctcagtggaacgaaaactcacgttaagggattttggtcatgagattatcaaaaaggatcttcacctagatccttttaaattaaaaatgaagttttaaatcaatctaaagtatatatgagtaaacttggtctgacagttaccaatgcttaatcagtgaggcacctatctcagcgatctgtctatttcgttcatccatagttgcctgactccccgtcgtgtagataactacgatacgggagggcttaccatctggccccagtgctgcaatgataccgcgagacccacgctcaccggctccagatttatcagcaataaaccagccagccggaagggccgagcgcagaagtggtcctgcaactttatccgcctccatccagtctattaattgttgccgggaagctagagtaagtagttcgccagttaatagtttgcgcaacgttgttgccattgctacaggcatcgtggtgtcacgctcgtcgtttggtatggcttcattcagctccggttcccaacgatcaaggcgagttacatgatcccccatgttgtgcaaaaaagcggttagctccttcggtcctccgatcgttgtcagaagtaagttggccgcagtgttatcactcatggttatggcagcactgcataattctcttactgtcatgccatccgtaagatgcttttctgtgactggtgagtactcaaccaagtcattctgagaatagtgtatgcggcgaccgagttgctcttgcccggcgtcaatacgggataataccgcgccacatagcagaactttaaaagtgctcatcattggaaaacgttcttcggggcgaaaactctcaaggatcttaccgctgttgagatccagttcgatgtaacccactcgtgcacccaactgatcttcagcatcttttactttcaccagcgtttctgggtgagcaaaaacaggaaggcaaaatgccgcaaaaaagggaataagggcgacacggaaatgttgaatactcatactcttcctttttcaatattattgaagcatttatcagggttattgtctcatgagcggatacatatttgaatgtatttagaaaaataaacaaataggggttccgcgcacatttccccgaaaagtgccacctgacgtctaagaaaccattattatcatgacattaacctataaaaataggcgtatcacgaggccctttcgtc

SEQ ID NO: 53 - DNA, 3680 bp, Artificial
  pTK-NSP4B
tcgcgcgtttcggtgatgacggtgaaaacctctgacacatgcagctcccggagacggtcacagcttgtctgtaagcggatgccgggagcagacaagcccgtcagggcgcgtcagcgggtgttggcgggtgtcggggctggcttaactatgcggcatcagagcagattgtactgagagtgcaccatatgcggtgtgaaataccgcacagatgcgtaaggagaaaataccgcatcaggcgccattcgccattcaggctgcgcaactgttgggaagggcgatcggtgcgggcctcttcgctattacgccagctggcgaaagggggatgtgctgcaaggcgattaagttgggtaacgccagggttttcccagtcacgacgttgtaaaacgacggccagtgaattctaatacgactcactataggcttttaaaagttctgttccgagagagcgcgtgcggaaagatggaaaagcttaccgacctcaactatacattgagtgtaatcactctaatgaacagcacattgcacacgatacttgaggatccaggaatggcgtattttccctatatagcatctgtcctaacagttttgttcacgttgcacaaagcatctattccaacaatgaaaattgcattgaagacgtccaagtgttcatataaagtagtgaagtattgtattgtgacgattttcaatgcgttgttgaaattggcaggttataaagaacagattaccactaaagatgagatagaaaagcaaatggacagggtagtcaaagagatgagacgtcagctagaaatgattgataagttgactacacgtgaaattgagcaggtggaattactaaaacgcattcacgataagttgatgatacgagcagtagacgaaatagatatgacgaaggaaattaaccaaaagaacgtgaaaacgctagaagaatgggaaaatggaaaaaatccttatgaaccaaaagaagtgactgcagcaatgtaagaggttgagctgccgtcgactgtcttcggaagcgacggagttcttcacagtaagccccatcggacctgatggctgactgagaagccacagtcagtcatatcgcgtgtggcttaagccttaatcccgtttaaccaatccggtcagcaccggacgttaatggaaggaacggtcttaatgtgaccgggtcggcatggcatctccacctcctcgcggtccgacctgggcatccgaaggaggacgtcgtccactcggatggctaagggagagctcaaaaaaaaggatccggctgctaacaaagcccgaaaggaagctgagttggctgctgccaccgctgagcaataactagcataaccccttggggcctctaaacgggtcttgaggggttttttgggtacctcgcgaatgcatctagatatcggatcccgggcccgtcgactgcagaggcctgcatgcaagcttggcgtaatcatggtcatagctgtttcctgtgtgaaattgttatccgctcacaattccacacaacatacgagccggaagcataaagtgtaaagcctggggtgcctaatgagtgagctaactcacattaattgcgttgcgctcactgcccgctttccagtcgggaaacctgtcgtgccagctgcattaatgaatcggccaacgcgcggggagaggcggtttgcgtattgggcgctcttccgcttcctcgctcactgactcgctgcgctcggtcgttcggctgcggcgagcggtatcagctcactcaaaggcggtaatacggttatccacagaatcaggggataacgcaggaaagaacatgtgagcaaaaggccagcaaaaggccaggaaccgtaaaaaggccgcgttgctggcgtttttccataggctccgcccccctgacgagcatcacaaaaatcgacgctcaagtcagaggtggcgaaacccgacaggactataaagataccaggcgtttccccctggaagctccctcgtgcgctctcctgttccgaccctgccgcttaccggatacctgtccgcctttctcccttcgggaagcgtggcgctttctcatagctcacgctgtaggtatctcagttcggtgtaggtcgttcgctccaagctgggctgtgtgcacgaaccccccgttcagcccgaccgctgcgccttatccggtaactatcgtcttgagtccaacccggtaagacacgacttatcgccactggcagcagccactggtaacaggattagcagagcgaggtatgtaggcggtgctacagagttcttgaagtggtggcctaactacggctacactagaagaacagtatttggtatctgcgctctgctgaagccagttaccttcggaaaaagagttggtagctcttgatccggcaaacaaaccaccgctggtagcggtggtttttttgtttgcaagcagcagattacgcgcagaaaaaaaggatctcaagaagatcctttgatcttttctacggggtctgacgctcagtggaacgaaaactcacgttaagggattttggtcatgagattatcaaaaaggatcttcacctagatccttttaaattaaaaatgaagttttaaatcaatctaaagtatatatgagtaaacttggtctgacagttaccaatgcttaatcagtgaggcacctatctcagcgatctgtctatttcgttcatccatagttgcctgactccccgtcgtgtagataactacgatacgggagggcttaccatctggccccagtgctgcaatgataccgcgagacccacgctcaccggctccagatttatcagcaataaaccagccagccggaagggccgagcgcagaagtggtcctgcaactttatccgcctccatccagtctattaattgttgccgggaagctagagtaagtagttcgccagttaatagtttgcgcaacgttgttgccattgctacaggcatcgtggtgtcacgctcgtcgtttggtatggcttcattcagctccggttcccaacgatcaaggcgagttacatgatcccccatgttgtgcaaaaaagcggttagctccttcggtcctccgatcgttgtcagaagtaagttggccgcagtgttatcactcatggttatggcagcactgcataattctcttactgtcatgccatccgtaagatgcttttctgtgactggtgagtactcaaccaagtcattctgagaatagtgtatgcggcgaccgagttgctcttgcccggcgtcaatacgggataataccgcgccacatagcagaactttaaaagtgctcatcattggaaaacgttcttcggggcgaaaactctcaaggatcttaccgctgttgagatccagttcgatgtaacccactcgtgcacccaactgatcttcagcatcttttactttcaccagcgtttctgggtgagcaaaaacaggaaggcaaaatgccgcaaaaaagggaataagggcgacacggaaatgttgaatactcatactcttcctttttcaatattattgaagcatttatcagggttattgtctcatgagcggatacatatttgaatgtatttagaaaaataaacaaataggggttccgcgcacatttccccgaaaagtgccacctgacgtctaagaaaccattattatcatgacattaacctataaaaataggcgtatcacgaggccctttcgtc

SEQ ID NO: 54 - DNA, 3568 bp, Artificial
  pTK-NSP5B
tcgcgcgtttcggtgatgacggtgaaaacctctgacacatgcagctcccggagacggtcacagcttgtctgtaagcggatgccgggagcagacaagcccgtcagggcgcgtcagcgggtgttggcgggtgtcggggctggcttaactatgcggcatcagagcagattgtactgagagtgcaccatatgcggtgtgaaataccgcacagatgcgtaaggagaaaataccgcatcaggcgccattcgccattcaggctgcgcaactgttgggaagggcgatcggtgcgggcctcttcgctattacgccagctggcgaaagggggatgtgctgcaaggcgattaagttgggtaacgccagggttttcccagtcacgacgttgtaaaacgacggccagtgaattcgagctcggtacctaatacgactcactataggcttttaaagcgctacagtgatgtctctcagtattgacgtgacgagtcttccttctatttcttctagtatatacaaaaatgaatcatcttcaacaacgtcaactctttctggaaaatctattggtaggagtgaacaatacatttcaccagatgcagaagcattcagtaaatacatgctgtcaaagtctccagaagatattggaccatctgattctgcttcaaacgatccactcaccagcttttcgattagatcgaatgcagttaagacaaatgcagacgctggcgtgtctatggattcatcaacacaatcacggccatcaagcaatgttgggtgcgatcaagtggatttctcctttaataaaggaattaaaatgaacgcgaacctggattcatcaatatccatatcaactatttcgaaaaaggagaaatccaaaagcgaccataaaagtaggaaacactaccctaaaatagaagcagaatctgattcagatgactacgtactcgatgattctgatagtgatgatggtaaatgtaaaaactgtaaatataagaggaagtatttcgcactaagaatgagaatgaaacaagttgcaatgcaattgatcgaagatttgtaggtctaacctgagaggtcactagggagctccccactcccgttttgtgaccgggtcggcatggcatctccacctcctcgcggtccgacctgggcatccgaaggaggacgtcgtccactcggatggctaagggagagctcaaaaaaaaggatccggctgctaacaaagcccgaaaggaagctgagttggctgctgccaccgctgagcaataactagcataaccccttggggcctctaaacgggtcttgaggggttttttggtcgactgcagaggcctgcatgcaagcttggcgtaatcatggtcatagctgtttcctgtgtgaaattgttatccgctcacaattccacacaacatacgagccggaagcataaagtgtaaagcctggggtgcctaatgagtgagctaactcacattaattgcgttgcgctcactgcccgctttccagtcgggaaacctgtcgtgccagctgcattaatgaatcggccaacgcgcggggagaggcggtttgcgtattgggcgctcttccgcttcctcgctcactgactcgctgcgctcggtcgttcggctgcggcgagcggtatcagctcactcaaaggcggtaatacggttatccacagaatcaggggataacgcaggaaagaacatgtgagcaaaaggccagcaaaaggccaggaaccgtaaaaaggccgcgttgctggcgtttttccataggctccgcccccctgacgagcatcacaaaaatcgacgctcaagtcagaggtggcgaaacccgacaggactataaagataccaggcgtttccccctggaagctccctcgtgcgctctcctgttccgaccctgccgcttaccggatacctgtccgcctttctcccttcgggaagcgtggcgctttctcatagctcacgctgtaggtatctcagttcggtgtaggtcgttcgctccaagctgggctgtgtgcacgaaccccccgttcagcccgaccgctgcgccttatccggtaactatcgtcttgagtccaacccggtaagacacgacttatcgccactggcagcagccactggtaacaggattagcagagcgaggtatgtaggcggtgctacagagttcttgaagtggtggcctaactacggctacactagaagaacagtatttggtatctgcgctctgctgaagccagttaccttcggaaaaagagttggtagctcttgatccggcaaacaaaccaccgctggtagcggtggtttttttgtttgcaagcagcagattacgcgcagaaaaaaaggatctcaagaagatcctttgatcttttctacggggtctgacgctcagtggaacgaaaactcacgttaagggattttggtcatgagattatcaaaaaggatcttcacctagatccttttaaattaaaaatgaagttttaaatcaatctaaagtatatatgagtaaacttggtctgacagttaccaatgcttaatcagtgaggcacctatctcagcgatctgtctatttcgttcatccatagttgcctgactccccgtcgtgtagataactacgatacgggagggcttaccatctggccccagtgctgcaatgataccgcgagacccacgctcaccggctccagatttatcagcaataaaccagccagccggaagggccgagcgcagaagtggtcctgcaactttatccgcctccatccagtctattaattgttgccgggaagctagagtaagtagttcgccagttaatagtttgcgcaacgttgttgccattgctacaggcatcgtggtgtcacgctcgtcgtttggtatggcttcattcagctccggttcccaacgatcaaggcgagttacatgatcccccatgttgtgcaaaaaagcggttagctccttcggtcctccgatcgttgtcagaagtaagttggccgcagtgttatcactcatggttatggcagcactgcataattctcttactgtcatgccatccgtaagatgcttttctgtgactggtgagtactcaaccaagtcattctgagaatagtgtatgcggcgaccgagttgctcttgcccggcgtcaatacgggataataccgcgccacatagcagaactttaaaagtgctcatcattggaaaacgttcttcggggcgaaaactctcaaggatcttaccgctgttgagatccagttcgatgtaacccactcgtgcacccaactgatcttcagcatcttttactttcaccagcgtttctgggtgagcaaaaacaggaaggcaaaatgccgcaaaaaagggaataagggcgacacggaaatgttgaatactcatactcttcctttttcaatattattgaagcatttatcagggttattgtctcatgagcggatacatatttgaatgtatttagaaaaataaacaaataggggttccgcgcacatttccccgaaaagtgccacctgacgtctaagaaaccattattatcatgacattaacctataaaaataggcgtatcacgaggccctttcgtc

SEQ ID NO: 55 - DNA, 6364 bp, Artificial
  pCMVTK-D1R
tcgcgcgtttcggtgatgacggtgaaaacctctgacacatgcagctcccggagacggtcacagcttgtctgtaagcggatgccgggagcagacaagcccgtcagggcgcgtcagcgggtgttggcgggtgtcggggctggcttaactatgcggcatcagagcagattgtactgagagtgcaccatatgcggtgtgaaataccgcacagatgcgtaaggagaaaataccgcatcaggcgccattcgccattcaggctgcgcaactgttgggaagggcgatcggtgcgggcctcttcgctattacgccagctggcgaaagggggatgtgctgcaaggcgattaagttgggtaacgccagggttttcccagtcacgacgttgtaaaacgacggccagtgaattcacattgattattgactagttattaatagtaatcaattacggggtcattagttcatagcccatatatggagttccgcgttacataacttacggtaaatggcccgcctggctgaccgcccaacgacccccgcccattgacgtcaataatgacgtatgttcccatagtaacgccaatagggactttccattgacgtcaatgggtggagtatttacggtaaactgcccacttggcagtacatcaagtgtatcatatgccaagtacgccccctattgacgtcaatgacggtaaatggcccgcctggcattatgcccagtacatgaccttatgggactttcctacttggcagtacatctacgtattagtcatcgctattaccatggtgatgcggttttggcagtacatcaatgggcgtggatagcggtttgactcacggggatttccaagtctccaccccattgacgtcaatgggagtttgttttggcaccaaaatcaacgggactttccaaaatgtcgtaacaactccgccccattgacgcaaatgggcggtaggcgtgtacggtgggaggtctatataagcagagctctctggctaactagagaacccactgcttactggcttatcgaaatgagctcggtaccatggatgccaacgtagtatcatcttctactattgcgacgtatatagacgctttagcgaagaatgcttcggaattagaacagaggtctaccgcatacgaaataaataatgaattggaactagtatttattaagccgccattgattactttgacaaatgtagtgaatatctctacgattcaggaatcgtttattcgatttaccgttactaataaggaaggtgttaaaattagaactaagattccattatctaaggtacatggtctagatgtaaaaaatgtacagttagtagatgctatagataacatagtttgggaaaagaaatcattagtgacggaaaatcgtcttcacaaagaatgcttgttgagactatcgacagaggaacgtcatatatttttggattacaagaaatatggatcctctatccgactagaattagtcaatcttattcaagcaaaaacaaaaaactttacgatagactttaagctaaaatattttctaggatccggtgcccagtctaaaagttctttattacacgctattaatcatccaaagtcaaggcctaatacatctctggaaatagaatttacacctagagacaatgaaacagttccatatgatgaactaataaaggaattgacgactctctcgcgtcatatatttatggcttctccagagaatgtaattctttctccgcctattaacgcgcctataaaaacctttatgttgcctaaacaagatatagtaggtttggatctggaaaatctatatgccgtaactaagactgacggcattcctataactatcagagttacatcaaacgggttgtattgttattttacacatcttggttatattattagatatcctgttaagagaataatagattccgaagtagtagtctttggtgaggcagttaaggataagaactggaccgtatatctcattaagctaatagagcctgtgaatgcaatcaatgatagactagaagaaagtaagtatgttgaatctaaactagtggatatttgtgatcggatagtattcaagtcaaagaaatacgaaggtccgtttactacaactagtgaagtcgtcgatatgttatctacatatttaccaaagcaaccagaaggtgttattctgttctattcaaagggacctaaatctaacattgattttaaaattaaaaaggaaaatactatagaccaaactgcaaatgtagtatttaggtacatgtccagtgaaccaattatctttggagagtcgtctatctttgtagagtataagaaatttagcaacgataaaggctttcctaaagaatatggttctggtaagattgtgttatataacggcgttaattatctaaataatatctattgtttggaatatattaatacacataatgaagtgggtattaagtccgtggttgtacctattaagtttatagcagaattcttagttaatggagaaatacttaaacctagaattgataaaaccatgaaatatattaactcagaagattattatggaaatcaacataatatcatagtcgaacatttaagagatcaaagcatcaaaataggagatatctttaacgaggataaactatcggatgtgggacatcaatacgccaataatgataaatttagattaaatccagaagttagttattttacgaataaacgaactagaggaccgttgggaattttatcaaactacgtcaagactcttcttatttctatgtattgttccaaaacatttttagacgattccaacaaacgaaaggtattggcgattgattttggaaacggtgctgacctggaaaaatacttttatggagagattgcgttattggtagcgacggatccggatgctgatgctatagctagaggaaatgaaagatacaacaaattaaactctggaattaaaaccaagtactacaaatttgactacattcaggaaactattcgatccgatacatttgtctctagtgtcagagaagtattctattttggaaagtttaatatcatcgactggcagtttgctatccattattcttttcatccgagacattatgctaccgtcatgaataacttatccgaactaactgcttctggaggcaaggtattaatcactaccatggacggagacaaattatcaaaattaacagataaaaagacttttataattcataagaatttacctagtagcgaaaactatatgtctgtagaaaaaatagctgatgatagaatagtggtatataatccatcaacaatgtctactccaatgactgaatacattatcaaaaagaacgatatagtcagagtgtttaacgaatacggatttgttcttgtagataacgttgatttcgctacaattatagaacgaagtaaaaagtttattaatggcgcatctacaatggaagatagaccatctacaagaaactttttcgaactaaatagaggagccattaaatgtgaaggtttagatgtcgaagacttacttagttactatgttgtttatgtcttttctaagcggtaagtcgactgcagaggcctgcatgcctcctcaggtgcaggctgcctatcagaaggtggtggctggtgtggccaatgccctggctcacaaataccactgagatcgatctttttccctctgccaaaaattatggggacatcatgaagccccttgagcatctgacttctggctaataaaggaaatttattttcattgcaatagtgtgttggaattttttgtgtctctcactcggaaggacatatgggagggcaaatcatttaaaacatcagaatgagtatttggtttagagtttggcaacatatgcccatatgctggctgccatgaacaaaggttggctataaagaggtcatcagtatatgaaacagccccctgctgtccattccttattccatagaaaagccttgacttgaggttagattttttttatattttgttttgtgttatttttttctttaacatccctaaaattttccttacatgttttactagccagatttttcctcctctcctgactactcccagtcatagctgtccctcttctcttatggagataagcttggcgtaatcatggtcatagctgtttcctgtgtgaaattgttatccgctcacaattccacacaacatacgagccggaagcataaagtgtaaagcctggggtgcctaatgagtgagctaactcacattaattgcgttgcgctcactgcccgctttccagtcgggaaacctgtcgtgccagctgcattaatgaatcggccaacgcgcggggagaggcggtttgcgtattgggcgctcttccgcttcctcgctcactgactcgctgcgctcggtcgttcggctgcggcgagcggtatcagctcactcaaaggcggtaatacggttatccacagaatcaggggataacgcaggaaagaacatgtgagcaaaaggccagcaaaaggccaggaaccgtaaaaaggccgcgttgctggcgtttttccataggctccgcccccctgacgagcatcacaaaaatcgacgctcaagtcagaggtggcgaaacccgacaggactataaagataccaggcgtttccccctggaagctccctcgtgcgctctcctgttccgaccctgccgcttaccggatacctgtccgcctttctcccttcgggaagcgtggcgctttctcatagctcacgctgtaggtatctcagttcggtgtaggtcgttcgctccaagctgggctgtgtgcacgaaccccccgttcagcccgaccgctgcgccttatccggtaactatcgtcttgagtccaacccggtaagacacgacttatcgccactggcagcagccactggtaacaggattagcagagcgaggtatgtaggcggtgctacagagttcttgaagtggtggcctaactacggctacactagaagaacagtatttggtatctgcgctctgctgaagccagttaccttcggaaaaagagttggtagctcttgatccggcaaacaaaccaccgctggtagcggtggtttttttgtttgcaagcagcagattacgcgcagaaaaaaaggatctcaagaagatcctttgatcttttctacggggtctgacgctcagtggaacgaaaactcacgttaagggattttggtcatgagattatcaaaaaggatcttcacctagatccttttaaattaaaaatgaagttttaaatcaatctaaagtatatatgagtaaacttggtctgacagttaccaatgcttaatcagtgaggcacctatctcagcgatctgtctatttcgttcatccatagttgcctgactccccgtcgtgtagataactacgatacgggagggcttaccatctggccccagtgctgcaatgataccgcgagacccacgctcaccggctccagatttatcagcaataaaccagccagccggaagggccgagcgcagaagtggtcctgcaactttatccgcctccatccagtctattaattgttgccgggaagctagagtaagtagttcgccagttaatagtttgcgcaacgttgttgccattgctacaggcatcgtggtgtcacgctcgtcgtttggtatggcttcattcagctccggttcccaacgatcaaggcgagttacatgatcccccatgttgtgcaaaaaagcggttagctccttcggtcctccgatcgttgtcagaagtaagttggccgcagtgttatcactcatggttatggcagcactgcataattctcttactgtcatgccatccgtaagatgcttttctgtgactggtgagtactcaaccaagtcattctgagaatagtgtatgcggcgaccgagttgctcttgcccggcgtcaatacgggataataccgcgccacatagcagaactttaaaagtgctcatcattggaaaacgttcttcggggcgaaaactctcaaggatcttaccgctgttgagatccagttcgatgtaacccactcgtgcacccaactgatcttcagcatcttttactttcaccagcgtttctgggtgagcaaaaacaggaaggcaaaatgccgcaaaaaagggaataagggcgacacggaaatgttgaatactcatactcttcctttttcaatattattgaagcatttatcagggttattgtctcatgagcggatacatatttgaatgtatttagaaaaataaacaaataggggttccgcgcacatttccccgaaaagtgccacctgacgtctaagaaaccattattatcatgacattaacctataaaaataggcgtatcacgaggccctttcgtc

SEQ ID NO: 56 - DNA, 4693 bp, Artificial
  pCMVTK-D12L
tcgcgcgtttcggtgatgacggtgaaaacctctgacacatgcagctcccggagacggtcacagcttgtctgtaagcggatgccgggagcagacaagcccgtcagggcgcgtcagcgggtgttggcgggtgtcggggctggcttaactatgcggcatcagagcagattgtactgagagtgcaccatatgcggtgtgaaataccgcacagatgcgtaaggagaaaataccgcatcaggcgccattcgccattcaggctgcgcaactgttgggaagggcgatcggtgcgggcctcttcgctattacgccagctggcgaaagggggatgtgctgcaaggcgattaagttgggtaacgccagggttttcccagtcacgacgttgtaaaacgacggccagtgaattcacattgattattgactagttattaatagtaatcaattacggggtcattagttcatagcccatatatggagttccgcgttacataacttacggtaaatggcccgcctggctgaccgcccaacgacccccgcccattgacgtcaataatgacgtatgttcccatagtaacgccaatagggactttccattgacgtcaatgggtggagtatttacggtaaactgcccacttggcagtacatcaagtgtatcatatgccaagtacgccccctattgacgtcaatgacggtaaatggcccgcctggcattatgcccagtacatgaccttatgggactttcctacttggcagtacatctacgtattagtcatcgctattaccatggtgatgcggttttggcagtacatcaatgggcgtggatagcggtttgactcacggggatttccaagtctccaccccattgacgtcaatgggagtttgttttggcaccaaaatcaacgggactttccaaaatgtcgtaacaactccgccccattgacgcaaatgggcggtaggcgtgtacggtgggaggtctatataagcagagctctctggctaactagagaacccactgcttactggcttatcgaaatgagctcggtaccatggatgaaattgtaaaaaatatccgggagggaacgcatgtccttcttccattttatgaaacattgccagaacttaatctgtctctaggtaaaagcccattacctagtctggaatacggagctaattactttcttcagatttctagagttaatgatctaaatagaatgccgaccgacatgttaaaactttttacacatgatatcatgttaccagaaagcgatctagataaagtctatgaaattttaaagattaatagcgtaaagtattatgggaggagtactaaagcggacgccgtagttgccgacctcagcgcacgcaataaactgttcaaacgtgaacgagatgctattaaatctaataatcatctcactgaaaacaatctatacattagcgattataagatgttaaccttcgacgtgtttcgaccattatttgattttgtaaacgaaaaatattgtattattaaacttccaactttattcggtagaggtgtaatcgatactatgagaatatattgtagtctctttaaaaatgttagactgctaaaatgcgtaagcgatagctggttaaaagatagcgccattatggtggctagtgatgtttgtaaaaaaaatttggatttatttatgtctcatgttaagtccgtcactaagtcttcttcttggaaggatgtgaacagtgttcaatttagtattttaaacaatccagtggatacggaattcattaataagttcttagagttttcgaatagagtatacgaagctctctattacgttcactcgttgctttattctagtatgacttctgattcaaaaagtatcgaaaacaaacatcagagaagactagttaaactactgctgtgagtcgactgcagaggcctgcatgcctcctcaggtgcaggctgcctatcagaaggtggtggctggtgtggccaatgccctggctcacaaataccactgagatcgatctttttccctctgccaaaaattatggggacatcatgaagccccttgagcatctgacttctggctaataaaggaaatttattttcattgcaatagtgtgttggaattttttgtgtctctcactcggaaggacatatgggagggcaaatcatttaaaacatcagaatgagtatttggtttagagtttggcaacatatgcccatatgctggctgccatgaacaaaggttggctataaagaggtcatcagtatatgaaacagccccctgctgtccattccttattccatagaaaagccttgacttgaggttagattttttttatattttgttttgtgttatttttttctttaacatccctaaaattttccttacatgttttactagccagatttttcctcctctcctgactactcccagtcatagctgtccctcttctcttatggagataagcttggcgtaatcatggtcatagctgtttcctgtgtgaaattgttatccgctcacaattccacacaacatacgagccggaagcataaagtgtaaagcctggggtgcctaatgagtgagctaactcacattaattgcgttgcgctcactgcccgctttccagtcgggaaacctgtcgtgccagctgcattaatgaatcggccaacgcgcggggagaggcggtttgcgtattgggcgctcttccgcttcctcgctcactgactcgctgcgctcggtcgttcggctgcggcgagcggtatcagctcactcaaaggcggtaatacggttatccacagaatcaggggataacgcaggaaagaacatgtgagcaaaaggccagcaaaaggccaggaaccgtaaaaaggccgcgttgctggcgtttttccataggctccgcccccctgacgagcatcacaaaaatcgacgctcaagtcagaggtggcgaaacccgacaggactataaagataccaggcgtttccccctggaagctccctcgtgcgctctcctgttccgaccctgccgcttaccggatacctgtccgcctttctcccttcgggaagcgtggcgctttctcatagctcacgctgtaggtatctcagttcggtgtaggtcgttcgctccaagctgggctgtgtgcacgaaccccccgttcagcccgaccgctgcgccttatccggtaactatcgtcttgagtccaacccggtaagacacgacttatcgccactggcagcagccactggtaacaggattagcagagcgaggtatgtaggcggtgctacagagttcttgaagtggtggcctaactacggctacactagaagaacagtatttggtatctgcgctctgctgaagccagttaccttcggaaaaagagttggtagctcttgatccggcaaacaaaccaccgctggtagcggtggtttttttgtttgcaagcagcagattacgcgcagaaaaaaaggatctcaagaagatcctttgatcttttctacggggtctgacgctcagtggaacgaaaactcacgttaagggattttggtcatgagattatcaaaaaggatcttcacctagatccttttaaattaaaaatgaagttttaaatcaatctaaagtatatatgagtaaacttggtctgacagttaccaatgcttaatcagtgaggcacctatctcagcgatctgtctatttcgttcatccatagttgcctgactccccgtcgtgtagataactacgatacgggagggcttaccatctggccccagtgctgcaatgataccgcgagacccacgctcaccggctccagatttatcagcaataaaccagccagccggaagggccgagcgcagaagtggtcctgcaactttatccgcctccatccagtctattaattgttgccgggaagctagagtaagtagttcgccagttaatagtttgcgcaacgttgttgccattgctacaggcatcgtggtgtcacgctcgtcgtttggtatggcttcattcagctccggttcccaacgatcaaggcgagttacatgatcccccatgttgtgcaaaaaagcggttagctccttcggtcctccgatcgttgtcagaagtaagttggccgcagtgttatcactcatggttatggcagcactgcataattctcttactgtcatgccatccgtaagatgcttttctgtgactggtgagtactcaaccaagtcattctgagaatagtgtatgcggcgaccgagttgctcttgcccggcgtcaatacgggataataccgcgccacatagcagaactttaaaagtgctcatcattggaaaacgttcttcggggcgaaaactctcaaggatcttaccgctgttgagatccagttcgatgtaacccactcgtgcacccaactgatcttcagcatcttttactttcaccagcgtttctgggtgagcaaaaacaggaaggcaaaatgccgcaaaaaagggaataagggcgacacggaaatgttgaatactcatactcttcctttttcaatattattgaagcatttatcagggttattgtctcatgagcggatacatatttgaatgtatttagaaaaataaacaaataggggttccgcgcacatttccccgaaaagtgccacctgacgtctaagaaaccattattatcatgacattaacctataaaaataggcgtatcacgaggccctttcgtc